European Patent Specification EP 3 694 886 B1, published April 1, 2026. Title: COMPOUND CHIMERIC ANTIGEN RECEPTOR (cCAR) TARGETING MULTIPLE ANTIGENS, COMPOSITIONS AND METHODS OF USE THEREOF. Applicant: iCELL GENE THERAPEUTICS LLC MA, Yupo. The sequence listing filed with the application follows.

SEQUENCE LISTING (61 sequences)

SEQ ID NO: 1 - protein, 734 aa, Artificial Sequence
  Synthetic Sequence
MALPVTALLLPLALLLHAARPEVQLQQSGPELIKPGASVKMSCKASGYTFTSYVMHWVKQKPGQGLEWIGYINPYNDGTKYNEKFKGKATLTSDKSSSTAYMELSSLTSEDSAVYYCARGTYYYGSRVFDYWGQGTTLTVSSGGGGSGGGGSGGGGSDIVMTQAAPSIPVTPGESVSISCRSSKSLLNSNGNTYLYWFLQRPGQSPQLLIYRMSNLASGVPDRFSGSGSGTAFTLRISRVEAEDVGVYYCMQHLEYPFTFGAGTKLELKRTTTPAPRPPTPAPTIASQPLSLRPEACRPAAGGAVHTRGLDFACDIYIWAPLAGTCGVLLLSLVITLYCRSKRSRLLHSDYMNMTPRRPGPTRKHYQPYAPPRDFAAYRSRVKFSRSADAPAYQQGQNQLYNELNLGRREEYDVLDKRRGRDPEMGGKPQRRKNPQEGLYNELQKDKMAEAYSEIGMKGERRRGKGHDGLYQGLSTATKDTYDALHMQALPPRGSGEGRGSLLTCGDVEENPGPMYRMQLLSCIALSLALVTNSQGQDRHMIRMRQLIDIVDQLKNYVNDLVPEFLPAPEDVETNCEWSAFSCFQKAQLKSANTGNNERIINVSIKKLKRKPPSTNAGRRQKHRLTCPSCDSYEKKPPKEFLERFKSLLQKMIHQHLSSRTHGSEDSTTTPAPRPPTPAPTIASQPLSLRPEACRPAAGGAVHTRGLDFACDVAISTSTVLLCGLSAVSLLACY

SEQ ID NO: 2 - DNA, 2221 bp, Artificial Sequence
  Synthetic Sequence
gcgatcgcatggccttaccagtgaccgccttgctcctgccgctggccttgctgctccacgccgccaggccggaggtccagctgcagcagtctggacctgagctgataaagcctggggcttcagtgaagatgtcctgcaaggcttctggatacacattcactagctatgttatgcactgggtgaagcagaagcctgggcagggccttgagtggattggatatattaatccttacaatgatggtactaagtacaatgagaagttcaaaggcaaggccacactgacttcagacaaatcctccagcacagcctacatggagctcagcagcctgacctctgaggactctgcggtctattactgtgcaagagggacttattactacggtagtagggtatttgactactggggccaaggcaccactctcacagtctcctcaggtggagggggctcaggcggaggtggctctgggggtggaggctcggacattgtgatgactcaggctgcaccctctatacctgtcactcctggagagtcagtatccatctcctgcaggtctagtaagagtctcctgaatagtaatggcaacacttacttgtattggttcctgcagaggccaggccagtctcctcagctcctgatatatcggatgtccaaccttgcctcaggagtcccagacaggttcagtggcagtgggtcaggaactgctttcacactgagaatcagtagagtggaggctgaggatgtgggtgtttattactgtatgcaacatctagaatatccgttcacgttcggtgctgggaccaagctggagctgaaacggaccacgacgccagcgccgcgaccaccaacaccggcgcccaccatcgcgtcgcagcccctgtccctgcgcccagaggcgtgccggccagcggcggggggcgcagtgcacacgagggggctggacttcgcctgtgatatctacatctgggcgcccttggccgggacttgtggggtccttctcctgtcactggttatcaccctttactgcaggagtaagaggagcaggctcctgcacagtgactacatgaacatgactccccgccgccccgggcccacccgcaagcattaccagccctatgccccaccacgcgacttcgcagcctatcgctccagagtgaagttcagcaggagcgcagacgcccccgcgtaccagcagggccagaaccagctctataacgagctcaatctaggacgaagagaggagtacgatgttttggacaagagacgtggccgggaccctgagatggggggaaagccgcagagaaggaagaaccctcaggaaggcctgtacaatgaactgcagaaagataagatggcggaggcctacagtgagattgggatgaaaggcgagcgccggaggggcaaggggcacgatggcctttaccagggtctcagtacagccaccaaggacacctacgacgcccttcacatgcaggccctgccccctcgcggcagcggcgaaggccgcggcagcctgctgacctgcggcgatgtggaagaaaacccgggccccatgtacagaatgcagctgctgagctgcatcgccctgagcctggccctggtgaccaacagccagggccaggacaggcacatgatcaggatgaggcagctgatcgacatcgtggaccagctgaagaactacgtgaacgacctggtgcccgagttcctgcccgcccccgaggacgtggagaccaactgcgagtggagcgccttcagctgcttccagaaggcccagctgaagagcgccaacaccggcaacaacgagaggatcatcaacgtgagcatcaagaagctgaagaggaagccccccagcaccaacgccggcaggaggcagaagcacaggctgacctgccccagctgcgacagctacgagaagaagccccccaaggagttcctggagaggttcaagagcctgctgcagaagatgatccaccagcacctgagcagcaggacccacggcagcgaggacagcaccaccacccccgcccccaggccccccacccccgcccccaccatcgccagccagcccctgagcctgaggcccgaggcctgcaggcccgccgccggcggcgccgtgcacaccaggggcctggacttcgcctgcgacgtggctatctccacgtccactgtcctgctgtgtgggctgagcgctgtgtctctcctggcatgctactaagtttaaac

SEQ ID NO: 3 - protein, 997 aa, Artificial Sequence
  Synthetic Sequence
MALPVTALLLPLALLLHAARPDVVMTQSHRFMSTSVGDRVSITCRASQDVNTAVSWYQQKPGQSPKLLIFSASYRYTGVPDRFTGSGSGADFTLTISSVQAEDLAVYYCQQHYSTPWTFGGGTKLDIKGGGGSGGGGSGGGGSQIQLVQSGPDLKKPGETVKLSCKASGYTFTNFGMNWVKQAPGKGFKWMAWINTYTGESYFADDFKGRFAFSVETSATTAYLQINNLKTEDTATYFCARGEIYYGYDGGFAYWGQGTLVTVSATTTPAPRPPTPAPTIASQPLSLRPEACRPAAGGAVHTRGLDFACDIYIWAPLAGTCGVLLLSLVITLYCRSKRSRLLHSDYMNMTPRRPGPTRKHYQPYAPPRDFAAYRSRVKFSRSADAPAYQQGQNQLYNELNLGRREEYDVLDKRRGRDPEMGGKPQRRKNPQEGLYNELQKDKMAEAYSEIGMKGERRRGKGHDGLYQGLSTATKDTYDALHMQALPPRGSGATNFSLLKQAGDVEENPGPMALPVTALLLPLALLLHAARPDIVLTQSPPSLAMSLGKRATISCRASESVTILGSHLIHWYQQKPGQPPTLLIQLASNVQTGVPARFSGSGSRTDFTLTIDPVEEDDVAVYYCLQSRTIPRTFGGGTKLEIKGGGGSGGGGSGGGGSQIQLVQSGPELKKPGETVKISCKASGYTFTDYSINWVKRAPGKGLKWMGWINTETREPAYAYDFRGRFAFSLETSASTAYLQINNLKYEDTATYFCALDYSYAMDYWGQGTSVTVSSTTTPAPRPPTPAPTIASQPLSLRPEACRPAAGGAVHTRGLDFACDIYIWAPLAGTCGVLLLSLVITLYCRSKRSRLLHSDYMNMTPRRPGPTRKHYQPYAPPRDFAAYRSRVKFSRSADAPAYQQGQNQLYNELNLGRREEYDVLDKRRGRDPEMGGKPQRRKNPQEGLYNELQKDKMAEAYSEIGMKGERRRGKGHDGLYQGLSTATKDTYDALHMQALPPR

SEQ ID NO: 4 - DNA, 3013 bp, Artificial Sequence
  Synthetic Sequence
ggcgatcgcaccatggccttaccagtgaccgccttgctcctgccgctggccttgctgctccacgccgccaggccggacgtggtgatgacccagaccacaggttcatgagcaccagcgtgggcgacagggtgagcatcacctgcagggccagccaggacgtgaacaccgccgtgagctggtaccagcagaagcccggccagagccccaagctgctgatcttcagcgccagctacaggtacaccggcgtgcccgacaggttcaccggcagcggcagcggcgccgacttcaccctgaccatcagcagcgtgcaggccgaggacctggccgtgtactactgccagcagcactacagcaccccctggaccttcggcggcggcaccaagctggacatcaagggaggggggggatccgggggaggaggctccggcggaggcggaagccagatccagctggtgcagagcggccccgacctgaagaagcccggcgagaccgtgaagctgagctgcaaggccagcggctacaccttcaccaacttcggcatgaactgggtgaagcaggcccccggcaagggcttcaagtggatggcctggatcaacacctacaccggcgagagctacttcgccgacgacttcaagggcaggttcgccttcagcgtggagaccagcgccaccaccgcctacctgcagatcaacaacctgaagaccgaggacaccgccacctacttctgcgccaggggcgagatctactacggctacgacggcggcttcgcctactggggccagggcaccctggtgaccgtgagcgccaccacgacgccagcgccgcgaccaccaacaccggcgcccaccatcgcgtcgcagcccctgtccctgcgcccagaggcgtgccggccagcggcggggggcgcagtgcacacgagggggctggacttcgcctgtgatatctacatctgggcgcccttggccgggacttgtggggtccttctcctgtcactggttatcaccctttactgcaggagtaagaggagcaggctcctgcacagtgactacatgaacatgactccccgccgccccgggcccacccgcaagcattaccagccctatgccccaccacgcgacttcgcagcctatcgctccagagtgaagttcagcaggagcgcagacgcccccgcgtaccagcagggccagaaccagctctataacgagctcaatctaggacgaagagaggagtacgatgttttggacaagagacgtggccgggaccctgagatggggggaaagccgcagagaaggaagaaccctcaggaaggcctgtacaatgaactgcagaaagataagatggcggaggcctacagtgagattgggatgaaaggcgagcgccggaggggcaaggggcacgatggcctttaccagggtctcagtacagccaccaaggacacctacgacgcccttcacatgcaggccctgccccctcgcggaagcggagccaccaacttcagcctgctgaagcaggccggcgacgtggaggagaaccccggccccatggccttaccagtgaccgccttgctcctgccgctggccttgctgctccacgccgccaggccggacatcgtgctgacccagagcccccccagcctggccatgagcctgggcaagagggccaccatcagctgcagggccagcgagagcgtgaccatcctgggcagccacctgatccactggtaccagcagaagcccggccagccccccaccctgctgatccagctggccagcaacgtgcagaccggcgtgcccgccaggttcagcggcagcggcagcaggaccgacttcaccctgaccatcgaccccgtggaggaggacgacgtggccgtgtactactgcctgcagagcaggaccatccccaggaccttcggcggcggcaccaagctggagatcaagggaggggggggatccgggggaggaggctccggcggaggcggaagccagatccagctggtgcagagcggccccgagctgaagaagcccggcgagaccgtgaagatcagctgcaaggccagcggctacaccttcaccgactacagcatcaactgggtgaagagggcccccggcaagggcctgaagtggatgggctggatcaacaccgagaccagggagcccgcctacgcctacgacttcaggggcaggttcgccttcagcctggagaccagcgccagcaccgcctacctgcagatcaacaacctgaagtacgaggacaccgccacctacttctgcgccctggactacagctacgccatggactactggggccagggcaccagcgtgaccgtgagcagcaccacgacgccagcgccgcgaccaccaacaccggcgcccaccatcgcgtcgcagcccctgtccctgcgcccagaggcgtgccggccagcggcggggggcgcagtgcacacgagggggctggacttcgcctgtgatatctacatctgggcgcccttggccgggacttgtggggtccttctcctgtcactggttatcaccctttactgcaggagtaagaggagcaggctcctgcacagtgactacatgaacatgactccccgccgccccgggcccacccgcaagcattaccagccctatgccccaccacgcgacttcgcagcctatcgctccagagtgaagttcagcaggagcgcagacgcccccgcgtaccagcagggccagaaccagctctataacgagctcaatctaggacgaagagaggagtacgatgttttggacaagagacgtggccgggaccctgagatggggggaaagccgcagagaaggaagaaccctcaggaaggcctgtacaatgaactgcagaaagataagatggcggaggcctacagtgagattgggatgaaaggcgagcgccggaggggcaaggggcacgatggcctttaccagggtctcagtacagccaccaaggacacctacgacgcccttcacatgcaggccctgccccctcgctaagtttaaac

SEQ ID NO: 5 - protein, 1005 aa, Artificial Sequence
  Synthetic Sequence
MALPVTALLLPLALLLHAARPDVVMTQSHRFMSTSVGDRVSITCRASQDVNTAVSWYQQKPGQSPKLLIFSASYRYTGVPDRFTGSGSGADFTLTISSVQAEDLAVYYCQQHYSTPWTFGGGTKLDIKGGGGSGGGGSGGGGSQIQLVQSGPDLKKPGETVKLSCKASGYTFTNFGMNWVKQAPGKGFKWMAWINTYTGESYFADDFKGRFAFSVETSATTAYLQINNLKTEDTATYFCARGEIYYGYDGGFAYWGQGTLVTVSATTTPAPRPPTPAPTIASQPLSLRPEACRPAAGGAVHTRGLDFACDIYIWAPLAGTCGVLLLSLVITLYCRSKRSRLLHSDYMNMTPRRPGPTRKHYQPYAPPRDFAAYRSRVKFSRSADAPAYQQGQNQLYNELNLGRREEYDVLDKRRGRDPEMGGKPQRRKNPQEGLYNELQKDKMAEAYSEIGMKGERRRGKGHDGLYQGLSTATKDTYDALHMQALPPRGSGATNFSLLKQAGDVEENPGPMALPVTALLLPLALLLHAARPDIVMTQSPLSLPVTPGEPASISCRSSQSLLFIDGNNYLNWYLQKPGQSPQLLIYLGSNRASGVPDRFSGSGSGTDFTLKISRVEAEDVGVYYCQQYSSKSATFGQGTKVEIKRTGGGGSGGGGSGGGGSQVQLVQSGAEVKKPGASVKVSCKASGYTFTSYSINWVRQAPGQGLEWMGYIDPNRGNTNYAQKFQGRVTMTRDTSISTAYMELSSLRSEDTAVYYCAREYIYFIHGMLDFWGQGTLVTVSSTTTPAPRPPTPAPTIASQPLSLRPEACRPAAGGAVHTRGLDFACDIYIWAPLAGTCGVLLLSLVITLYCKRGRKKLLYIFKQPFMRPVQTTQEEDGCSCRFPEEEEGGCELRVKFSRSADAPAYQQGQNQLYNELNLGRREEYDVLDKRRGRDPEMGGKPQRRKNPQEGLYNELQKDKMAEAYSEIGMKGERRRGKGHDGLYQGLSTATKDTYDALHMQALPPR

SEQ ID NO: 6 - DNA, 2966 bp, Artificial Sequence
  Synthetic Sequence
atggccttaccagtgaccgccttgctcctgccgctggccttgctgctccacgccgccaggccggacgtggtgatgacccagagccacaggttcatgagcaccagcgtgggcgacagggtgagcatcacctgcagggccagccaggacgtgaacaccgccgtgagctggtaccagcagaagcccggccagagccccaagctgctgatcttcagcgccagctacaggtacaccggcgtgcccgacaggttcaccggcagcggcagcggcgccgacttcaccctgaccatcagcagcgtgcaggccgaggacctggccgtgtactactgccagcagcactacagcaccccctggaccttcggcggcggcaccaagctggacatcaagggaggggggggatccgggggaggaggctccggcggaggcggaagccagatccagctggtgcagagcggccccgacctgaagaagcccggcgagaccgtgaagctgagctgcaaggccagcggctacaccttcaccaacttcggcatgaactgggtgaagcaggcccccggcaagggcttcaagtggatggcctggatcaacacctacaccggcgagagctacttcgccgacgacttcaagggcaggttcgccttcagcgtggagaccagcgccaccaccgcctacctgcagatcaacaacctgaagaccgaggacaccgccacctacttctgcgccaggggcgagatctactacggctacgacggcggcttcgcctactggggccagggcaccctggtgaccgtgagcgccaccacgacgccagcgccgcgaccaccaacaccggcgcccaccatcgcgtcgcagcccctgtccctgcgcccagaggcgtgccggccagcggcggggggcgcagtgcacacgagggggctggacttcgcctgtgatatctacatctgggcgcccttggccgggacttgtggggtccttctcctgtcactggttatcaccctttactgcaggagtaagaggagcaggctcctgcacagtgactacatgaacatgactccccgccgccccgggcccacccgcaagcattaccagccctatgccccaccacgcgacttcgcagcctatcgctccagagtgaagttcagcaggagcgcagacgcccccgcgtaccagcagggccagaaccagctctataacgagctcaatctaggacgaagagaggagtacgatgttttggacaagagacgtggccgggaccctgagatggggggaaagccgcagagaaggaagaaccctcaggaaggcctgtacaatgaactgcagaaagataagatggcggaggcctacagtgagattgggatgaaaggcgagcgccggaggggcaaggggcacgatggcctttaccagggtctcagtacagccaccaaggacacctacgacgcccttcacatgcaggccctgccccctcgcggaagcggagccaccaacttcagcctgctgaagcaggccggcgacgtggaggagaaccccggccccatggccctgcccgtgaccgccctgctgctgcccctggccctgctgctgcacgccgccaggcccgacatcgtgatgacccagagccccctgagcctgcccgtgacccccggcgagcccgccagctacctgcagaagcccggccagagcccccagctgctgatctacctgggcagcaacagggccagcggcgtgcccgacaggttcagcggcagcggcagcggcaccgacttcaccctgaagatcagcagggtggaggccgaggacgtgggcgtgtactactgccagcagtacagcagcaagagcgccaccttcggccagggcaccaaggtggagatcaagaggaccggcggcggcggcagcggcggcggcggcagcggcggcggcggcagccaggtgcagctggtgcagagcggcgccgaggtgaagaagcccggcgccagcgtgaaggtgagctgcaaggccagcggctacaccttcaccagctacagcatcaactgggtgaggcaggcccccggccagggcctggagtggatgggctacatcgaccccaacaggggcaacaccaactacgcccagaagttccagggcagggtgaccatgaccagggacaccagcatcagcaccgcctacatggagctgagcagcctgaggagcgaggacaccgccgtgtactactgcgccagggagtacatctacttcatccacggcatgctggacttctggggccagggcaccctggtgaccgtgagcagcaccaccacccccgcccccaggccccccacccccgcccccaccatcgccagccagcccctgagcctgaggcccgaggcctgcaggcccgccgccggcggcgccgtgcacaccaggggcctggacttcgcctgcgacatctacatctgggcccccctggccggcacctgcggcgtgctgctgctgagcctggtgatcaccctgtactgcaaacggggcagaaagaaactcctgtatatattcaaacaaccatttatgagaccagtacaaactactcaagaggaagatggctgtagctgccgatttccagaagaagaagaaggaggatgtgaactgagggtgaagttcagcaggagcgccgacgcccccgcctaccagcagggccagaaccagctgtacaacgagctgaacctgggcaggagggaggagtacgacgtgctggacaagaggaggggcagggaccccgagatgggcggcaagccccagaggaggaagaacccccaggagggcctgtacaacgagctgcagaaggacaagatggccgaggcctacagcgagatcggcatgaagggcgagaggaggaggggcaagggccacgacggcctgtaccagggcctgagcaccgccaccaaggacacctacgacgccctgcacatgcaggccctgccccccaggtaagtttaaac

SEQ ID NO: 7 - protein, 1001 aa, Artificial Sequence
  Synthetic Sequence
MALPVTALLLPLALLLHAARPDVVMTQSHRFMSTSVGDRVSITCRASQDVNTAVSWYQQKPGQSPKLLIFSASYRYTGVPDRFTGSGSGADFTLTISSVQAEDLAVYYCQQHYSTPWTFGGGTKLDIKGGGGSGGGGSGGGGSQIQLVQSGPDLKKPGETVKLSCKASGYTFTNFGMNWVKQAPGKGFKWMAWINTYTGESYFADDFKGRFAFSVETSATTAYLQINNLKTEDTATYFCARGEIYYGYDGGFAYWGQGTLVTVSATTTPAPRPPTPAPTIASQPLSLRPEACRPAAGGAVHTRGLDFACDIYIWAPLAGTCGVLLLSLVITLYCRSKRSRLLHSDYMNMTPRRPGPTRKHYQPYAPPRDFAAYRSRVKFSRSADAPAYQQGQNQLYNELNLGRREEYDVLDKRRGRDPEMGGKPQRRKNPQEGLYNELQKDKMAEAYSEIGMKGERRRGKGHDGLYQGLSTATKDTYDALHMQALPPRGSGATNFSLLKQAGDVEENPGPMALPVTALLLPLALLLHAARPDIQMTQSPSSLSASVGDRVTITCRASQDISAFLNWYQQKPGKAPKLLITKVSNLQSGVPSRFSGSGSGTDFTLTISSLQPEDFATYYCQQAYSGSITFGQGTKVEIKRTGGGGSGGGGSGGGGSQVQLVESGGGLVQPGGSLRLSCAASGFTFSNYGMHWVRQAPGKGLEWVSNIRSDGSWTYYADSVKGRFTISRDNSKNTLYLQMNSLRAEDTAVYYCARRYWSKSHASVTDYWGQGTLVTVSSTTTPAPRPPTPAPTIASQPLSLRPEACRPAAGGAVHTRGLDFACDIYIWAPLAGTCGVLLLSLVITLYCKRGRKKLLYIFKQPFMRPVQTTQEEDGCSCRFPEEEEGGCELRVKFSRSADAPAYQQGQNQLYNELNLGRREEYDVLDKRRGRDPEMGGKPQRRKNPQEGLYNELQKDKMAEAYSEIGMKGERRRGKGHDGLYQGLSTATKDTYDALHMQALPPR

SEQ ID NO: 8 - DNA, 3014 bp, Artificial Sequence
  Synthetic Sequences
atggccttaccagtgaccgccttgctcctgccgctggccttgctgctccacgccgccaggccggacgtggtgatgacccagagccacaggttcatgagcaccagcgtgggcgacagggtgagcatcacctgcagggccagccaggacgtgaacaccgccgtgagctggtaccagcagaagcccggccagagccccaagctgctgatcttcagcgccagctacaggtacaccggcgtgcccgacaggttcaccggcagcggcagcggcgccgacttcaccctgaccatcagcagcgtgcaggccgaggacctggccgtgtactactgccagcagcactacagcaccccctggaccttcggcggcggcaccaagctggacatcaagggaggggggggatccgggggaggaggctccggcggaggcggaagccagatccagctggtgcagagcggccccgacctgaagaagcccggcgagaccgtgaagctgagctgcaaggccagcggctacaccttcaccaacttcggcatgaactgggtgaagcaggcccccggcaagggcttcaagtggatggcctggatcaacacctacaccggcgagagctacttcgccgacgacttcaagggcaggttcgccttcagcgtggagaccagcgccaccaccgcctacctgcagatcaacaacctgaagaccgaggacaccgccacctacttctgcgccaggggcgagatctactacggctacgacggcggcttcgcctactggggccagggcaccctggtgaccgtgagcgccaccacgacgccagcgccgcgaccaccaacaccggcgcccaccatcgcgtcgcagcccctgtccctgcgcccagaggcgtgccggccagcggcggggggcgcagtgcacacgagggggctggacttcgcctgtgatatctacatctgggcgcccttggccgggacttgtggggtccttctcctgtcactggttatcaccctttactgcaggagtaagaggagcaggctcctgcacagtgactacatgaacatgactccccgccgccccgggcccacccgcaagcattaccagccctatgccccaccacgcgacttcgcagcctatcgctccagagtgaagttcagcaggagcgcagacgcccccgcgtaccagcagggccagaaccagctctataacgagctcaatctaggacgaagagaggagtacgatgttttggacaagagacgtggccgggaccctgagatggggggaaagccgcagagaaggaagaaccctcaggaaggcctgtacaatgaactgcagaaagataagatggcggaggcctacagtgagattgggatgaaaggcgagcgccggaggggcaaggggcacgatggcctttaccagggtctcagtacagccaccaaggacacctacgacgcccttcacatgcaggccctgccccctcgcggaagcggagccaccaacttcagcctgctgaagcaggccggcgacgtggaggagaaccccggccccatggccctgcccgtgaccgccctgctgctgcccctggccctgctgctgcacgccgccaggcccgacatccagatgacccagagccccagcagcctgagcgccagcgtgggcgacagggtgaccatcacctgcagggccagccaggacatcagcgccttcctgaactggtaccagcagaagcccggcaaggcccccaagctgctgatcaccaaggtgagcaacctgcagagcggcgtgcccagcaggttcagcggcagcggcagcggcaccgacttcaccctgaccatcagcagcctgcagcccgaggacttcgccacctactactgccagcaggcctacagcggcagcatcaccttcggccagggcaccaaggtggagatcaagaggaccggcggcggcggcagcggcggcggcggcagcggcggcggcggcagccaggtgcagctggtggagagcggcggcggcctggtgcagcccggcggcagcctgaggctgagctgcgccgccagcggcttcaccttcagcaactacggcatgcactgggtgaggcaggcccccggcaagggcctggagtgggtgagcaacatcaggagcgacggcagctggacctactacgccgacagcgtgaagggcaggttcaccatcagcagggacaacagcaagaacaccctgtacctgcagatgaacagcctgagggccgaggacaccgccgtgtactactgcgccaggaggtactggagcaagagccacgccagcgtgaccgactactggggccagggcaccctggtgaccgtgagcagcaccaccacccccgcccccaggccccccacccccgcccccaccatcgccagccagcccctgagcctgaggcccgaggcctgcaggcccgccgccggcggcgccgtgcacaccaggggcctggacttcgcctgcgacatctacatctgggcccccctggccggcacctgcggcgtgctgctgctgagcctggtgatcaccctgtactgcaaacggggcagaaagaaactcctgtatatattcaaacaaccatttatgagaccagtacaaactactcaagaggaagatggctgtagctgccgatttccagaagaagaagaaggaggatgtgaactgagggtgaagttcagcaggagcgccgacgcccccgcctaccagcagggccagaaccagctgtacaacgagctgaacctgggcaggagggaggagtacgacgtgctggacaagaggaggggcagggaccccgagatgggcggcaagccccagaggaggaagaacccccaggagggcctgtacaacgagctgcagaaggacaagatggccgaggcctacagcgagatcggcatgaagggcgagaggaggaggggcaagggccacgacggcctgtaccagggcctgagcaccgccaccaaggacacctacgacgccctgcacatgcaggccctgccccccaggtaagtttaaac

SEQ ID NO: 9 - protein, 1004 aa, Artificial Sequence
  Synthetic Sequence
MALPVTALLLPLALLLHAARPDVVMTQSHRFMSTSVGDRVSITCRASQDVNTAVSWYQQKPGQSPKLLIFSASYRYTGVPDRFTGSGSGADFTLTISSVQAEDLAVYYCQQHYSTPWTFGGGTKLDIKGGGGSGGGGSGGGGSQIQLVQSGPDLKKPGETVKLSCKASGYTFTNFGMNWVKQAPGKGFKWMAWINTYTGESYFADDFKGRFAFSVETSATTAYLQINNLKTEDTATYFCARGEIYYGYDGGFAYWGQGTLVTVSATTTPAPRPPTPAPTIASQPLSLRPEACRPAAGGAVHTRGLDFACDIYIWAPLAGTCGVLLLSLVITLYCRSKRSRLLHSDYMNMTPRRPGPTRKHYQPYAPPRDFAAYRSRVKFSRSADAPAYQQGQNQLYNELNLGRREEYDVLDKRRGRDPEMGGKPQRRKNPQEGLYNELQKDKMAEAYSEIGMKGERRRGKGHDGLYQGLSTATKDTYDALHMQALPPRGSGATNFSLLKQAGDVEENPGPMALPVTALLLPLALLLHAARPAQPAMAKVQLQESGPSLVQPSQRLSITCTVSGFSLISYGVHWVRQSPGKGLEWLGVIWRGGSTDYNAAFMSRLSITKDNSKSQVFFKMNSLQADDTAIYFCAKTLITTGYAMDYWGQGTTVTVSSGGGGSGGGGSGGGGSDIELTQSPSSFSVSLGDRVTITCKASEDIYNRLAWYQQKPGNAPRLLISGATSLETGVPSRFSGSGSGKDYTLSITSLQTEDVATYYCQQYWSTPTFGGGTKLEIKRAATTTPAPRPPTPAPTIASQPLSLRPEACRPAAGGAVHTRGLDFACDIYIWAPLAGTCGVLLLSLVITLYCKRGRKKLLYIFKQPFMRPVQTTQEEDGCSCRFPEEEEGGCELRVKFSRSADAPAYQQGQNQLYNELNLGRREEYDVLDKRRGRDPEMGGKPQRRKNPQEGLYNELQKDKMAEAYSEIGMKGERRRGKGHDGLYQGLSTATKDTYDALHMQALPPR

SEQ ID NO: 10 - DNA, 3023 bp, Artificial Sequence
  Synthetic Sequence
atggccttaccagtgaccgccttgctcctgccgctggccttgctgctccacgccgccaggccggacgtggtgatgacccagagccacaggttcatgagcaccagcgtgggcgacagggtgagcatcacctgcagggccagccaggacgtgaacaccgccgtgagctggtaccagcagaagcccggccagagccccaagctgctgatcttcagcgccagctacaggtacaccggcgtgcccgacaggttcaccggcagcggcagcggcgccgacttcaccctgaccatcagcagcgtgcaggccgaggacctggccgtgtactactgccagcagcactacagcaccccctggaccttcggcggcggcaccaagctggacatcaagggaggggggggatccgggggaggaggctccggcggaggcggaagccagatccagctggtgcagagcggccccgacctgaagaagcccggcgagaccgtgaagctgagctgcaaggccagcggctacaccttcaccaacttcggcatgaactgggtgaagcaggcccccggcaagggcttcaagtggatggcctggatcaacacctacaccggcgagagctacttcgccgacgacttcaagggcaggttcgccttcagcgtggagaccagcgccaccaccgcctacctgcagatcaacaacctgaagaccgaggacaccgccacctacttctgcgccaggggcgagatctactacggctacgacggcggcttcgcctactggggccagggcaccctggtgaccgtgagcgccaccacgacgccagcgccgcgaccaccaacaccggcgcccaccatcgcgtcgcagcccctgtccctgcgcccagaggcgtgccggccagcggcggggggcgcagtgcacacgagggggctggacttcgcctgtgatatctacatctgggcgcccttggccgggacttgtggggtccttctcctgtcactggttatcaccctttactgcaggagtaagaggagcaggctcctgcacagtgactacatgaacatgactccccgccgccccgggcccacccgcaagcattaccagccctatgccccaccacgcgacttcgcagcctatcgctccagagtgaagttcagcaggagcgcagacgcccccgcgtaccagcagggccagaaccagctctataacgagctcaatctaggacgaagagaggagtacgatgttttggacaagagacgtggccgggaccctgagatggggggaaagccgcagagaaggaagaaccctcaggaaggcctgtacaatgaactgcagaaagataagatggcggaggcctacagtgagattgggatgaaaggcgagcgccggaggggcaaggggcacgatggcctttaccagggtctcagtacagccaccaaggacacctacgacgcccttcacatgcaggccctgccccctcgcggaagcggagccaccaacttcagcctgctgaagcaggccggcgacgtggaggagaaccccggccccatggccctgcccgtgaccgccctgctgctgcccctggccctgctgctgcacgccgccaggcccgcccagcccgccatggccaaggtgcagctgcaggagagcggccccagcctggtgcagcccagccagaggctgagcatcacctgcaccgtgagcggcttcagcctgatcagctacggcgtgcactgggtgaggcagagccccggcaagggcctggagtggctgggcgtgatctggaggggcggcagcaccgactacaacgccgccttcatgagcaggctgagcatcaccaaggacaacagcaagagccaggtgttcttcaagatgaacagcctgcaggccgacgacaccgccatctacttctgcgccaagaccctgatcaccaccggctacgccatggactactggggccagggcaccaccgtgaccgtgagcagcggcggcggcggcagcggcggcggcggcagcggcggcggcggcagcgacatcgagctgacccagagccccagcagcttcagcgtgagcctgggcgacagggtgaccatcacctgcaaggccagcgaggacatctacaacaggctggcctggtaccagcagaagcccggcaacgcccccaggctgctgatcagcggcgccaccagcctggagaccggcgtgcccagcaggttcagcggcagcggcagcggcaaggactacaccctgagcatcaccagcctgcagaccgaggacgtggccacctactactgccagcagtactggagcacccccaccttcggcggcggcaccaagctggagatcaagagggccgccaccaccacccccgcccccaggccccccacccccgcccccaccatcgccagccagcccctgagcctgaggcccgaggcctgcaggcccgccgccggcggcgccgtgcacaccaggggcctggacttcgcctgcgacatctacatctgggcccccctggccggcacctgcggcgtgctgctgctgagcctggtgatcaccctgtactgcaaacggggcagaaagaaactcctgtatatattcaaacaaccatttatgagaccagtacaaactactcaagaggaagatggctgtagctgccgatttccagaagaagaagaaggaggatgtgaactgagggtgaagttcagcaggagcgccgacgcccccgcctaccagcagggccagaaccagctgtacaacgagctgaacctgggcaggagggaggagtacgacgtgctggacaagaggaggggcagggaccccgagatgggcggcaagccccagaggaggaagaacccccaggagggcctgtacaacgagctgcagaaggacaagatggccgaggcctacagcgagatcggcatgaagggcgagaggaggaggggcaagggccacgacggcctgtaccagggcctgagcaccgccaccaaggacacctacgacgccctgcacatgcaggccctgccccccaggtaagtttaaac

SEQ ID NO: 11 - protein, 687 aa, Artificial Sequence
  Synthetic Sequence
MALPVTALLLPLALLLHAARPDVVMTQSHRFMSTSVGDRVSITCRASQDVNTAVSWYQQKPGQSPKLLIFSASYRYTGVPDRFTGSGSGADFTLTISSVQAEDLAVYYCQQHYSTPWTFGGGTKLDIKGGGGSGGGGSGGGGSQIQLVQSGPDLKKPGETVKLSCKASGYTFTNFGMNWVKQAPGKGFKWMAWINTYTGESYFADDFKGRFAFSVETSATTAYLQINNLKTEDTATYFCARGEIYYGYDGGFAYWGQGTLVTVSATTTPAPRPPTPAPTIASQPLSLRPEACRPAAGGAVHTRGLDFACDIYIWAPLAGTCGVLLLSLVITLYCRSKRSRLLHSDYMNMTPRRPGPTRKHYQPYAPPRDFAAYRSRVKFSRSADAPAYQQGQNQLYNELNLGRREEYDVLDKRRGRDPEMGGKPQRRKNPQEGLYNELQKDKMAEAYSEIGMKGERRRGKGHDGLYQGLSTATKDTYDALHMQALPPRGSGATNFSLLKQAGDVEENPGPMYRMQLLSCIALSLALVTNSYFGKLESKLSVIRNLNDQVLFIDQGNRPLFEDMTDSDCRDNAPRTIFIISMYKDSQPRGMAVTISVKCEKISTLSCENKIISFKEMNPPDNIKDTKSDIIFFQRSVPGHDNKMQFESSSYEGYFLACEKERDLFKLILKKEDELGDRSIMFTVQNED

SEQ ID NO: 12 - DNA, 2061 bp, Artificial Sequence
  Synthetic Sequence
atggccttaccagtgaccgccttgctcctgccgctggccttgctgctccacgccgccaggccggacgtggtgatgacccagagccacaggttcatgagcaccagcgtgggcgacagggtgagcatcacctgcagggccagccaggacgtgaacaccgccgtgagctggtaccagcagaagcccggccagagccccaagctgctgatcttcagcgccagctacaggtacaccggcgtgcccgacaggttcaccggcagcggcagcggcgccgacttcaccctgaccatcagcagcgtgcaggccgaggacctggccgtgtactactgccagcagcactacagcaccccctggaccttcggcggcggcaccaagctggacatcaagggaggggggggatccgggggaggaggctccggcggaggcggaagccagatccagctggtgcagagcggccccgacctgaagaagcccggcgagaccgtgaagctgagctgcaaggccagcggctacaccttcaccaacttcggcatgaactgggtgaagcaggcccccggcaagggcttcaagtggatggcctggatcaacacctacaccggcgagagctacttcgccgacgacttcaagggcaggttcgccttcagcgtggagaccagcgccaccaccgcctacctgcagatcaacaacctgaagaccgaggacaccgccacctacttctgcgccaggggcgagatctactacggctacgacggcggcttcgcctactggggccagggcaccctggtgaccgtgagcgccaccacgacgccagcgccgcgaccaccaacaccggcgcccaccatcgcgtcgcagcccctgtccctgcgcccagaggcgtgccggccagcggcggggggcgcagtgcacacgagggggctggacttcgcctgtgatatctacatctgggcgcccttggccgggacttgtggggtccttctcctgtcactggttatcaccctttactgcaggagtaagaggagcaggctcctgcacagtgactacatgaacatgactccccgccgccccgggcccacccgcaagcattaccagccctatgccccaccacgcgacttcgcagcctatcgctccagagtgaagttcagcaggagcgcagacgcccccgcgtaccagcagggccagaaccagctctataacgagctcaatctaggacgaagagaggagtacgatgttttggacaagagacgtggccgggaccctgagatggggggaaagccgcagagaaggaagaaccctcaggaaggcctgtacaatgaactgcagaaagataagatggcggaggcctacagtgagattgggatgaaaggcgagcgccggaggggcaaggggcacgatggcctttaccagggtctcagtacagccaccaaggacacctacgacgcccttcacatgcaggccctgccccctcgcggaagcggagccaccaacttcagcctgctgaagcaggccggcgacgtggaggagaaccccggccccatgtacagaatgcagctgctgagctgcatcgccctgagcctggccctggtgaccaacagctacttcggcaagctggagagcaagctgagcgtgatcaggaacctgaacgaccaggtgctgttcatcgaccagggcaacaggcccctgttcgaggacatgaccgacagcgactgcagggacaacgcccccaggaccatcttcatcatcagcatgtacaaggacagccagcccaggggcatggccgtgaccatcagcgtgaagtgcgagaagatcagcaccctgagctgcgagaacaagatcatcagcttcaaggagatgaacccccccgacaacatcaaggacaccaagagcgacatcatcttcttccagaggagcgtgcccggccacgacaacaagatgcagttcgagagcagcagctacgagggctacttcctggcctgcgagaaggagagggacctgttcaagctgatcctgaagaaggaggacgagctgggcgacaggagcatcatgttcaccgtgcagaacgaggac

SEQ ID NO: 13 - protein, 754 aa, Artificial Sequence
  Synthetic Sequence
MALPVTALLLPLALLLHAARPDVVMTQSHRFMSTSVGDRVSITCRASQDVNTAVSWYQQKPGQSPKLLIFSASYRYTGVPDRFTGSGSGADFTLTISSVQAEDLAVYYCQQHYSTPWTFGGGTKLDIKGGGGSGGGGSGGGGSQIQLVQSGPDLKKPGETVKLSCKASGYTFTNFGMNWVKQAPGKGFKWMAWINTYTGESYFADDFKGRFAFSVETSATTAYLQINNLKTEDTATYFCARGEIYYGYDGGFAYWGQGTLVTVSATTTPAPRPPTPAPTIASQPLSLRPEACRPAAGGAVHTRGLDFACDIYIWAPLAGTCGVLLLSLVITLYCRSKRSRLLHSDYMNMTPRRPGPTRKHYQPYAPPRDFAAYRSRVKFSRSADAPAYQQGQNQLYNELNLGRREEYDVLDKRRGRDPEMGGKPQRRKNPQEGLYNELQKDKMAEAYSEIGMKGERRRGKGHDGLYQGLSTATKDTYDALHMQALPPRGSGATNFSLLKQAGDVEENPGPMYRMQLLSCIALSLALVTNSYFGKLESKLSVIRNLNDQVLFIDQGNRPLFEDMTDSDCRDNAPRTIFIISMYKDSQPRGMAVTISVKCEKISTLSCENKIISFKEMNPPDNIKDTKSDIIFFQRSVPGHDNKMQFESSSYEGYFLACEKERDLFKLILKKEDELGDRSIMFTVQNEDTTTPAPRPPTPAPTIASQPLSLRPEACRPAAGGAVHTRGLDFACDVAISTSTVLLCGLSAVSLLACY

SEQ ID NO: 14 - DNA, 2273 bp, Artificial Sequence
  Synthetic Sequence
atggccttaccagtgaccgccttgctcctgccgctggccttgctgctccacgccgccaggccggacgtggtgatgacccagagccacaggttcatgagcaccagcgtgggcgacagggtgagcatcacctgcagggccagccaggacgtgaacaccgccgtgagctggtaccagcagaagcccggccagagccccaagctgctgatcttcagcgccagctacaggtacaccggcgtgcccgacaggttcaccggcagcggcagcggcgccgacttcaccctgaccatcagcagcgtgcaggccgaggacctggccgtgtactactgccagcagcactacagcaccccctggaccttcggcggcggcaccaagctggacatcaagggaggggggggatccgggggaggaggctccggcggaggcggaagccagatccagctggtgcagagcggccccgacctgaagaagcccggcgagaccgtgaagctgagctgcaaggccagcggctacaccttcaccaacttcggcatgaactgggtgaagcaggcccccggcaagggcttcaagtggatggcctggatcaacacctacaccggcgagagctacttcgccgacgacttcaagggcaggttcgccttcagcgtggagaccagcgccaccaccgcctacctgcagatcaacaacctgaagaccgaggacaccgccacctacttctgcgccaggggcgagatctactacggctacgacggcggcttcgcctactggggccagggcaccctggtgaccgtgagcgccaccacgacgccagcgccgcgaccaccaacaccggcgcccaccatcgcgtcgcagcccctgtccctgcgcccagaggcgtgccggccagcggcggggggcgcagtgcacacgagggggctggacttcgcctgtgatatctacatctgggcgcccttggccgggacttgtggggtccttctcctgtcactggttatcaccctttactgcaggagtaagaggagcaggctcctgcacagtgactacatgaacatgactccccgccgccccgggcccacccgcaagcattaccagccctatgccccaccacgcgacttcgcagcctatcgctccagagtgaagttcagcaggagcgcagacgcccccgcgtaccagcagggccagaaccagctctataacgagctcaatctaggacgaagagaggagtacgatgttttggacaagagacgtggccgggaccctgagatggggggaaagccgcagagaaggaagaaccctcaggaaggcctgtacaatgaactgcagaaagataagatggcggaggcctacagtgagattgggatgaaaggcgagcgccggaggggcaaggggcacgatggcctttaccagggtctcagtacagccaccaaggacacctacgacgcccttcacatgcaggccctgccccctcgcggaagcggagccaccaacttcagcctgctgaagcaggccggcgacgtggaggagaaccccggccccatgtacagaatgcagctgctgagctgcatcgccctgagcctggccctggtgaccaacagctacttcggcaagctggagagcaagctgagcgtgatcaggaacctgaacgaccaggtgctgttcatcgaccagggcaacaggcccctgttcgaggacatgaccgacagcgactgcagggacaacgcccccaggaccatcttcatcatcagcatgtacaaggacagccagcccaggggcatggccgtgaccatcagcgtgaagtgcgagaagatcagcaccctgagctgcgagaacaagatcatcagcttcaaggagatgaacccccccgacaacatcaaggacaccaagagcgacatcatcttcttccagaggagcgtgcccggccacgacaacaagatgcagttcgagagcagcagctacgagggctacttcctggcctgcgagaaggagagggacctgttcaagctgatcctgaagaaggaggacgagctgggcgacaggagcatcatgttcaccgtgcagaacgaggacaccaccacccccgcccccaggccccccacccccgcccccaccatcgccagccagcccctgagcctgaggcccgaggcctgcaggcccgccgccggcggcgccgtgcacaccaggggcctggacttcgcctgcgacgtggctatctccacgtccactgtcctgctgtgtgggctgagcgctgtgtctctcctggcatgctactaagtttaaac

SEQ ID NO: 15 - protein, 258 aa, Artificial Sequence
  Synthetic Sequence
VPRWRQQWSGPGTTKRFPETVLARCVKYTEIHPEMRHVDCQSVWDAFKGAFISKHPCNITEEDYQPLMKLGTQTVPCNKILLWSRIKDLAHQFTQVQRDMFTLEDTLLGYLADDLTWCGEFNTSKINYQSCPDWRKDCSNNPVSVFWKTVSRRFAEAACDVVHVMLNGSRSKIFDKNSTFGSVEVHNLQPEKVQTLEAWVIHGGREDSRDLCQDPTIKELESIISKRNIQFSCKNIYRPDKFLQCVKNPEDSSCTSEI

SEQ ID NO: 16 - protein, 667 aa, Artificial Sequence
  Synthetic Sequence
MALPVTALLLPLALLLHAARPEVQLQQSGPELIKPGASVKMSCKASGYTFTSYVMHWVKQKPGQGLEWIGYINPYNDGTKYNEKFKGKATLTSDKSSSTAYMELSSLTSEDSAVYYCARGTYYYGSRVFDYWGQGTTLTVSSGGGGSGGGGSGGGGSDIVMTQAAPSIPVTPGESVSISCRSSKSLLNSNGNTYLYWFLQRPGQSPQLLIYRMSNLASGVPDRFSGSGSGTAFTLRISRVEAEDVGVYYCMQHLEYPFTFGAGTKLELKRTTTPAPRPPTPAPTIASQPLSLRPEACRPAAGGAVHTRGLDFACDIYIWAPLAGTCGVLLLSLVITLYCRSKRSRLLHSDYMNMTPRRPGPTRKHYQPYAPPRDFAAYRSRVKFSRSADAPAYQQGQNQLYNELNLGRREEYDVLDKRRGRDPEMGGKPQRRKNPQEGLYNELQKDKMAEAYSEIGMKGERRRGKGHDGLYQGLSTATKDTYDALHMQALPPRGSGEGRGSLLTCGDVEENPGPMYRMQLLSCIALSLALVTNSQGQDRHMIRMRQLIDIVDQLKNYVNDLVPEFLPAPEDVETNCEWSAFSCFQKAQLKSANTGNNERIINVSIKKLKRKPPSTNAGRRQKHRLTCPSCDSYEKKPPKEFLERFKSLLQKMIHQHLSSRTHGSEDS

SEQ ID NO: 17 - DNA, 2012 bp, Artificial Sequence
  Synthetic Sequence
atggccttaccagtgaccgccttgctcctgccgctggccttgctgctccacgccgccaggccggaggtccagctgcagcagtctggacctgagctgataaagcctggggcttcagtgaagatgtcctgcaaggcttctggatacacattcactagctatgttatgcactgggtgaagcagaagcctgggcagggccttgagtggattggatatattaatccttacaatgatggtactaagtacaatgagaagttcaaaggcaaggccacactgacttcagacaaatcctccagcacagcctacatggagctcagcagcctgacctctgaggactctgcggtctattactgtgcaagagggacttattactacggtagtagggtatttgactactggggccaaggcaccactctcacagtctcctcaggtggagggggctcaggcggaggtggctctgggggtggaggctcggacattgtgatgactcaggctgcaccctctatacctgtcactcctggagagtcagtatccatctcctgcaggtctagtaagagtctcctgaatagtaatggcaacacttacttgtattggttcctgcagaggccaggccagtctcctcagctcctgatatatcggatgtccaaccttgcctcaggagtcccagacaggttcagtggcagtgggtcaggaactgctttcacactgagaatcagtagagtggaggctgaggatgtgggtgtttattactgtatgcaacatctagaatatccgttcacgttcggtgctgggaccaagctggagctgaaacggaccacgacgccagcgccgcgaccaccaacaccggcgcccaccatcgcgtcgcagcccctgtccctgcgcccagaggcgtgccggccagcggcggggggcgcagtgcacacgagggggctggacttcgcctgtgatatctacatctgggcgcccttggccgggacttgtggggtccttctcctgtcactggttatcaccctttactgcaggagtaagaggagcaggctcctgcacagtgactacatgaacatgactccccgccgccccgggcccacccgcaagcattaccagccctatgccccaccacgcgacttcgcagcctatcgctccagagtgaagttcagcaggagcgcagacgcccccgcgtaccagcagggccagaaccagctctataacgagctcaatctaggacgaagagaggagtacgatgttttggacaagagacgtggccgggaccctgagatggggggaaagccgcagagaaggaagaaccctcaggaaggcctgtacaatgaactgcagaaagataagatggcggaggcctacagtgagattgggatgaaaggcgagcgccggaggggcaaggggcacgatggcctttaccagggtctcagtacagccaccaaggacacctacgacgcccttcacatgcaggccctgccccctcgcggcagcggcgaaggccgcggcagcctgctgacctgcggcgatgtggaagaaaacccgggccccatgtacagaatgcagctgctgagctgcatcgccctgagcctggccctggtgaccaacagccagggccaggacaggcacatgatcaggatgaggcagctgatcgacatcgtggaccagctgaagaactacgtgaacgacctggtgcccgagttcctgcccgcccccgaggacgtggagaccaactgcgagtggagcgccttcagctgcttccagaaggcccagctgaagagcgccaacaccggcaacaacgagaggatcatcaacgtgagcatcaagaagctgaagaggaagccccccagcaccaacgccggcaggaggcagaagcacaggctgacctgccccagctgcgacagctacgagaagaagccccccaaggagttcctggagaggttcaagagcctgctgcagaagatgatccaccagcacctgagcagcaggacccacggcagcgaggacagctaagtttaaac

SEQ ID NO: 18 - protein, 1055 aa, Artificial Sequence
  Synthetic Sequence
DRMALPVTALLLPLALLLHAARPDIQMTQSPSSLSASVGDRVTITCSASSSVSYMNWYQQTPGKAPKRWIYDTSKLASGVPSRFSGSGSGTDYTFTISSLQPEDIATYYCQQWSSNPFTFGQGTKLQIGGGGSGGGGSGGGGSQVQLVQSGGGVVQPGRSLRLSCKASGYTFTRYTMHWVRQAPGKGLEWIGYINPSRGYTNYNQKVKDRFTISRDNSKNTAFLQMDSLRPEDTGVYFCARYYDDHYCLDYWGQGTPVTVSSTTTPAPRPPTPAPTIASQPLSLRPEACRPAAGGAVHTRGLDFACDIYIWAPLAGTCGVLLLSLVITLYCRSKRSRLLHSDYMNMTPRRPGPTRKHYQPYAPPRDFAAYRSRVKFSRSADAPAYQQGQNQLYNELNLGRREEYDVLDKRRGRDPEMGGKPQRRKNPQEGLYNELQKDKMAEAYSEIGMKGERRRGKGHDGLYQGLSTATKDTYDALHMQALPPRGSGEGRGSLLTCGDVEENPGPMEYASDASLDPEAPWPPAPRARACRVLPWALVAGLLLLLLLAAACAVFLACPWAVSGARASPGSAASPRLREGPELSPDDPAGLLDLRQGMFAQLVAQNVLLIDGPLSWYSDPGLAGVSLTGGLSYKEDTKELVVAKAGVYYVFFQLELRRVVAGEGSGSVSLALHLQPLRSAAGAAALALTVDLPPASSEARNSAFGFQGRLLHLSAGQRLGVHLHTEARARHAWQLTQGATVLGLFRVTPEIPAGLPSPRSEGSGATNFSLLKQAGDVEENPGPMYRMQLLSCIALSLALVTNSGIHVFILGCFSAGLPKTEANWVNVISDLKKIEDLIQSMHIDATLYTESDVHPSCKVTAMKCFLLELQVISLESGDASIHDTVENLIILANNSLSSNGNVTESGCKECEELEEKNIKEFLQSFVHIVQMFINTSSGGGSGGGGSGGGGSGGGGSGGGSLQAPRRARGCRTLGLPALLLLLLLRPPATRGITCPPPMSVEHADIWVKSYSLYSRERYICNSGFKRKAGTSSLTECVLNKATNVAHWTTPSLKCIR

SEQ ID NO: 19 - DNA, 3170 bp, Artificial Sequence
  Synthetic Sequence
atggccttaccagtgaccgccttgctcctgccgctggccttgctgctccacgccgccaggccggacatccagatgacccagagccccagcagcctgagcgccagcgtgggcgacagagtgaccatcacctgcagcgccagcagcagcgtgagctacatgaactggtaccagcagacccccggcaaggcccccaagagatggatctacgacaccagcaagctggccagcggcgtgcccagcagattcagcggcagcggcagcggcaccgactacaccttcaccatcagcagcctgcagcccgaggacatcgccacctactactgccagcagtggagcagcaaccccttcaccttcggccagggcaccaagctgcagatcggcggcggcggcagcggcggcggcggcagcggcggcggcggcagccaggtgcagctggtgcagagcggcggcggcgtggtgcagcccggcagaagcctgagactgagctgcaaggccagcggctacaccttcaccagatacaccatgcactgggtgagacaggcccccggcaagggcctggagtggatcggctacatcaaccccagcagaggctacaccaactacaaccagaaggtgaaggacagattcaccatcagcagagacaacagcaagaacaccgccttcctgcagatggacagcctgagacccgaggacaccggcgtgtacttctgcgccagatactacgacgaccactactgcctggactactggggccagggcacccccgtgaccgtgagcagcaccacgacgccagcgccgcgaccaccaacaccggcgcccaccatcgcgtcgcagcccctgtccctgcgcccagaggcgtgccggccagcggcggggggcgcagtgcacacgagggggctggacttcgcctgtgatatctacatctgggcgcccttggccgggacttgtggggtccttctcctgtcactggttatcaccctttactgcaggagtaagaggagcaggctcctgcacagtgactacatgaacatgactccccgccgccccgggcccacccgcaagcattaccagccctatgccccaccacgcgacttcgcagcctatcgctccagagtgaagttcagcaggagcgcagacgcccccgcgtaccagcagggccagaaccagctctataacgagctcaatctaggacgaagagaggagtacgatgttttggacaagagacgtggccgggaccctgagatggggggaaagccgcagagaaggaagaaccctcaggaaggcctgtacaatgaactgcagaaagataagatggcggaggcctacagtgagattgggatgaaaggcgagcgccggaggggcaaggggcacgatggcctttaccagggtctcagtacagccaccaaggacacctacgacgcccttcacatgcaggccctgccccctcgcggcagcggcgaaggccgcggcagcctgctgacctgcggcgatgtggaagaaaacccgggccccatggaatacgcctctgacgcttcactggaccccgaagccccgtggcctcccgcgccccgcgctcgcgcctgccgcgtactgccttgggccctggtcgcggggctgctgctgctgctgctgctcgctgccgcctgcgccgtcttcctcgcctgcccctgggccgtgtccggggctcgcgcctcgcccggctccgcggccagcccgagactccgcgagggtcccgagctttcgcccgacgatcccgccggcctcttggacctgcggcagggcatgtttgcgcagctggtggcccaaaatgttctgctgatcgatgggcccctgagctggtacagtgacccaggcctggcaggcgtgtccctgacggggggcctgagctacaaagaggacacgaaggagctggtggtggccaaggctggagtctactatgtcttctttcaactagagctgcggcgcgtggtggccggcgagggctcaggctccgtttcacttgcgctgcacctgcagccactgcgctctgctgctggggccgccgccctggctttgaccgtggacctgccacccgcctcctccgaggctcggaactcggccttcggtttccagggccgcttgctgcacctgagtgccggccagcgcctgggcgtccatcttcacactgaggccagggcacgccatgcctggcagcttacccagggcgccacagtcttgggactcttccgggtgacccccgaaatcccagccggactcccttcaccgaggtcggaaggaagcggagctactaacttcagcctgctgaagcaggctggagacgtggaggagaaccctggacctatgtacagaatgcagctgctgagctgcatcgccctgagcctggccctggtgaccaacagcggcatccacgtgttcatcctgggctgcttcagcgccggcctgcccaagaccgaggccaactgggtgaacgtgatcagcgacctgaagaagatcgaggacctgatccagagcatgcacatcgacgccaccctgtacaccgagagcgacgtgcaccccagctgcaaggtgaccgccatgaagtgcttcctgctggagctgcaggtgatcagcctggagagcggcgacgccagcatccacgacaccgtggagaacctgatcatcctggccaacaacagcctgagcagcaacggcaacgtgaccgagagcggctgcaaggagtgcgaggagctggaggagaagaacatcaaggagttcctgcagagcttcgtgcacatcgtgcagatgttcatcaacaccagctccggcggcggctccggcggcggcggctccggcggcggcggctccggcggcggcggctccggcggcggctccctgcaggcccccagaagagccagaggctgcagaaccctgggcctgcccgccctgctgctgctgctgctgctgagaccccccgccaccagaggcatcacctgccccccccccatgagcgtggagcacgccgacatctgggtgaagagctacagcctgtacagcagagagagatacatctgcaacagcggcttcaagagaaaggccggcaccagcagcctgaccgagtgcgtgctgaacaaggccaccaacgtggcccactggaccacccccagcctgaagtgcatcagataagtttaaac

SEQ ID NO: 20 - protein, 1066 aa, Artificial Sequence
  Synthetic Sequence
DRTMALPVTALLLPLALLLHAARPDIVMTQSPDSLAVSLGERVTMNCKSSQSLLYSTNQKNYLAWYQQKPGQSPKLLIYWASTRESGVPDRFSGSGSGTDFTLTISSVQAEDVAVYYCQQYYSYRTFGGGTKLEIKGGGGSGGGGSGGGGSQVQLQQSGPEVVKPGASVKMSCKASGYTFTSYVIHWVRQKPGQGLDWIGYINPYNDGTDYDEKFKGKATLTSDTSTSTAYMELSSLRSEDTAVYYCAREKDNYATGAWFAYWGQGTLVTVSSTTTPAPRPPTPAPTIASQPLSLRPEACRPAAGGAVHTRGLDFACDIYIWAPLAGTCGVLLLSLVITLYCRSKRSRLLHSDYMNMTPRRPGPTRKHYQPYAPPRDFAAYRSRVKFSRSADAPAYQQGQNQLYNELNLGRREEYDVLDKRRGRDPEMGGKPQRRKNPQEGLYNELQKDKMAEAYSEIGMKGERRRGKGHDGLYQGLSTATKDTYDALHMQALPPRGSGEGRGSLLTCGDVEENPGPMEYASDASLDPEAPWPPAPRARACRVLPWALVAGLLLLLLLAAACAVFLACPWAVSGARASPGSAASPRLREGPELSPDDPAGLLDLRQGMFAQLVAQNVLLIDGPLSWYSDPGLAGVSLTGGLSYKEDTKELVVAKAGVYYVFFQLELRRVVAGEGSGSVSLALHLQPLRSAAGAAALALTVDLPPASSEARNSAFGFQGRLLHLSAGQRLGVHLHTEARARHAWQLTQGATVLGLFRVTPEIPAGLPSPRSEGSGATNFSLLKQAGDVEENPGPMYRMQLLSCIALSLALVTNSGIHVFILGCFSAGLPKTEANWVNVISDLKKIEDLIQSMHIDATLYTESDVHPSCKVTAMKCFLLELQVISLESGDASIHDTVENLIILANNSLSSNGNVTESGCKECEELEEKNIKEFLQSFVHIVQMFINTSSGGGSGGGGSGGGGSGGGGSGGGSLQAPRRARGCRTLGLPALLLLLLLRPPATRGITCPPPMSVEHADIWVKSYSLYSRERYICNSGFKRKAGTSSLTECVLNKATNVAHWTTPSLKCIR

SEQ ID NO: 21 - DNA, 3200 bp, Artificial Sequence
  Synthetic Sequence
atggccctgcccgtgaccgccctgctgctgcccctggccctgctgctgcacgccgccaggcccgacatcgtgatgacccaaagccccgacagcctggccgtgagcctgggcgagagggtgaccatgaactgcaaaagcagccagtccctgctgtactccaccaaccagaagaactacctggcttggtatcaacagaagcccggacagagccccaagctgctgatctattgggccagcactagggaaagcggcgtgcccgataggttcagcggcagcgggagcggcacagacttcactctgaccattagcagcgtgcaggctgaggatgtggccgtctactactgccagcagtactacagctacaggacctttgggggcggaactaagctggagatcaagggaggggggggatccgggggaggaggctccggcggaggcggaagccaagtgcaactgcagcagagcggcccagaggtggtcaaacctggggcaagcgtgaagatgagctgcaaggctagcggctataccttcaccagctatgtgatccactgggtgaggcagaaaccaggacagggcctggactggatcggctacatcaacccctacaatgacggcaccgattatgacgaaaaattcaaggggaaggccaccctgaccagcgacaccagcacaagcaccgcctacatggagctgtccagcctgaggtccgaggacaccgccgtgtattactgtgccagggagaaggacaattacgccaccggcgcttggttcgcctactggggccagggcacactggtgacagtgagcagcaccacgacgccagcgccgcgaccaccaacaccggcgcccaccatcgcgtcgcagcccctgtccctgcgcccagaggcgtgccggccagcggcggggggcgcagtgcacacgagggggctggacttcgcctgtgatatctacatctgggcccccctggccggcacctgcggcgtgctgctgctgagcctggtgatcaccctgtactgcaggagtaagaggagcaggctcctgcacagtgactacatgaacatgactccccgccgccccgggcccacccgcaagcattaccagccctatgccccaccacgcgacttcgcagcctatcgctccagagtgaagttcagcaggagcgcagacgcccccgcgtaccagcagggccagaaccagctctataacgagctcaatctaggacgaagagaggagtacgatgttttggacaagagacgtggccgggaccctgagatggggggaaagccgcagagaaggaagaaccctcaggaaggcctgtacaatgaactgcagaaagataagatggcggaggcctacagtgagattgggatgaaaggcgagcgccggaggggcaaggggcacgatggcctttaccagggtctcagtacagccaccaaggacacctacgacgcccttcacatgcaggccctgccccctcgcggcagcggcgaaggccgcggcagcctgctgacctgcggcgatgtggaagaaaacccgggccccatggaatacgcctctgacgcttcactggaccccgaagccccgtggcctcccgcgccccgcgctcgcgcctgccgcgtactgccttgggccctggtcgcggggctgctgctgctgctgctgctcgctgccgcctgcgccgtcttcctcgcctgcccctgggccgtgtccggggctcgcgcctcgcccggctccgcggccagcccgagactccgcgagggtcccgagctttcgcccgacgatcccgccggcctcttggacctgcggcagggcatgtttgcgcagctggtggcccaaaatgttctgctgatcgatgggcccctgagctggtacagtgacccaggcctggcaggcgtgtccctgacggggggcctgagctacaaagaggacacgaaggagctggtggtggccaaggctggagtctactatgtcttctttcaactagagctgcggcgcgtggtggccggcgagggctcaggctccgtttcacttgcgctgcacctgcagccactgcgctctgctgctggggccgccgccctggctttgaccgtggacctgccacccgcctcctccgaggctcggaactcggccttcggtttccagggccgcttgctgcacctgagtgccggccagcgcctgggcgtccatcttcacactgaggccagggcacgccatgcctggcagcttacccagggcgccacagtcttgggactcttccgggtgacccccgaaatcccagccggactcccttcaccgaggtcggaaggaagcggagctactaacttcagcctgctgaagcaggctggagacgtggaggagaaccctggacctatgtacagaatgcagctgctgagctgcatcgccctgagcctggccctggtgaccaacagcggcatccacgtgttcatcctgggctgcttcagcgccggcctgcccaagaccgaggccaactgggtgaacgtgatcagcgacctgaagaagatcgaggacctgatccagagcatgcacatcgacgccaccctgtacaccgagagcgacgtgcaccccagctgcaaggtgaccgccatgaagtgcttcctgctggagctgcaggtgatcagcctggagagcggcgacgccagcatccacgacaccgtggagaacctgatcatcctggccaacaacagcctgagcagcaacggcaacgtgaccgagagcggctgcaaggagtgcgaggagctggaggagaagaacatcaaggagttcctgcagagcttcgtgcacatcgtgcagatgttcatcaacaccagctccggcggcggctccggcggcggcggctccggcggcggcggctccggcggcggcggctccggcggcggctccctgcaggcccccagaagagccagaggctgcagaaccctgggcctgcccgccctgctgctgctgctgctgctgagaccccccgccaccagaggcatcacctgccccccccccatgagcgtggagcacgccgacatctgggtgaagagctacagcctgtacagcagagagagatacatctgcaacagcggcttcaagagaaaggccggcaccagcagcctgaccgagtgcgtgctgaacaaggccaccaacgtggcccactggaccacccccagcctgaagtgcatcagataagtttaaac

SEQ ID NO: 22 - protein, 832 aa, Artificial Sequence
  Synthetic Sequence
DRMALPVTALLLPLALLLHAARPDIVMTQSPDSLAVSLGERVTMNCKSSQSLLYSTNQKNYLAWYQQKPGQSPKLLIYWASTRESGVPDRFSGSGSGTDFTLTISSVQAEDVAVYYCQQYYSYRTFGGGTKLEIKGGGGSGGGGSGGGGSQVQLQQSGPEVVKPGASVKMSCKASGYTFTSYVIHWVRQKPGQGLDWIGYINPYNDGTDYDEKFKGKATLTSDTSTSTAYMELSSLRSEDTAVYYCAREKDNYATGAWFAYWGQGTLVTVSSTTTPAPRPPTPAPTIASQPLSLRPEACRPAAGGAVHTRGLDFACDIYIWAPLAGTCGVLLLSLVITLYCRSKRSRLLHSDYMNMTPRRPGPTRKHYQPYAPPRDFAAYRSKRGRKKLLYIFKQPFMRPVQTTQEEDGCSCRFPEEEEGGCELRVKFSRSADAPAYQQGQNQLYNELNLGRREEYDVLDKRRGRDPEMGGKPQRRKNPQEGLYNELQKDKMAEAYSEIGMKGERRRGKGHDGLYQGLSTATKDTYDALHMQALPPRGSGATNFSLLKQAGDVEENPGPMYRMQLLSCIALSLALVTNSGIHVFILGCFSAGLPKTEANWVNVISDLKKIEDLIQSMHIDATLYTESDVHPSCKVTAMKCFLLELQVISLESGDASIHDTVENLIILANNSLSSNGNVTESGCKECEELEEKNIKEFLQSFVHIVQMFINTSSGGGSGGGGSGGGGSGGGGSGGGSLQAPRRARGCRTLGLPALLLLLLLRPPATRGITCPPPMSVEHADIWVKSYSLYSRERYICNSGFKRKAGTSSLTECVLNKATNVAHWTTPSLKCIR

SEQ ID NO: 23 - DNA, 2501 bp, Artificial Sequence
  Synthetic Sequence
atggccttaccagtgaccgccttgctcctgccgctggccttgctgctccacgccgccaggccggacatcgtgatgacccaaagccccgacagcctggccgtgagcctgggcgagagggtgaccatgaactgcaaaagcagccagtccctgctgtactccaccaaccagaagaactacctggcttggtatcaacagaagcccggacagagccccaagctgctgatctattgggccagcactagggaaagcggcgtgcccgataggttcagcggcagcgggagcggcacagacttcactctgaccattagcagcgtgcaggctgaggatgtggccgtctactactgccagcagtactacagctacaggacctttgggggcggaactaagctggagatcaagggaggggggggatccgggggaggaggctccggcggaggcggaagccaagtgcaactgcagcagagcggcccagaggtggtcaaacctggggcaagcgtgaagatgagctgcaaggctagcggctataccttcaccagctatgtgatccactgggtgaggcagaaaccaggacagggcctggactggatcggctacatcaacccctacaatgacggcaccgattatgacgaaaaattcaaggggaaggccaccctgaccagcgacaccagcacaagcaccgcctacatggagctgtccagcctgaggtccgaggacaccgccgtgtattactgtgccagggagaaggacaattacgccaccggcgcttggttcgcctactggggccagggcacactggtgacagtgagcagcaccacgacgccagcgccgcgaccaccaacaccggcgcccaccatcgcgtcgcagcccctgtccctgcgcccagaggcgtgccggccagcggcggggggcgcagtgcacacgagggggctggacttcgcctgtgatatctacatctgggcgcccttggccgggacttgtggggtccttctcctgtcactggttatcaccctttactgcaggagtaagaggagcaggctcctgcacagtgactacatgaacatgactccccgccgccccgggcccacccgcaagcattaccagccctatgccccaccacgcgacttcgcagcctatcgctccaaacggggcagaaagaaactcctgtatatattcaaacaaccatttatgagaccagtacaaactactcaagaggaagatggctgtagctgccgatttccagaagaagaagaaggaggatgtgaactgagagtgaagttcagcaggagcgcagacgcccccgcgtaccagcagggccagaaccagctctataacgagctcaatctaggacgaagagaggagtacgatgttttggacaagagacgtggccgggaccctgagatggggggaaagccgcagagaaggaagaaccctcaggaaggcctgtacaatgaactgcagaaagataagatggcggaggcctacagtgagattgggatgaaaggcgagcgccggaggggcaaggggcacgatggcctttaccagggtctcagtacagccaccaaggacacctacgacgcccttcacatgcaggccctgccccctcgcggaagcggagccaccaacttcagcctgctgaagcaggccggcgacgtggaggagaaccccggccccatgtacagaatgcagctgctgagctgcatcgccctgagcctggccctggtgaccaacagcggcatccacgtgttcatcctgggctgcttcagcgccggcctgcccaagaccgaggccaactgggtgaacgtgatcagcgacctgaagaagatcgaggacctgatccagagcatgcacatcgacgccaccctgtacaccgagagcgacgtgcaccccagctgcaaggtgaccgccatgaagtgcttcctgctggagctgcaggtgatcagcctggagagcggcgacgccagcatccacgacaccgtggagaacctgatcatcctggccaacaacagcctgagcagcaacggcaacgtgaccgagagcggctgcaaggagtgcgaggagctggaggagaagaacatcaaggagttcctgcagagcttcgtgcacatcgtgcagatgttcatcaacaccagctccggcggcggctccggcggcggcggctccggcggcggcggctccggcggcggcggctccggcggcggctccctgcaggcccccagaagagccagaggctgcagaaccctgggcctgcccgccctgctgctgctgctgctgctgagaccccccgccaccagaggcatcacctgccccccccccatgagcgtggagcacgccgacatctgggtgaagagctacagcctgtacagcagagagagatacatctgcaacagcggcttcaagagaaaggccggcaccagcagcctgaccgagtgcgtgctgaacaaggccaccaacgtggcccactggaccacccccagcctgaagtgcatcagataagtttaaac

SEQ ID NO: 24 - protein, 789 aa, Artificial Sequence
  Synthetic Sequence
DRMALPVTALLLPLALLLHAARPEVQLQQSGPELIKPGASVKMSCKASGYTFTSYVMHWVKQKPGQGLEWIGYINPYNDGTKYNEKFKGKATLTSDKSSSTAYMELSSLTSEDSAVYYCARGTYYYGSRVFDYWGQGTTLTVSSGGGGSGGGGSGGGGSDIVMTQAAPSIPVTPGESVSISCRSSKSLLNSNGNTYLYWFLQRPGQSPQLLIYRMSNLASGVPDRFSGSGSGTAFTLRISRVEAEDVGVYYCMQHLEYPFTFGAGTKLELKRTTTPAPRPPTPAPTIASQPLSLRPEACRPAAGGAVHTRGLDFACDIYIWAPLAGTCGVLLLSLVITLYCRSKRSRLLHSDYMNMTPRRPGPTRKHYQPYAPPRDFAAYRSRVKFSRSADAPAYQQGQNQLYNELNLGRREEYDVLDKRRGRDPEMGGKPQRRKNPQEGLYNELQKDKMAEAYSEIGMKGERRRGKGHDGLYQGLSTATKDTYDALHMQALPPRGSGEGRGSLLTCGDVEENPGPMYRMQLLSCIALSLALVTNSGIHVFILGCFSAGLPKTEANWVNVISDLKKIEDLIQSMHIDATLYTESDVHPSCKVTAMKCFLLELQVISLESGDASIHDTVENLIILANNSLSSNGNVTESGCKECEELEEKNIKEFLQSFVHIVQMFINTSSGGGSGGGGSGGGGSGGGGSGGGSLQAPRRARGCRTLGLPALLLLLLLRPPATRGITCPPPMSVEHADIWVKSYSLYSRERYICNSGFKRKAGTSSLTECVLNKATNVAHWTTPSLKCIR

SEQ ID NO: 25 - DNA, 2372 bp, Artificial Sequence
  Synthetic Sequence
atggccttaccagtgaccgccttgctcctgccgctggccttgctgctccacgccgccaggccggaggtccagctgcagcagtctggacctgagctgataaagcctggggcttcagtgaagatgtcctgcaaggcttctggatacacattcactagctatgttatgcactgggtgaagcagaagcctgggcagggccttgagtggattggatatattaatccttacaatgatggtactaagtacaatgagaagttcaaaggcaaggccacactgacttcagacaaatcctccagcacagcctacatggagctcagcagcctgacctctgaggactctgcggtctattactgtgcaagagggacttattactacggtagtagggtatttgactactggggccaaggcaccactctcacagtctcctcaggtggagggggctcaggcggaggtggctctgggggtggaggctcggacattgtgatgactcaggctgcaccctctatacctgtcactcctggagagtcagtatccatctcctgcaggtctagtaagagtctcctgaatagtaatggcaacacttacttgtattggttcctgcagaggccaggccagtctcctcagctcctgatatatcggatgtccaaccttgcctcaggagtcccagacaggttcagtggcagtgggtcaggaactgctttcacactgagaatcagtagagtggaggctgaggatgtgggtgtttattactgtatgcaacatctagaatatccgttcacgttcggtgctgggaccaagctggagctgaaacggaccacgacgccagcgccgcgaccaccaacaccggcgcccaccatcgcgtcgcagcccctgtccctgcgcccagaggcgtgccggccagcggcggggggcgcagtgcacacgagggggctggacttcgcctgtgatatctacatctgggcgcccttggccgggacttgtggggtccttctcctgtcactggttatcaccctttactgcaggagtaagaggagcaggctcctgcacagtgactacatgaacatgactccccgccgccccgggcccacccgcaagcattaccagccctatgccccaccacgcgacttcgcagcctatcgctccagagtgaagttcagcaggagcgcagacgcccccgcgtaccagcagggccagaaccagctctataacgagctcaatctaggacgaagagaggagtacgatgttttggacaagagacgtggccgggaccctgagatggggggaaagccgcagagaaggaagaaccctcaggaaggcctgtacaatgaactgcagaaagataagatggcggaggcctacagtgagattgggatgaaaggcgagcgccggaggggcaaggggcacgatggcctttaccagggtctcagtacagccaccaaggacacctacgacgcccttcacatgcaggccctgccccctcgcggcagcggcgaaggccgcggcagcctgctgacctgcggcgatgtggaagaaaacccgggccccatgtacagaatgcagctgctgagctgcatcgccctgagcctggccctggtgaccaacagcggcatccacgtgttcatcctgggctgcttcagcgccggcctgcccaagaccgaggccaactgggtgaacgtgatcagcgacctgaagaagatcgaggacctgatccagagcatgcacatcgacgccaccctgtacaccgagagcgacgtgcaccccagctgcaaggtgaccgccatgaagtgcttcctgctggagctgcaggtgatcagcctggagagcggcgacgccagcatccacgacaccgtggagaacctgatcatcctggccaacaacagcctgagcagcaacggcaacgtgaccgagagcggctgcaaggagtgcgaggagctggaggagaagaacatcaaggagttcctgcagagcttcgtgcacatcgtgcagatgttcatcaacaccagctccggcggcggctccggcggcggcggctccggcggcggcggctccggcggcggcggctccggcggcggctccctgcaggcccccagaagagccagaggctgcagaaccctgggcctgcccgccctgctgctgctgctgctgctgagaccccccgccaccagaggcatcacctgccccccccccatgagcgtggagcacgccgacatctgggtgaagagctacagcctgtacagcagagagagatacatctgcaacagcggcttcaagagaaaggccggcaccagcagcctgaccgagtgcgtgctgaacaaggccaccaacgtggcccactggaccacccccagcctgaagtgcatcagataagtttaaac

SEQ ID NO: 26 - protein, 1066 aa, Artificial Sequence
  Synthetic Sequence
DRTMALPVTALLLPLALLLHAARPEVQLQQSGPELIKPGASVKMSCKASGYTFTSYVMHWVKQKPGQGLEWIGYINPYNDGTKYNEKFKGKATLTSDKSSSTAYMELSSLTSEDSAVYYCARGTYYYGSRVFDYWGQGTTLTVSSGGGGSGGGGSGGGGSDIVMTQAAPSIPVTPGESVSISCRSSKSLLNSNGNTYLYWFLQRPGQSPQLLIYRMSNLASGVPDRFSGSGSGTAFTLRISRVEAEDVGVYYCMQHLEYPFTFGAGTKLELKRTTTPAPRPPTPAPTIASQPLSLRPEACRPAAGGAVHTRGLDFACDIYIWAPLAGTCGVLLLSLVITLYCRSKRSRLLHSDYMNMTPRRPGPTRKHYQPYAPPRDFAAYRSRVKFSRSADAPAYQQGQNQLYNELNLGRREEYDVLDKRRGRDPEMGGKPQRRKNPQEGLYNELQKDKMAEAYSEIGMKGERRRGKGHDGLYQGLSTATKDTYDALHMQALPPRGSGEGRGSLLTCGDVEENPGPMEYASDASLDPEAPWPPAPRARACRVLPWALVAGLLLLLLLAAACAVFLACPWAVSGARASPGSAASPRLREGPELSPDDPAGLLDLRQGMFAQLVAQNVLLIDGPLSWYSDPGLAGVSLTGGLSYKEDTKELVVAKAGVYYVFFQLELRRVVAGEGSGSVSLALHLQPLRSAAGAAALALTVDLPPASSEARNSAFGFQGRLLHLSAGQRLGVHLHTEARARHAWQLTQGATVLGLFRVTPEIPAGLPSPRSEGSGATNFSLLKQAGDVEENPGPMYRMQLLSCIALSLALVTNSGIHVFILGCFSAGLPKTEANWVNVISDLKKIEDLIQSMHIDATLYTESDVHPSCKVTAMKCFLLELQVISLESGDASIHDTVENLIILANNSLSSNGNVTESGCKECEELEEKNIKEFLQSFVHIVQMFINTSSGGGSGGGGSGGGGSGGGGSGGGSLQAPRRARGCRTLGLPALLLLLLLRPPATRGITCPPPMSVEHADIWVKSYSLYSRERYICNSGFKRKAGTSSLTECVLNKATNVAHWTTPSLKCIR

SEQ ID NO: 27 - DNA, 3200 bp, Artificial Sequence
  Synthetic Sequence
atggccttaccagtgaccgccttgctcctgccgctggccttgctgctccacgccgccaggccggaggtccagctgcagcagtctggacctgagctgataaagcctggggcttcagtgaagatgtcctgcaaggcttctggatacacattcactagctatgttatgcactgggtgaagcagaagcctgggcagggccttgagtggattggatatattaatccttacaatgatggtactaagtacaatgagaagttcaaaggcaaggccacactgacttcagacaaatcctccagcacagcctacatggagctcagcagcctgacctctgaggactctgcggtctattactgtgcaagagggacttattactacggtagtagggtatttgactactggggccaaggcaccactctcacagtctcctcaggtggagggggctcaggcggaggtggctctgggggtggaggctcggacattgtgatgactcaggctgcaccctctatacctgtcactcctggagagtcagtatccatctcctgcaggtctagtaagagtctcctgaatagtaatggcaacacttacttgtattggttcctgcagaggccaggccagtctcctcagctcctgatatatcggatgtccaaccttgcctcaggagtcccagacaggttcagtggcagtgggtcaggaactgctttcacactgagaatcagtagagtggaggctgaggatgtgggtgtttattactgtatgcaacatctagaatatccgttcacgttcggtgctgggaccaagctggagctgaaacggaccacgacgccagcgccgcgaccaccaacaccggcgcccaccatcgcgtcgcagcccctgtccctgcgcccagaggcgtgccggccagcggcggggggcgcagtgcacacgagggggctggacttcgcctgtgatatctacatctgggcgcccttggccgggacttgtggggtccttctcctgtcactggttatcaccctttactgcaggagtaagaggagcaggctcctgcacagtgactacatgaacatgactccccgccgccccgggcccacccgcaagcattaccagccctatgccccaccacgcgacttcgcagcctatcgctccagagtgaagttcagcaggagcgcagacgcccccgcgtaccagcagggccagaaccagctctataacgagctcaatctaggacgaagagaggagtacgatgttttggacaagagacgtggccgggaccctgagatggggggaaagccgcagagaaggaagaaccctcaggaaggcctgtacaatgaactgcagaaagataagatggcggaggcctacagtgagattgggatgaaaggcgagcgccggaggggcaaggggcacgatggcctttaccagggtctcagtacagccaccaaggacacctacgacgcccttcacatgcaggccctgccccctcgcggcagcggcgaaggccgcggcagcctgctgacctgcggcgatgtggaagaaaacccgggccccatggaatacgcctctgacgcttcactggaccccgaagccccgtggcctcccgcgccccgcgctcgcgcctgccgcgtactgccttgggccctggtcgcggggctgctgctgctgctgctgctcgctgccgcctgcgccgtcttcctcgcctgcccctgggccgtgtccggggctcgcgcctcgcccggctccgcggccagcccgagactccgcgagggtcccgagctttcgcccgacgatcccgccggcctcttggacctgcggcagggcatgtttgcgcagctggtggcccaaaatgttctgctgatcgatgggcccctgagctggtacagtgacccaggcctggcaggcgtgtccctgacggggggcctgagctacaaagaggacacgaaggagctggtggtggccaaggctggagtctactatgtcttctttcaactagagctgcggcgcgtggtggccggcgagggctcaggctccgtttcacttgcgctgcacctgcagccactgcgctctgctgctggggccgccgccctggctttgaccgtggacctgccacccgcctcctccgaggctcggaactcggccttcggtttccagggccgcttgctgcacctgagtgccggccagcgcctgggcgtccatcttcacactgaggccagggcacgccatgcctggcagcttacccagggcgccacagtcttgggactcttccgggtgacccccgaaatcccagccggactcccttcaccgaggtcggaaggaagcggagctactaacttcagcctgctgaagcaggctggagacgtggaggagaaccctggacctatgtacagaatgcagctgctgagctgcatcgccctgagcctggccctggtgaccaacagcggcatccacgtgttcatcctgggctgcttcagcgccggcctgcccaagaccgaggccaactgggtgaacgtgatcagcgacctgaagaagatcgaggacctgatccagagcatgcacatcgacgccaccctgtacaccgagagcgacgtgcaccccagctgcaaggtgaccgccatgaagtgcttcctgctggagctgcaggtgatcagcctggagagcggcgacgccagcatccacgacaccgtggagaacctgatcatcctggccaacaacagcctgagcagcaacggcaacgtgaccgagagcggctgcaaggagtgcgaggagctggaggagaagaacatcaaggagttcctgcagagcttcgtgcacatcgtgcagatgttcatcaacaccagctccggcggcggctccggcggcggcggctccggcggcggcggctccggcggcggcggctccggcggcggctccctgcaggcccccagaagagccagaggctgcagaaccctgggcctgcccgccctgctgctgctgctgctgctgagaccccccgccaccagaggcatcacctgccccccccccatgagcgtggagcacgccgacatctgggtgaagagctacagcctgtacagcagagagagatacatctgcaacagcggcttcaagagaaaggccggcaccagcagcctgaccgagtgcgtgctgaacaaggccaccaacgtggcccactggaccacccccagcctgaagtgcatcagataagtttaaac

SEQ ID NO: 28 - protein, 1300 aa, Artificial Sequence
  Synthetic Sequence
DRTMALPVTALLLPLALLLHAARPDIQLTQSPSSLSASVGDRVTMTCRASSSVSYIHWFQQKPGKAPKPWIYATSNLASGVPVRFSGSGSGTDYTFTISSLQPEDIATYYCQQWTSNPPTFGGGTKLEIKRGGGGSGGGGSGGGGSQVQLQQSGAEVKKPGSSVKVSCKASGYTFSSYNMHWVRQAPGQGLEWMGAIYPGNGDTSYNQKFKGRATITADESTNTAYMELSSLRSEDTAFYFCARSTYYGGDWYFDVWGQGTTVTVSSTTTPAPRPPTPAPTIASQPLSLRPEACRPAAGGAVHTRGLDFACDIYIWAPLAGTCGVLLLSLVITLYCRSKRSRLLHSDYMNMTPRRPGPTRKHYQPYAPPRDFAAYRSRVKFSRSADAPAYQQGQNQLYNELNLGRREEYDVLDKRRGRDPEMGGKPQRRKNPQEGLYNELQKDKMAEAYSEIGMKGERRRGKGHDGLYQGLSTATKDTYDALHMQALPPRGSGATNFSLLKQAGDVEENPGPMALPVTALLLPLALLLHAARPEVQLQQSGPELIKPGASVKMSCKASGYTFTSYVMHWVKQKPGQGLEWIGYINPYNDGTKYNEKFKGKATLTSDKSSSTAYMELSSLTSEDSAVYYCARGTYYYGSRVFDYWGQGTTLTVSSGGGGSGGGGSGGGGSDIVMTQAAPSIPVTPGESVSISCRSSKSLLNSNGNTYLYWFLQRPGQSPQLLIYRMSNLASGVPDRFSGSGSGTAFTLRISRVEAEDVGVYYCMQHLEYPFTFGAGTKLELKRTTTPAPRPPTPAPTIASQPLSLRPEACRPAAGGAVHTRGLDFACDIYIWAPLAGTCGVLLLSLVITLYCKRGRKKLLYIFKQPFMRPVQTTQEEDGCSCRFPEEEEGGCELRVKFSRSADAPAYQQGQNQLYNELNLGRREEYDVLDKRRGRDPEMGGKPQRRKNPQEGLYNELQKDKMAEAYSEIGMKGERRRGKGHDGLYQGLSTATKDTYDALHMQALPPRGSGEGRGSLLTCGDVEENPGPMYRMQLLSCIALSLALVTNSGIHVFILGCFSAGLPKTEANWVNVISDLKKIEDLIQSMHIDATLYTESDVHPSCKVTAMKCFLLELQVISLESGDASIHDTVENLIILANNSLSSNGNVTESGCKECEELEEKNIKEFLQSFVHIVQMFINTSSGGGSGGGGSGGGGSGGGGSGGGSLQAPRRARGCRTLGLPALLLLLLLRPPATRGITCPPPMSVEHADIWVKSYSLYSRERYICNSGFKRKAGTSSLTECVLNKATNVAHWTTPSLKCIR

SEQ ID NO: 29 - DNA, 3902 bp, Artificial Sequence
  Synthetic Sequence
atggccttaccagtgaccgccttgctcctgccgctggccttgctgctccacgccgccaggccggacatccagctgacccagagccccagcagcctgagcgccagcgtgggcgacagggtgaccatgacctgcagggccagcagcagcgtgagctacatccactggttccagcagaagcccggcaaggcccccaagccctggatctacgccaccagcaacctggccagcggcgtgcccgtgaggttcagcggcagcggcagcggcaccgactacaccttcaccatcagcagcctgcagcccgaggacatcgccacctactactgccagcagtggaccagcaacccccccaccttcggcggcggcaccaagctggagatcaagaggggcggcggcggcagcggcggcggcggcagcggcggcggcggcagccaggtgcagctgcagcagagcggcgccgaggtgaagaagcccggcagcagcgtgaaggtgagctgcaaggccagcggctacaccttcagcagctacaacatgcactgggtgaggcaggcccccggccagggcctggagtggatgggcgccatctaccccggcaacggcgacaccagctacaaccagaagttcaagggcagggccaccatcaccgccgacgagagcaccaacaccgcctacatggagctgagcagcctgaggagcgaggacaccgccttctacttctgcgccaggagcacctactacggcggcgactggtacttcgacgtgtggggccagggcaccaccgtgaccgtgagcagcaccacgacgccagcgccgcgaccaccaacaccggcgcccaccatcgcgtcgcagcccctgtccctgcgcccagaggcgtgccggccagcggcggggggcgcagtgcacacgagggggctggacttcgcctgtgatatctacatctgggcgcccttggccgggacttgtggggtccttctcctgtcactggttatcaccctttactgcaggagtaagaggagcaggctcctgcacagtgactacatgaacatgactccccgccgccccgggcccacccgcaagcattaccagccctatgccccaccacgcgacttcgcagcctatcgctccagagtgaagttcagcaggagcgcagacgcccccgcgtaccagcagggccagaaccagctctataacgagctcaatctaggacgaagagaggagtacgatgttttggacaagagacgtggccgggaccctgagatggggggaaagccgcagagaaggaagaaccctcaggaaggcctgtacaatgaactgcagaaagataagatggcggaggcctacagtgagattgggatgaaaggcgagcgccggaggggcaaggggcacgatggcctttaccagggtctcagtacagccaccaaggacacctacgacgcccttcacatgcaggccctgccccctcgcggaagcggagccaccaacttcagcctgctgaagcaggccggcgacgtggaggagaaccccggccccatggccctgcccgtgaccgccctgctgctgcccctggccctgctgctgcacgccgccaggcccgaggtccagctgcagcagtctggacctgagctgataaagcctggggcttcagtgaagatgtcctgcaaggcttctggatacacattcactagctatgttatgcactgggtgaagcagaagcctgggcagggccttgagtggattggatatattaatccttacaatgatggtactaagtacaatgagaagttcaaaggcaaggccacactgacttcagacaaatcctccagcacagcctacatggagctcagcagcctgacctctgaggactctgcggtctattactgtgcaagagggacttattactacggtagtagggtatttgactactggggccaaggcaccactctcacagtctcctcaggtggagggggctcaggcggaggtggctctgggggtggaggctcggacattgtgatgactcaggctgcaccctctatacctgtcactcctggagagtcagtatccatctcctgcaggtctagtaagagtctcctgaatagtaatggcaacacttacttgtattggttcctgcagaggccaggccagtctcctcagctcctgatatatcggatgtccaaccttgcctcaggagtcccagacaggttcagtggcagtgggtcaggaactgctttcacactgagaatcagtagagtggaggctgaggatgtgggtgtttattactgtatgcaacatctagaatatccgttcacgttcggtgctgggaccaagctggagctgaaacggaccaccacccccgcccccaggccccccacccccgcccccaccatcgccagccagcccctgagcctgaggcccgaggcctgcaggcccgccgccggcggcgccgtgcacaccaggggcctggacttcgcctgcgacatctacatctgggcccccctggccggcacctgcggcgtgctgctgctgagcctggtgatcaccctgtactgcaaacggggcagaaagaaactcctgtatatattcaaacaaccatttatgagaccagtacaaactactcaagaggaagatggctgtagctgccgatttccagaagaagaagaaggaggatgtgaactgagggtgaagttcagcaggagcgccgacgcccccgcctaccagcagggccagaaccagctgtacaacgagctgaacctgggcaggagggaggagtacgacgtgctggacaagaggaggggcagggaccccgagatgggcggcaagccccagaggaggaagaacccccaggagggcctgtacaacgagctgcagaaggacaagatggccgaggcctacagcgagatcggcatgaagggcgagaggaggaggggcaagggccacgacggcctgtaccagggcctgagcaccgccaccaaggacacctacgacgccctgcacatgcaggccctgccccccaggggcagcggcgaaggccgcggcagcctgctgacctgcggcgatgtggaagaaaacccgggccccatgtacagaatgcagctgctgagctgcatcgccctgagcctggccctggtgaccaacagcggcatccacgtgttcatcctgggctgcttcagcgccggcctgcccaagaccgaggccaactgggtgaacgtgatcagcgacctgaagaagatcgaggacctgatccagagcatgcacatcgacgccaccctgtacaccgagagcgacgtgcaccccagctgcaaggtgaccgccatgaagtgcttcctgctggagctgcaggtgatcagcctggagagcggcgacgccagcatccacgacaccgtggagaacctgatcatcctggccaacaacagcctgagcagcaacggcaacgtgaccgagagcggctgcaaggagtgcgaggagctggaggagaagaacatcaaggagttcctgcagagcttcgtgcacatcgtgcagatgttcatcaacaccagctccggcggcggctccggcggcggcggctccggcggcggcggctccggcggcggcggctccggcggcggctccctgcaggcccccagaagagccagaggctgcagaaccctgggcctgcccgccctgctgctgctgctgctgctgagaccccccgccaccagaggcatcacctgccccccccccatgagcgtggagcacgccgacatctgggtgaagagctacagcctgtacagcagagagagatacatctgcaacagcggcttcaagagaaaggccggcaccagcagcctgaccgagtgcgtgctgaacaaggccaccaacgtggcccactggaccacccccagcctgaagtgcatcagataagtttaaac

SEQ ID NO: 30 - protein, 1069 aa, Artificial Sequence
  Synthetic Sequence
DRTMALPVTALLLPLALLLHAARPMADYKDIVMTQSHKFLLVSVGDRVSITCKASQDVSTAVAWYQQKPGQSPKLLIYSASYRYTGVPDRFIGSGSGTDFTLTISSVQAEDLADYFCQQHYSTPLTFGAGTKLEIKRGGGGSGGGGSGGGGSSGGGSEVQLKESGPGLVAPSQSLSITCTVSGFPLTSYGVSWVRQPPGKGLEWLGVIWGDGSTNYHSALISRLSISKDNSKSQVFLKLNNLQTDDTATYYCARDTYYPYYAMDYWGQGTSVTVSSTTTPAPRPPTPAPTIASQPLSLRPEACRPAAGGAVHTRGLDFACDIYIWAPLAGTCGVLLLSLVITLYCRSKRSRLLHSDYMNMTPRRPGPTRKHYQPYAPPRDFAAYRSRVKFSRSADAPAYQQGQNQLYNELNLGRREEYDVLDKRRGRDPEMGGKPQRRKNPQEGLYNELQKDKMAEAYSEIGMKGERRRGKGHDGLYQGLSTATKDTYDALHMQALPPRGSGEGRGSLLTCGDVEENPGPMEYASDASLDPEAPWPPAPRARACRVLPWALVAGLLLLLLLAAACAVFLACPWAVSGARASPGSAASPRLREGPELSPDDPAGLLDLRQGMFAQLVAQNVLLIDGPLSWYSDPGLAGVSLTGGLSYKEDTKELVVAKAGVYYVFFQLELRRVVAGEGSGSVSLALHLQPLRSAAGAAALALTVDLPPASSEARNSAFGFQGRLLHLSAGQRLGVHLHTEARARHAWQLTQGATVLGLFRVTPEIPAGLPSPRSEGSGATNFSLLKQAGDVEENPGPMYRMQLLSCIALSLALVTNSGIHVFILGCFSAGLPKTEANWVNVISDLKKIEDLIQSMHIDATLYTESDVHPSCKVTAMKCFLLELQVISLESGDASIHDTVENLIILANNSLSSNGNVTESGCKECEELEEKNIKEFLQSFVHIVQMFINTSSGGGSGGGGSGGGGSGGGGSGGGSLQAPRRARGCRTLGLPALLLLLLLRPPATRGITCPPPMSVEHADIWVKSYSLYSRERYICNSGFKRKAGTSSLTECVLNKATNVAHWTTPSLKCIR

SEQ ID NO: 31 - DNA, 3209 bp, Artificial Sequence
  Synthetic Sequence
atggccctgcccgtgaccgccctgctgctgcccctggccctgctgctgcacgccgccaggcccatggccgactacaaggacatcgtgatgacccagagccacaagttcctgctggtgagcgtgggcgacagggtgagcatcacctgcaaggccagccaggacgtgagcaccgccgtggcctggtaccagcagaagcccggccagagccccaagctgctgatctacagcgccagctacaggtacaccggcgtgcccgacaggttcatcggcagcggcagcggcaccgacttcaccctgaccatcagcagcgtgcaggccgaggacctggccgactacttctgccagcagcactacagcacccccctgaccttcggcgccggcaccaagctggagatcaagaggggcggcggcggcagcggcggcggcggcagcggcggcggcggcagcagcggcggcggcagcgaggtgcagctgaaggagagcggccccggcctggtggcccccagccagagcctgagcatcacctgcaccgtgagcggcttccccctgaccagctacggcgtgagctgggtgaggcagccccccggcaagggcctggagtggctgggcgtgatctggggcgacggcagcaccaactaccacagcgccctgatcagcaggctgagcatcagcaaggacaacagcaagagccaggtgttcctgaagctgaacaacctgcagaccgacgacaccgccacctactactgcgccagggacacctactacccctactacgccatggactactggggccagggcaccagcgtgaccgtgagcagcaccaccacccccgcccccaggccccccacccccgcccccaccatcgccagccagcccctgagcctgaggcccgaggcctgcaggcccgccgccggcggcgccgtgcacaccaggggcctggacttcgcctgcgacatctacatctgggcccccctggccggcacctgcggcgtgctgctgctgagcctggtgatcaccctgtactgcaggagtaagaggagcaggctcctgcacagtgactacatgaacatgactccccgccgccccgggcccacccgcaagcattaccagccctatgccccaccacgcgacttcgcagcctatcgctccagagtgaagttcagcaggagcgcagacgcccccgcgtaccagcagggccagaaccagctctataacgagctcaatctaggacgaagagaggagtacgatgttttggacaagagacgtggccgggaccctgagatggggggaaagccgcagagaaggaagaaccctcaggaaggcctgtacaatgaactgcagaaagataagatggcggaggcctacagtgagattgggatgaaaggcgagcgccggaggggcaaggggcacgatggcctttaccagggtctcagtacagccaccaaggacacctacgacgcccttcacatgcaggccctgccccctcgcggcagcggcgaaggccgcggcagcctgctgacctgcggcgatgtggaagaaaacccgggccccatggaatacgcctctgacgcttcactggaccccgaagccccgtggcctcccgcgccccgcgctcgcgcctgccgcgtactgccttgggccctggtcgcggggctgctgctgctgctgctgctcgctgccgcctgcgccgtcttcctcgcctgcccctgggccgtgtccggggctcgcgcctcgcccggctccgcggccagcccgagactccgcgagggtcccgagctttcgcccgacgatcccgccggcctcttggacctgcggcagggcatgtttgcgcagctggtggcccaaaatgttctgctgatcgatgggcccctgagctggtacagtgacccaggcctggcaggcgtgtccctgacggggggcctgagctacaaagaggacacgaaggagctggtggtggccaaggctggagtctactatgtcttctttcaactagagctgcggcgcgtggtggccggcgagggctcaggctccgtttcacttgcgctgcacctgcagccactgcgctctgctgctggggccgccgccctggctttgaccgtggacctgccacccgcctcctccgaggctcggaactcggccttcggtttccagggccgcttgctgcacctgagtgccggccagcgcctgggcgtccatcttcacactgaggccagggcacgccatgcctggcagcttacccagggcgccacagtcttgggactcttccgggtgacccccgaaatcccagccggactcccttcaccgaggtcggaaggaagcggagctactaacttcagcctgctgaagcaggctggagacgtggaggagaaccctggacctatgtacagaatgcagctgctgagctgcatcgccctgagcctggccctggtgaccaacagcggcatccacgtgttcatcctgggctgcttcagcgccggcctgcccaagaccgaggccaactgggtgaacgtgatcagcgacctgaagaagatcgaggacctgatccagagcatgcacatcgacgccaccctgtacaccgagagcgacgtgcaccccagctgcaaggtgaccgccatgaagtgcttcctgctggagctgcaggtgatcagcctggagagcggcgacgccagcatccacgacaccgtggagaacctgatcatcctggccaacaacagcctgagcagcaacggcaacgtgaccgagagcggctgcaaggagtgcgaggagctggaggagaagaacatcaaggagttcctgcagagcttcgtgcacatcgtgcagatgttcatcaacaccagctccggcggcggctccggcggcggcggctccggcggcggcggctccggcggcggcggctccggcggcggctccctgcaggcccccagaagagccagaggctgcagaaccctgggcctgcccgccctgctgctgctgctgctgctgagaccccccgccaccagaggcatcacctgccccccccccatgagcgtggagcacgccgacatctgggtgaagagctacagcctgtacagcagagagagatacatctgcaacagcggcttcaagagaaaggccggcaccagcagcctgaccgagtgcgtgctgaacaaggccaccaacgtggcccactggaccacccccagcctgaagtgcatcagataagtttaaac

SEQ ID NO: 32 - protein, 1081 aa, Artificial Sequence
  Synthetic Sequence
DRTMALPVTALLLPLALLLHAARPMADYKDIVMTQSHKFMSTSVGDRVNITCKASQNVDSAVAWYQQKPGQSPKALIYSASYRYSGVPDRFTGRGSGTDFTLTISSVQAEDLAVYYCQQYYSTPWTFGGGTKLEIKRGGGGSGGGGSGGGGSGGGGSEVKLVESGGGLVQPGGSLSLSCAASGFTFTDYYMSWVRQPPGKALEWLALIRSKADGYTTEYSASVKGRFTLSRDDSQSILYLQMNALRPEDSATYYCARDAAYYSYYSPEGAMDYWGQGTSVTVSSASGATTTPAPRPPTPAPTIASQPLSLRPEACRPAAGGAVHTRGLDFACDIYIWAPLAGTCGVLLLSLVITLYCRSKRSRLLHSDYMNMTPRRPGPTRKHYQPYAPPRDFAAYRSRVKFSRSADAPAYQQGQNQLYNELNLGRREEYDVLDKRRGRDPEMGGKPQRRKNPQEGLYNELQKDKMAEAYSEIGMKGERRRGKGHDGLYQGLSTATKDTYDALHMQALPPRGSGEGRGSLLTCGDVEENPGPMEYASDASLDPEAPWPPAPRARACRVLPWALVAGLLLLLLLAAACAVFLACPWAVSGARASPGSAASPRLREGPELSPDDPAGLLDLRQGMFAQLVAQNVLLIDGPLSWYSDPGLAGVSLTGGLSYKEDTKELVVAKAGVYYVFFQLELRRVVAGEGSGSVSLALHLQPLRSAAGAAALALTVDLPPASSEARNSAFGFQGRLLHLSAGQRLGVHLHTEARARHAWQLTQGATVLGLFRVTPEIPAGLPSPRSEGSGATNFSLLKQAGDVEENPGPMYRMQLLSCIALSLALVTNSGIHVFILGCFSAGLPKTEANWVNVISDLKKIEDLIQSMHIDATLYTESDVHPSCKVTAMKCFLLELQVISLESGDASIHDTVENLIILANNSLSSNGNVTESGCKECEELEEKNIKEFLQSFVHIVQMFINTSSGGGSGGGGSGGGGSGGGGSGGGSLQAPRRARGCRTLGLPALLLLLLLRPPATRGITCPPPMSVEHADIWVKSYSLYSRERYICNSGFKRKAGTSSLTECVLNKATNVAHWTTPSLKCIR

SEQ ID NO: 33 - DNA, 3245 bp, Artificial Sequence
  Synthetic Sequence
atggccttaccagtgaccgccttgctcctgccgctggccttgctgctccacgccgccaggccgatggccgactacaaggacatcgtgatgacccagagccacaagttcatgagcaccagcgtgggcgacagggtgaacatcacctgcaaggccagccagaacgtggacagcgccgtggcctggtaccagcagaagcccggccagagccccaaggccctgatctacagcgccagctacaggtacagcggcgtgcccgacaggttcaccggcaggggcagcggcaccgacttcaccctgaccatcagcagcgtgcaggccgaggacctggccgtgtactactgccagcagtactacagcaccccctggaccttcggcggcggcaccaagctggagatcaagaggggcggcggcggcagcggcggcggcggcagcggcggcggcggcagcggcggcggcggcagcgaggtgaagctggtggagagcggcggcggcctggtgcagcccggcggcagcctgagcctgagctgcgccgccagcggcttcaccttcaccgactactacatgagctgggtgaggcagccccccggcaaggccctggagtggctggccctgatcaggagcaaggccgacggctacaccaccgagtacagcgccagcgtgaagggcaggttcaccctgagcagggacgacagccagagcatcctgtacctgcagatgaacgccctgaggcccgaggacagcgccacctactactgcgccagggacgccgcctactacagctactacagccccgagggcgccatggactactggggccagggcaccagcgtgaccgtgagcagcgccagcggcgccaccacgacgccagcgccgcgaccaccaacaccggcgcccaccatcgcgtcgcagcccctgtccctgcgcccagaggcgtgccggccagcggcggggggcgcagtgcacacgagggggctggacttcgcctgtgatatctacatctgggcgcccttggccgggacttgtggggtccttctcctgtcactggttatcaccctttactgcaggagtaagaggagcaggctcctgcacagtgactacatgaacatgactccccgccgccccgggcccacccgcaagcattaccagccctatgccccaccacgcgacttcgcagcctatcgctccagagtgaagttcagcaggagcgcagacgcccccgcgtaccagcagggccagaaccagctctataacgagctcaatctaggacgaagagaggagtacgatgttttggacaagagacgtggccgggaccctgagatggggggaaagccgcagagaaggaagaaccctcaggaaggcctgtacaatgaactgcagaaagataagatggcggaggcctacagtgagattgggatgaaaggcgagcgccggaggggcaaggggcacgatggcctttaccagggtctcagtacagccaccaaggacacctacgacgcccttcacatgcaggccctgccccctcgcggcagcggcgaaggccgcggcagcctgctgacctgcggcgatgtggaagaaaacccgggccccatggaatacgcctctgacgcttcactggaccccgaagccccgtggcctcccgcgccccgcgctcgcgcctgccgcgtactgccttgggccctggtcgcggggctgctgctgctgctgctgctcgctgccgcctgcgccgtcttcctcgcctgcccctgggccgtgtccggggctcgcgcctcgcccggctccgcggccagcccgagactccgcgagggtcccgagctttcgcccgacgatcccgccggcctcttggacctgcggcagggcatgtttgcgcagctggtggcccaaaatgttctgctgatcgatgggcccctgagctggtacagtgacccaggcctggcaggcgtgtccctgacggggggcctgagctacaaagaggacacgaaggagctggtggtggccaaggctggagtctactatgtcttctttcaactagagctgcggcgcgtggtggccggcgagggctcaggctccgtttcacttgcgctgcacctgcagccactgcgctctgctgctggggccgccgccctggctttgaccgtggacctgccacccgcctcctccgaggctcggaactcggccttcggtttccagggccgcttgctgcacctgagtgccggccagcgcctgggcgtccatcttcacactgaggccagggcacgccatgcctggcagcttacccagggcgccacagtcttgggactcttccgggtgacccccgaaatcccagccggactcccttcaccgaggtcggaaggaagcggagctactaacttcagcctgctgaagcaggctggagacgtggaggagaaccctggacctatgtacagaatgcagctgctgagctgcatcgccctgagcctggccctggtgaccaacagcggcatccacgtgttcatcctgggctgcttcagcgccggcctgcccaagaccgaggccaactgggtgaacgtgatcagcgacctgaagaagatcgaggacctgatccagagcatgcacatcgacgccaccctgtacaccgagagcgacgtgcaccccagctgcaaggtgaccgccatgaagtgcttcctgctggagctgcaggtgatcagcctggagagcggcgacgccagcatccacgacaccgtggagaacctgatcatcctggccaacaacagcctgagcagcaacggcaacgtgaccgagagcggctgcaaggagtgcgaggagctggaggagaagaacatcaaggagttcctgcagagcttcgtgcacatcgtgcagatgttcatcaacaccagctccggcggcggctccggcggcggcggctccggcggcggcggctccggcggcggcggctccggcggcggctccctgcaggcccccagaagagccagaggctgcagaaccctgggcctgcccgccctgctgctgctgctgctgctgagaccccccgccaccagaggcatcacctgccccccccccatgagcgtggagcacgccgacatctgggtgaagagctacagcctgtacagcagagagagatacatctgcaacagcggcttcaagagaaaggccggcaccagcagcctgaccgagtgcgtgctgaacaaggccaccaacgtggcccactggaccacccccagcctgaagtgcatcagataagtttaaac

SEQ ID NO: 34 - protein, 1324 aa, Artificial Sequence
  Synthetic Sequence
DRTMALPVTALLLPLALLLHAARPMADYKDIVMTQSHKFMSTSVGDRVNITCKASQNVDSAVAWYQQKPGQSPKALIYSASYRYSGVPDRFTGRGSGTDFTLTISSVQAEDLAVYYCQQYYSTPWTFGGGTKLEIKRGGGGSGGGGSGGGGSGGGGSEVKLVESGGGLVQPGGSLSLSCAASGFTFTDYYMSWVRQPPGKALEWLALIRSKADGYTTEYSASVKGRFTLSRDDSQSILYLQMNALRPEDSATYYCARDAAYYSYYSPEGAMDYWGQGTSVTVSSASGATTTPAPRPPTPAPTIASQPLSLRPEACRPAAGGAVHTRGLDFACDIYIWAPLAGTCGVLLLSLVITLYCRSKRSRLLHSDYMNMTPRRPGPTRKHYQPYAPPRDFAAYRSRVKFSRSADAPAYQQGQNQLYNELNLGRREEYDVLDKRRGRDPEMGGKPQRRKNPQEGLYNELQKDKMAEAYSEIGMKGERRRGKGHDGLYQGLSTATKDTYDALHMQALPPRGSGATNFSLLKQAGDVEENPGPMALPVTALLLPLALLLHAARPMADYKDIVMTQSHKFLLVSVGDRVSITCKASQDVSTAVAWYQQKPGQSPKLLIYSASYRYTGVPDRFIGSGSGTDFTLTISSVQAEDLADYFCQQHYSTPLTFGAGTKLEIKRGGGGSGGGGSGGGGSSGGGSEVQLKESGPGLVAPSQSLSITCTVSGFPLTSYGVSWVRQPPGKGLEWLGVIWGDGSTNYHSALISRLSISKDNSKSQVFLKLNNLQTDDTATYYCARDTYYPYYAMDYWGQGTSVTVSSTTTPAPRPPTPAPTIASQPLSLRPEACRPAAGGAVHTRGLDFACDIYIWAPLAGTCGVLLLSLVITLYCKRGRKKLLYIFKQPFMRPVQTTQEEDGCSCRFPEEEEGGCELRVKFSRSADAPAYQQGQNQLYNELNLGRREEYDVLDKRRGRDPEMGGKPQRRKNPQEGLYNELQKDKMAEAYSEIGMKGERRRGKGHDGLYQGLSTATKDTYDALHMQALPPRGSGEGRGSLLTCGDVEENPGPMYRMQLLSCIALSLALVTNSGIHVFILGCFSAGLPKTEANWVNVISDLKKIEDLIQSMHIDATLYTESDVHPSCKVTAMKCFLLELQVISLESGDASIHDTVENLIILANNSLSSNGNVTESGCKECEELEEKNIKEFLQSFVHIVQMFINTSSGGGSGGGGSGGGGSGGGGSGGGSLQAPRRARGCRTLGLPALLLLLLLRPPATRGITCPPPMSVEHADIWVKSYSLYSRERYICNSGFKRKAGTSSLTECVLNKATNVAHWTTPSLKCIR

SEQ ID NO: 35 - DNA, 3985 bp, Artificial Sequence
  Synthetic Sequence
gcgatcgcaccatggccttaccagtgaccgccttgctcctgccgctggccttgctgctccacgccgccaggccgatggccgactacaaggacatcgtgatgacccagagccacaagttcatgagcaccagcgtgggcgacagggtgaacatcacctgcaaggccagccagaacgtggacagcgccgtggcctggtaccagcagaagcccggccagagccccaaggccctgatctacagcgccagctacaggtacagcggcgtgcccgacaggttcaccggcaggggcagcggcaccgacttcaccctgaccatcagcagcgtgcaggccgaggacctggccgtgtactactgccagcagtactacagcaccccctggaccttcggcggcggcaccaagctggagatcaagaggggcggcggcggcagcggcggcggcggcagcggcggcggcggcagcggcggcggcggcagcgaggtgaagctggtggagagcggcggcggcctggtgcagcccggcggcagcctgagcctgagctgcgccgccagcggcttcaccttcaccgactactacatgagctgggtgaggcagccccccggcaaggccctggagtggctggccctgatcaggagcaaggccgacggctacaccaccgagtacagcgccagcgtgaagggcaggttcaccctgagcagggacgacagccagagcatcctgtacctgcagatgaacgccctgaggcccgaggacagcgccacctactactgcgccagggacgccgcctactacagctactacagccccgagggcgccatggactactggggccagggcaccagcgtgaccgtgagcagcgccagcggcgccaccacgacgccagcgccgcgaccaccaacaccggcgcccaccatcgcgtcgcagcccctgtccctgcgcccagaggcgtgccggccagcggcggggggcgcagtgcacacgagggggctggacttcgcctgtgatatctacatctgggcgcccttggccgggacttgtggggtccttctcctgtcactggttatcaccctttactgcaggagtaagaggagcaggctcctgcacagtgactacatgaacatgactccccgccgccccgggcccacccgcaagcattaccagccctatgccccaccacgcgacttcgcagcctatcgctccagagtgaagttcagcaggagcgcagacgcccccgcgtaccagcagggccagaaccagctctataacgagctcaatctaggacgaagagaggagtacgatgttttggacaagagacgtggccgggaccctgagatggggggaaagccgcagagaaggaagaaccctcaggaaggcctgtacaatgaactgcagaaagataagatggcggaggcctacagtgagattgggatgaaaggcgagcgccggaggggcaaggggcacgatggcctttaccagggtctcagtacagccaccaaggacacctacgacgcccttcacatgcaggccctgccccctcgcggaagcggagccaccaacttcagcctgctgaagcaggccggcgacgtggaggagaaccccggccccatggccctgcccgtgaccgccctgctgctgcccctggccctgctgctgcacgccgccaggcccatggccgactacaaggacatcgtgatgacccagagccacaagttcctgctggtgagcgtgggcgacagggtgagcatcacctgcaaggccagccaggacgtgagcaccgccgtggcctggtaccagcagaagcccggccagagccccaagctgctgatctacagcgccagctacaggtacaccggcgtgcccgacaggttcatcggcagcggcagcggcaccgacttcaccctgaccatcagcagcgtgcaggccgaggacctggccgactacttctgccagcagcactacagcacccccctgaccttcggcgccggcaccaagctggagatcaagaggggcggcggcggcagcggcggcggcggcagcggcggcggcggcagcagcggcggcggcagcgaggtgcagctgaaggagagcggccccggcctggtggcccccagccagagcctgagcatcacctgcaccgtgagcggcttccccctgaccagctacggcgtgagctgggtgaggcagccccccggcaagggcctggagtggctgggcgtgatctggggcgacggcagcaccaactaccacagcgccctgatcagcaggctgagcatcagcaaggacaacagcaagagccaggtgttcctgaagctgaacaacctgcagaccgacgacaccgccacctactactgcgccagggacacctactacccctactacgccatggactactggggccagggcaccagcgtgaccgtgagcagcaccaccacccccgcccccaggccccccacccccgcccccaccatcgccagccagcccctgagcctgaggcccgaggcctgcaggcccgccgccggcggcgccgtgcacaccaggggcctggacttcgcctgcgacatctacatctgggcccccctggccggcacctgcggcgtgctgctgctgagcctggtgatcaccctgtactgcaaacggggcagaaagaaactcctgtatatattcaaacaaccatttatgagaccagtacaaactactcaagaggaagatggctgtagctgccgatttccagaagaagaagaaggaggatgtgaactgagggtgaagttcagcaggagcgccgacgcccccgcctaccagcagggccagaaccagctgtacaacgagctgaacctgggcaggagggaggagtacgacgtgctggacaagaggaggggcagggaccccgagatgggcggcaagccccagaggaggaagaacccccaggagggcctgtacaacgagctgcagaaggacaagatggccgaggcctacagcgagatcggcatgaagggcgagaggaggaggggcaagggccacgacggcctgtaccagggcctgagcaccgccaccaaggacacctacgacgccctgcacatgcaggccctgccccccaggggcagcggcgaaggccgcggcagcctgctgacctgcggcgatgtggaagaaaacccgggccccatgtacagaatgcagctgctgagctgcatcgccctgagcctggccctggtgaccaacagcggcatccacgtgttcatcctgggctgcttcagcgccggcctgcccaagaccgaggccaactgggtgaacgtgatcagcgacctgaagaagatcgaggacctgatccagagcatgcacatcgacgccaccctgtacaccgagagcgacgtgcaccccagctgcaaggtgaccgccatgaagtgcttcctgctggagctgcaggtgatcagcctggagagcggcgacgccagcatccacgacaccgtggagaacctgatcatcctggccaacaacagcctgagcagcaacggcaacgtgaccgagagcggctgcaaggagtgcgaggagctggaggagaagaacatcaaggagttcctgcagagcttcgtgcacatcgtgcagatgttcatcaacaccagctccggcggcggctccggcggcggcggctccggcggcggcggctccggcggcggcggctccggcggcggctccctgcaggcccccagaagagccagaggctgcagaaccctgggcctgcccgccctgctgctgctgctgctgctgagaccccccgccaccagaggcatcacctgccccccccccatgagcgtggagcacgccgacatctgggtgaagagctacagcctgtacagcagagagagatacatctgcaacagcggcttcaagagaaaggccggcaccagcagcctgaccgagtgcgtgctgaacaaggccaccaacgtggcccactggaccacccccagcctgaagtgcatcagataagtttaaac

SEQ ID NO: 36 - protein, 1313 aa, Artificial Sequence
  Synthetic Sequence
DRTMALPVTALLLPLALLLHAARPMADYKDIVMTQSHKFMSTSVGDRVNITCKASQNVDSAVAWYQQKPGQSPKALIYSASYRYSGVPDRFTGRGSGTDFTLTISSVQAEDLAVYYCQQYYSTPWTFGGGTKLEIKRGGGGSGGGGSGGGGSGGGGSEVKLVESGGGLVQPGGSLSLSCAASGFTFTDYYMSWVRQPPGKALEWLALIRSKADGYTTEYSASVKGRFTLSRDDSQSILYLQMNALRPEDSATYYCARDAAYYSYYSPEGAMDYWGQGTSVTVSSASGATTTPAPRPPTPAPTIASQPLSLRPEACRPAAGGAVHTRGLDFACDIYIWAPLAGTCGVLLLSLVITLYCRSKRSRLLHSDYMNMTPRRPGPTRKHYQPYAPPRDFAAYRSRVKFSRSADAPAYQQGQNQLYNELNLGRREEYDVLDKRRGRDPEMGGKPQRRKNPQEGLYNELQKDKMAEAYSEIGMKGERRRGKGHDGLYQGLSTATKDTYDALHMQALPPRGSGATNFSLLKQAGDVEENPGPMALPVTALLLPLALLLHAARPDIQMTQSHKFMSTSVGDRVSITCKASQDVSTAVAWFQQKPGQSPKLLIYSPSYRYTGVPDRFTGSGSGTDFTFTISSVQAEDLAVYYCQQLYSTPYTFGGGTKLEIKGGGGSGGGGSGGGGSEVQLQQSGPELVKPGASVKMSCKASGYTFTDYYLDWVKQSHGESFEWIGRVNPYNGGTIYNQKFKGKATLTVDKSSSTAYMDLNSLTSEDSAVYYCARDHYRYDPLLDYWGQGTTLTVSSTTTPAPRPPTPAPTIASQPLSLRPEACRPAAGGAVHTRGLDFACDIYIWAPLAGTCGVLLLSLVITLYCRSKRSRLLHSDYMNMTPRRPGPTRKHYQPYAPPRDFAAYRSRVKFSRSADAPAYQQGQNQLYNELNLGRREEYDVLDKRRGRDPEMGGKPQRRKNPQEGLYNELQKDKMAEAYSEIGMKGERRRGKGHDGLYQGLSTATKDTYDALHMQALPPRGSGEGRGSLLTCGDVEENPGPMYRMQLLSCIALSLALVTNSGIHVFILGCFSAGLPKTEANWVNVISDLKKIEDLIQSMHIDATLYTESDVHPSCKVTAMKCFLLELQVISLESGDASIHDTVENLIILANNSLSSNGNVTESGCKECEELEEKNIKEFLQSFVHIVQMFINTSSGGGSGGGGSGGGGSGGGGSGGGSLQAPRRARGCRTLGLPALLLLLLLRPPATRGITCPPPMSVEHADIWVKSYSLYSRERYICNSGFKRKAGTSSLTECVLNKATNVAHWTTPSLKCIR

SEQ ID NO: 37 - DNA, 3941 bp, Artificial Sequence
  Synthetic Sequence
atggccttaccagtgaccgccttgctcctgccgctggccttgctgctccacgccgccaggccgatggccgactacaaggacatcgtgatgacccagagccacaagttcatgagcaccagcgtgggcgacagggtgaacatcacctgcaaggccagccagaacgtggacagcgccgtggcctggtaccagcagaagcccggccagagccccaaggccctgatctacagcgccagctacaggtacagcggcgtgcccgacaggttcaccggcaggggcagcggcaccgacttcaccctgaccatcagcagcgtgcaggccgaggacctggccgtgtactactgccagcagtactacagcaccccctggaccttcggcggcggcaccaagctggagatcaagaggggcggcggcggcagcggcggcggcggcagcggcggcggcggcagcggcggcggcggcagcgaggtgaagctggtggagagcggcggcggcctggtgcagcccggcggcagcctgagcctgagctgcgccgccagcggcttcaccttcaccgactactacatgagctgggtgaggcagccccccggcaaggccctggagtggctggccctgatcaggagcaaggccgacggctacaccaccgagtacagcgccagcgtgaagggcaggttcaccctgagcagggacgacagccagagcatcctgtacctgcagatgaacgccctgaggcccgaggacagcgccacctactactgcgccagggacgccgcctactacagctactacagccccgagggcgccatggactactggggccagggcaccagcgtgaccgtgagcagcgccagcggcgccaccacgacgccagcgccgcgaccaccaacaccggcgcccaccatcgcgtcgcagcccctgtccctgcgcccagaggcgtgccggccagcggcggggggcgcagtgcacacgagggggctggacttcgcctgtgatatctacatctgggcgcccttggccgggacttgtggggtccttctcctgtcactggttatcaccctttactgcaggagtaagaggagcaggctcctgcacagtgactacatgaacatgactccccgccgccccgggcccacccgcaagcattaccagccctatgccccaccacgcgacttcgcagcctatcgctccagagtgaagttcagcaggagcgcagacgcccccgcgtaccagcagggccagaaccagctctataacgagctcaatctaggacgaagagaggagtacgatgttttggacaagagacgtggccgggaccctgagatggggggaaagccgcagagaaggaagaaccctcaggaaggcctgtacaatgaactgcagaaagataagatggcggaggcctacagtgagattgggatgaaaggcgagcgccggaggggcaaggggcacgatggcctttaccagggtctcagtacagccaccaaggacacctacgacgcccttcacatgcaggccctgccccctcgcggaagcggagccaccaacttcagcctgctgaagcaggccggcgacgtggaggagaaccccggccccatggccctgcccgtgaccgccctgctgctgcccctggccctgctgctgcacgccgccaggcccgacatccagatgacccagagccacaagttcatgagcaccagcgtgggcgacagggtgagcatcacctgcaaggccagccaggacgtgagcaccgccgtggcctggttccagcagaagcccggccagagccccaagctgctgatctacagccccagctacaggtacaccggcgtgcccgacaggttcaccggcagcggcagcggcaccgacttcaccttcaccatcagcagcgtgcaggccgaggacctggccgtgtactactgccagcagctgtacagcaccccctacaccttcggcggcggcaccaagctggagatcaagggaggggggggatccgggggaggaggctccggcggaggcggaagcgaggtgcagctgcagcagagcggccccgagctggtgaagcccggcgccagcgtgaagatgagctgcaaggccagcggctacaccttcaccgactactacctggactgggtgaagcagagccacggcgagagcttcgagtggatcggcagggtgaacccctacaacggcggcaccatctacaaccagaagttcaagggcaaggccaccctgaccgtggacaagagcagcagcaccgcctacatggacctgaacagcctgaccagcgaggacagcgccgtgtactactgcgccagggaccactacaggtacgaccccctgctggactactggggccagggcaccaccctgaccgtgagcagcaccaccacccccgcccccaggccccccacccccgcccccaccatcgccagccagcccctgagcctgaggcccgaggcctgcaggcccgccgccggcggcgccgtgcacaccaggggcctggacttcgcctgcgacatctacatctgggcccccctggccggcacctgcggcgtgctgctgctgagcctggtgatcaccctgtactgcaggagtaagaggagcaggctcctgcacagtgactacatgaacatgactccccgccgccccgggcccacccgcaagcattaccagccctatgccccaccacgcgacttcgcagcctatcgctccagggtgaagttcagcaggagcgccgacgcccccgcctaccagcagggccagaaccagctgtacaacgagctgaacctgggcaggagggaggagtacgacgtgctggacaagaggaggggcagggaccccgagatgggcggcaagccccagaggaggaagaacccccaggagggcctgtacaacgagctgcagaaggacaagatggccgaggcctacagcgagatcggcatgaagggcgagaggaggaggggcaagggccacgacggcctgtaccagggcctgagcaccgccaccaaggacacctacgacgccctgcacatgcaggccctgccccccaggggcagcggcgaaggccgcggcagcctgctgacctgcggcgatgtggaagaaaacccgggccccatgtacagaatgcagctgctgagctgcatcgccctgagcctggccctggtgaccaacagcggcatccacgtgttcatcctgggctgcttcagcgccggcctgcccaagaccgaggccaactgggtgaacgtgatcagcgacctgaagaagatcgaggacctgatccagagcatgcacatcgacgccaccctgtacaccgagagcgacgtgcaccccagctgcaaggtgaccgccatgaagtgcttcctgctggagctgcaggtgatcagcctggagagcggcgacgccagcatccacgacaccgtggagaacctgatcatcctggccaacaacagcctgagcagcaacggcaacgtgaccgagagcggctgcaaggagtgcgaggagctggaggagaagaacatcaaggagttcctgcagagcttcgtgcacatcgtgcagatgttcatcaacaccagctccggcggcggctccggcggcggcggctccggcggcggcggctccggcggcggcggctccggcggcggctccctgcaggcccccagaagagccagaggctgcagaaccctgggcctgcccgccctgctgctgctgctgctgctgagaccccccgccaccagaggcatcacctgccccccccccatgagcgtggagcacgccgacatctgggtgaagagctacagcctgtacagcagagagagatacatctgcaacagcggcttcaagagaaaggccggcaccagcagcctgaccgagtgcgtgctgaacaaggccaccaacgtggcccactggaccacccccagcctgaagtgcatcagataagtttaaac

SEQ ID NO: 38 - protein, 1061 aa, Artificial Sequence
  Synthetic Sequence
DRTMALPVTALLLPLALLLHAARPDVVMTQSHRFMSTSVGDRVSITCRASQDVNTAVSWYQQKPGQSPKLLIFSASYRYTGVPDRFTGSGSGADFTLTISSVQAEDLAVYYCQQHYSTPWTFGGGTKLDIKGGGGSGGGGSGGGGSQIQLVQSGPDLKKPGETVKLSCKASGYTFTNFGMNWVKQAPGKGFKWMAWINTYTGESYFADDFKGRFAFSVETSATTAYLQINNLKTEDTATYFCARGEIYYGYDGGFAYWGQGTLVTVSATTTPAPRPPTPAPTIASQPLSLRPEACRPAAGGAVHTRGLDFACDIYIWAPLAGTCGVLLLSLVITLYCRSKRSRLLHSDYMNMTPRRPGPTRKHYQPYAPPRDFAAYRSRVKFSRSADAPAYQQGQNQLYNELNLGRREEYDVLDKRRGRDPEMGGKPQRRKNPQEGLYNELQKDKMAEAYSEIGMKGERRRGKGHDGLYQGLSTATKDTYDALHMQALPPRGSGEGRGSLLTCGDVEENPGPMEYASDASLDPEAPWPPAPRARACRVLPWALVAGLLLLLLLAAACAVFLACPWAVSGARASPGSAASPRLREGPELSPDDPAGLLDLRQGMFAQLVAQNVLLIDGPLSWYSDPGLAGVSLTGGLSYKEDTKELVVAKAGVYYVFFQLELRRVVAGEGSGSVSLALHLQPLRSAAGAAALALTVDLPPASSEARNSAFGFQGRLLHLSAGQRLGVHLHTEARARHAWQLTQGATVLGLFRVTPEIPAGLPSPRSEGSGATNFSLLKQAGDVEENPGPMYRMQLLSCIALSLALVTNSGIHVFILGCFSAGLPKTEANWVNVISDLKKIEDLIQSMHIDATLYTESDVHPSCKVTAMKCFLLELQVISLESGDASIHDTVENLIILANNSLSSNGNVTESGCKECEELEEKNIKEFLQSFVHIVQMFINTSSGGGSGGGGSGGGGSGGGGSGGGSLQAPRRARGCRTLGLPALLLLLLLRPPATRGITCPPPMSVEHADIWVKSYSLYSRERYICNSGFKRKAGTSSLTECVLNKATNVAHWTTPSLKCIR

SEQ ID NO: 39 - DNA, 3185 bp, Artificial Sequence
  Synthetic Sequence
atggccttaccagtgaccgccttgctcctgccgctggccttgctgctccacgccgccaggccggacgtggtgatgacccagagccacaggttcatgagcaccagcgtgggcgacagggtgagcatcacctgcagggccagccaggacgtgaacaccgccgtgagctggtaccagcagaagcccggccagagccccaagctgctgatcttcagcgccagctacaggtacaccggcgtgcccgacaggttcaccggcagcggcagcggcgccgacttcaccctgaccatcagcagcgtgcaggccgaggacctggccgtgtactactgccagcagcactacagcaccccctggaccttcggcggcggcaccaagctggacatcaagggaggggggggatccgggggaggaggctccggcggaggcggaagccagatccagctggtgcagagcggccccgacctgaagaagcccggcgagaccgtgaagctgagctgcaaggccagcggctacaccttcaccaacttcggcatgaactgggtgaagcaggcccccggcaagggcttcaagtggatggcctggatcaacacctacaccggcgagagctacttcgccgacgacttcaagggcaggttcgccttcagcgtggagaccagcgccaccaccgcctacctgcagatcaacaacctgaagaccgaggacaccgccacctacttctgcgccaggggcgagatctactacggctacgacggcggcttcgcctactggggccagggcaccctggtgaccgtgagcgccaccacgacgccagcgccgcgaccaccaacaccggcgcccaccatcgcgtcgcagcccctgtccctgcgcccagaggcgtgccggccagcggcggggggcgcagtgcacacgagggggctggacttcgcctgtgatatctacatctgggcgcccttggccgggacttgtggggtccttctcctgtcactggttatcaccctttactgcaggagtaagaggagcaggctcctgcacagtgactacatgaacatgactccccgccgccccgggcccacccgcaagcattaccagccctatgccccaccacgcgacttcgcagcctatcgctccagagtgaagttcagcaggagcgcagacgcccccgcgtaccagcagggccagaaccagctctataacgagctcaatctaggacgaagagaggagtacgatgttttggacaagagacgtggccgggaccctgagatggggggaaagccgcagagaaggaagaaccctcaggaaggcctgtacaatgaactgcagaaagataagatggcggaggcctacagtgagattgggatgaaaggcgagcgccggaggggcaaggggcacgatggcctttaccagggtctcagtacagccaccaaggacacctacgacgcccttcacatgcaggccctgccccctcgcggcagcggcgaaggccgcggcagcctgctgacctgcggcgatgtggaagaaaacccgggccccatggaatacgcctctgacgcttcactggaccccgaagccccgtggcctcccgcgccccgcgctcgcgcctgccgcgtactgccttgggccctggtcgcggggctgctgctgctgctgctgctcgctgccgcctgcgccgtcttcctcgcctgcccctgggccgtgtccggggctcgcgcctcgcccggctccgcggccagcccgagactccgcgagggtcccgagctttcgcccgacgatcccgccggcctcttggacctgcggcagggcatgtttgcgcagctggtggcccaaaatgttctgctgatcgatgggcccctgagctggtacagtgacccaggcctggcaggcgtgtccctgacggggggcctgagctacaaagaggacacgaaggagctggtggtggccaaggctggagtctactatgtcttctttcaactagagctgcggcgcgtggtggccggcgagggctcaggctccgtttcacttgcgctgcacctgcagccactgcgctctgctgctggggccgccgccctggctttgaccgtggacctgccacccgcctcctccgaggctcggaactcggccttcggtttccagggccgcttgctgcacctgagtgccggccagcgcctgggcgtccatcttcacactgaggccagggcacgccatgcctggcagcttacccagggcgccacagtcttgggactcttccgggtgacccccgaaatcccagccggactcccttcaccgaggtcggaaggaagcggagctactaacttcagcctgctgaagcaggctggagacgtggaggagaaccctggacctatgtacagaatgcagctgctgagctgcatcgccctgagcctggccctggtgaccaacagcggcatccacgtgttcatcctgggctgcttcagcgccggcctgcccaagaccgaggccaactgggtgaacgtgatcagcgacctgaagaagatcgaggacctgatccagagcatgcacatcgacgccaccctgtacaccgagagcgacgtgcaccccagctgcaaggtgaccgccatgaagtgcttcctgctggagctgcaggtgatcagcctggagagcggcgacgccagcatccacgacaccgtggagaacctgatcatcctggccaacaacagcctgagcagcaacggcaacgtgaccgagagcggctgcaaggagtgcgaggagctggaggagaagaacatcaaggagttcctgcagagcttcgtgcacatcgtgcagatgttcatcaacaccagctccggcggcggctccggcggcggcggctccggcggcggcggctccggcggcggcggctccggcggcggctccctgcaggcccccagaagagccagaggctgcagaaccctgggcctgcccgccctgctgctgctgctgctgctgagaccccccgccaccagaggcatcacctgccccccccccatgagcgtggagcacgccgacatctgggtgaagagctacagcctgtacagcagagagagatacatctgcaacagcggcttcaagagaaaggccggcaccagcagcctgaccgagtgcgtgctgaacaaggccaccaacgtggcccactggaccacccccagcctgaagtgcatcagataagtttaaac

SEQ ID NO: 40 - protein, 1301 aa, Artificial Sequence
  Synthetic Sequence
DRTMALPVTALLLPLALLLHAARPDVVMTQSHRFMSTSVGDRVSITCRASQDVNTAVSWYQQKPGQSPKLLIFSASYRYTGVPDRFTGSGSGADFTLTISSVQAEDLAVYYCQQHYSTPWTFGGGTKLDIKGGGGSGGGGSGGGGSQIQLVQSGPDLKKPGETVKLSCKASGYTFTNFGMNWVKQAPGKGFKWMAWINTYTGESYFADDFKGRFAFSVETSATTAYLQINNLKTEDTATYFCARGEIYYGYDGGFAYWGQGTLVTVSATTTPAPRPPTPAPTIASQPLSLRPEACRPAAGGAVHTRGLDFACDIYIWAPLAGTCGVLLLSLVITLYCRSKRSRLLHSDYMNMTPRRPGPTRKHYQPYAPPRDFAAYRSRVKFSRSADAPAYQQGQNQLYNELNLGRREEYDVLDKRRGRDPEMGGKPQRRKNPQEGLYNELQKDKMAEAYSEIGMKGERRRGKGHDGLYQGLSTATKDTYDALHMQALPPRGSGATNFSLLKQAGDVEENPGPMALPVTALLLPLALLLHAARPDIELTQSPSSFSVSLGDRVTITCKASEDIYNRLAWYQQKPGNAPRLLISGATSLETGVPSRFSGSGSGKDYTLSITSLQTEDVATYYCQQYWSTPTFGGGTKLEIKRAAGGGGSGGGGSGGGGSAQPAMAKVQLQESGPSLVQPSQRLSITCTVSGFSLISYGVHWVRQSPGKGLEWLGVIWRGGSTDYNAAFMSRLSITKDNSKSQVFFKMNSLQADDTAIYFCAKTLITTGYAMDYWGQGTTVTVSSTTTPAPRPPTPAPTIASQPLSLRPEACRPAAGGAVHTRGLDFACDIYIWAPLAGTCGVLLLSLVITLYCKRGRKKLLYIFKQPFMRPVQTTQEEDGCSCRFPEEEEGGCELRVKFSRSADAPAYQQGQNQLYNELNLGRREEYDVLDKRRGRDPEMGGKPQRRKNPQEGLYNELQKDKMAEAYSEIGMKGERRRGKGHDGLYQGLSTATKDTYDALHMQALPPRGSGEGRGSLLTCGDVEENPGPMYRMQLLSCIALSLALVTNSGIHVFILGCFSAGLPKTEANWVNVISDLKKIEDLIQSMHIDATLYTESDVHPSCKVTAMKCFLLELQVISLESGDASIHDTVENLIILANNSLSSNGNVTESGCKECEELEEKNIKEFLQSFVHIVQMFINTSSGGGSGGGGSGGGGSGGGGSGGGSLQAPRRARGCRTLGLPALLLLLLLRPPATRGITCPPPMSVEHADIWVKSYSLYSRERYICNSGFKRKAGTSSLTECVLNKATNVAHWTTPSLKCIR

SEQ ID NO: 41 - DNA, 3905 bp, Artificial Sequence
  Synthetic Sequence
atggccttaccagtgaccgccttgctcctgccgctggccttgctgctccacgccgccaggccggacgtggtgatgacccagagccacaggttcatgagcaccagcgtgggcgacagggtgagcatcacctgcagggccagccaggacgtgaacaccgccgtgagctggtaccagcagaagcccggccagagccccaagctgctgatcttcagcgccagctacaggtacaccggcgtgcccgacaggttcaccggcagcggcagcggcgccgacttcaccctgaccatcagcagcgtgcaggccgaggacctggccgtgtactactgccagcagcactacagcaccccctggaccttcggcggcggcaccaagctggacatcaagggaggggggggatccgggggaggaggctccggcggaggcggaagccagatccagctggtgcagagcggccccgacctgaagaagcccggcgagaccgtgaagctgagctgcaaggccagcggctacaccttcaccaacttcggcatgaactgggtgaagcaggcccccggcaagggcttcaagtggatggcctggatcaacacctacaccggcgagagctacttcgccgacgacttcaagggcaggttcgccttcagcgtggagaccagcgccaccaccgcctacctgcagatcaacaacctgaagaccgaggacaccgccacctacttctgcgccaggggcgagatctactacggctacgacggcggcttcgcctactggggccagggcaccctggtgaccgtgagcgccaccacgacgccagcgccgcgaccaccaacaccggcgcccaccatcgcgtcgcagcccctgtccctgcgcccagaggcgtgccggccagcggcggggggcgcagtgcacacgagggggctggacttcgcctgtgatatctacatctgggcgcccttggccgggacttgtggggtccttctcctgtcactggttatcaccctttactgcaggagtaagaggagcaggctcctgcacagtgactacatgaacatgactccccgccgccccgggcccacccgcaagcattaccagccctatgccccaccacgcgacttcgcagcctatcgctccagagtgaagttcagcaggagcgcagacgcccccgcgtaccagcagggccagaaccagctctataacgagctcaatctaggacgaagagaggagtacgatgttttggacaagagacgtggccgggaccctgagatggggggaaagccgcagagaaggaagaaccctcaggaaggcctgtacaatgaactgcagaaagataagatggcggaggcctacagtgagattgggatgaaaggcgagcgccggaggggcaaggggcacgatggcctttaccagggtctcagtacagccaccaaggacacctacgacgcccttcacatgcaggccctgccccctcgcggaagcggagccaccaacttcagcctgctgaagcaggccggcgacgtggaggagaaccccggccccatggccctgcccgtgaccgccctgctgctgcccctggccctgctgctgcacgccgccaggcccgacatcgagctgacccagagccccagcagcttcagcgtgagcctgggcgacagggtgaccatcacctgcaaggccagcgaggacatctacaacaggctggcctggtaccagcagaagcccggcaacgcccccaggctgctgatcagcggcgccaccagcctggagaccggcgtgcccagcaggttcagcggcagcggcagcggcaaggactacaccctgagcatcaccagcctgcagaccgaggacgtggccacctactactgccagcagtactggagcacccccaccttcggcggcggcaccaagctggagatcaagagggccgccggcggcggcggcagcggcggcggcggcagcggcggcggcggcagcgcccagcccgccatggccaaggtgcagctgcaggagagcggccccagcctggtgcagcccagccagaggctgagcatcacctgcaccgtgagcggcttcagcctgatcagctacggcgtgcactgggtgaggcagagccccggcaagggcctggagtggctgggcgtgatctggaggggcggcagcaccgactacaacgccgccttcatgagcaggctgagcatcaccaaggacaacagcaagagccaggtgttcttcaagatgaacagcctgcaggccgacgacaccgccatctacttctgcgccaagaccctgatcaccaccggctacgccatggactactggggccagggcaccaccgtgaccgtgagcagcaccaccacccccgcccccaggccccccacccccgcccccaccatcgccagccagcccctgagcctgaggcccgaggcctgcaggcccgccgccggcggcgccgtgcacaccaggggcctggacttcgcctgcgacatctacatctgggcccccctggccggcacctgcggcgtgctgctgctgagcctggtgatcaccctgtactgcaaacggggcagaaagaaactcctgtatatattcaaacaaccatttatgagaccagtacaaactactcaagaggaagatggctgtagctgccgatttccagaagaagaagaaggaggatgtgaactgagggtgaagttcagcaggagcgccgacgcccccgcctaccagcagggccagaaccagctgtacaacgagctgaacctgggcaggagggaggagtacgacgtgctggacaagaggaggggcagggaccccgagatgggcggcaagccccagaggaggaagaacccccaggagggcctgtacaacgagctgcagaaggacaagatggccgaggcctacagcgagatcggcatgaagggcgagaggaggaggggcaagggccacgacggcctgtaccagggcctgagcaccgccaccaaggacacctacgacgccctgcacatgcaggccctgccccccaggggcagcggcgaaggccgcggcagcctgctgacctgcggcgatgtggaagaaaacccgggccccatgtacagaatgcagctgctgagctgcatcgccctgagcctggccctggtgaccaacagcggcatccacgtgttcatcctgggctgcttcagcgccggcctgcccaagaccgaggccaactgggtgaacgtgatcagcgacctgaagaagatcgaggacctgatccagagcatgcacatcgacgccaccctgtacaccgagagcgacgtgcaccccagctgcaaggtgaccgccatgaagtgcttcctgctggagctgcaggtgatcagcctggagagcggcgacgccagcatccacgacaccgtggagaacctgatcatcctggccaacaacagcctgagcagcaacggcaacgtgaccgagagcggctgcaaggagtgcgaggagctggaggagaagaacatcaaggagttcctgcagagcttcgtgcacatcgtgcagatgttcatcaacaccagctccggcggcggctccggcggcggcggctccggcggcggcggctccggcggcggcggctccggcggcggctccctgcaggcccccagaagagccagaggctgcagaaccctgggcctgcccgccctgctgctgctgctgctgctgagaccccccgccaccagaggcatcacctgccccccccccatgagcgtggagcacgccgacatctgggtgaagagctacagcctgtacagcagagagagatacatctgcaacagcggcttcaagagaaaggccggcaccagcagcctgaccgagtgcgtgctgaacaaggccaccaacgtggcccactggaccacccccagcctgaagtgcatcagataagtttaaac

SEQ ID NO: 42 - protein, 1291 aa, Artificial Sequence
  Synthetic Sequence
DRTMALPVTALLLPLALLLHAARPDVVMTQSHRFMSTSVGDRVSITCRASQDVNTAVSWYQQKPGQSPKLLIFSASYRYTGVPDRFTGSGSGADFTLTISSVQAEDLAVYYCQQHYSTPWTFGGGTKLDIKGGGGSGGGGSGGGGSQIQLVQSGPDLKKPGETVKLSCKASGYTFTNFGMNWVKQAPGKGFKWMAWINTYTGESYFADDFKGRFAFSVETSATTAYLQINNLKTEDTATYFCARGEIYYGYDGGFAYWGQGTLVTVSATTTPAPRPPTPAPTIASQPLSLRPEACRPAAGGAVHTRGLDFACDIYIWAPLAGTCGVLLLSLVITLYCRSKRSRLLHSDYMNMTPRRPGPTRKHYQPYAPPRDFAAYRSRVKFSRSADAPAYQQGQNQLYNELNLGRREEYDVLDKRRGRDPEMGGKPQRRKNPQEGLYNELQKDKMAEAYSEIGMKGERRRGKGHDGLYQGLSTATKDTYDALHMQALPPRGSGATNFSLLKQAGDVEENPGPMALPVTALLLPLALLLHAARPDIQMTQSPSSLSASVGDRVTITCKASQDVGIAVAWYQQKPGKVPKLLIYWASTRHTGVPDRFSGSGSGTDFTLTISSLQPEDVATYYCQQYSSYPYTFGQGTKVEIKGGGGSGGGGSGGGGSEVQLVESGGGLVQPGGSLRLSCAASGFFSRYWMSWVRQAPGKGLEWIGEINPDSSTINYAPSLKDKFIISRDNAKNSLYLQMNSLRAEDTAVYYCARPDGNYWYFDVWGQGTLVTVSSTTTPAPRPPTPAPTIASQPLSLRPEACRPAAGGAVHTRGLDFACDIYIWAPLAGTCGVLLLSLVITLYCRSKRSRLLHSDYMNMTPRRPGPTRKHYQPYAPPRDFAAYRSRVKFSRSADAPAYQQGQNQLYNELNLGRREEYDVLDKRRGRDPEMGGKPQRRKNPQEGLYNELQKDKMAEAYSEIGMKGERRRGKGHDGLYQGLSTATKDTYDALHMQALPPRGSGEGRGSLLTCGDVEENPGPMYRMQLLSCIALSLALVTNSGIHVFILGCFSAGLPKTEANWVNVISDLKKIEDLIQSMHIDATLYTESDVHPSCKVTAMKCFLLELQVISLESGDASIHDTVENLIILANNSLSSNGNVTESGCKECEELEEKNIKEFLQSFVHIVQMFINTSSGGGSGGGGSGGGGSGGGGSGGGSLQAPRRARGCRTLGLPALLLLLLLRPPATRGITCPPPMSVEHADIWVKSYSLYSRERYICNSGFKRKAGTSSLTECVLNKATNVAHWTTPSLKCIR

SEQ ID NO: 43 - DNA, 3875 bp, Artificial Sequence
  Synthetic Sequence
atggccttaccagtgaccgccttgctcctgccgctggccttgctgctccacgccgccaggccggacgtggtgatgacccagagccacaggttcatgagcaccagcgtgggcgacagggtgagcatcacctgcagggccagccaggacgtgaacaccgccgtgagctggtaccagcagaagcccggccagagccccaagctgctgatcttcagcgccagctacaggtacaccggcgtgcccgacaggttcaccggcagcggcagcggcgccgacttcaccctgaccatcagcagcgtgcaggccgaggacctggccgtgtactactgccagcagcactacagcaccccctggaccttcggcggcggcaccaagctggacatcaagggaggggggggatccgggggaggaggctccggcggaggcggaagccagatccagctggtgcagagcggccccgacctgaagaagcccggcgagaccgtgaagctgagctgcaaggccagcggctacaccttcaccaacttcggcatgaactgggtgaagcaggcccccggcaagggcttcaagtggatggcctggatcaacacctacaccggcgagagctacttcgccgacgacttcaagggcaggttcgccttcagcgtggagaccagcgccaccaccgcctacctgcagatcaacaacctgaagaccgaggacaccgccacctacttctgcgccaggggcgagatctactacggctacgacggcggcttcgcctactggggccagggcaccctggtgaccgtgagcgccaccacgacgccagcgccgcgaccaccaacaccggcgcccaccatcgcgtcgcagcccctgtccctgcgcccagaggcgtgccggccagcggcggggggcgcagtgcacacgagggggctggacttcgcctgtgatatctacatctgggcgcccttggccgggacttgtggggtccttctcctgtcactggttatcaccctttactgcaggagtaagaggagcaggctcctgcacagtgactacatgaacatgactccccgccgccccgggcccacccgcaagcattaccagccctatgccccaccacgcgacttcgcagcctatcgctccagagtgaagttcagcaggagcgcagacgcccccgcgtaccagcagggccagaaccagctctataacgagctcaatctaggacgaagagaggagtacgatgttttggacaagagacgtggccgggaccctgagatggggggaaagccgcagagaaggaagaaccctcaggaaggcctgtacaatgaactgcagaaagataagatggcggaggcctacagtgagattgggatgaaaggcgagcgccggaggggcaaggggcacgatggcctttaccagggtctcagtacagccaccaaggacacctacgacgcccttcacatgcaggccctgccccctcgcggaagcggagccaccaacttcagcctgctgaagcaggccggcgacgtggaggagaaccccggccccatggccttaccagtgaccgccttgctcctgccgctggccttgctgctccacgccgccaggccggacatccagatgacccagagccccagcagcctgagcgccagcgtgggcgacagggtgaccatcacctgcaaggccagccaggacgtgggcatcgccgtggcctggtaccagcagaagcccggcaaggtgcccaagctgctgatctactgggccagcaccaggcacaccggcgtgcccgacaggttcagcggcagcggcagcggcaccgacttcaccctgaccatcagcagcctgcagcccgaggacgtggccacctactactgccagcagtacagcagctacccctacaccttcggccagggcaccaaggtggagatcaagggaggggggggatccgggggaggaggctccggcggaggcggaagcgaggtgcagctggtggagagcggcggcggcctggtgcagcccggcggcagcctgaggctgagctgcgccgccagcggcttcttcagcaggtactggatgagctgggtgaggcaggcccccggcaagggcctggagtggatcggcgagatcaaccccgacagcagcaccatcaactacgcccccagcctgaaggacaagttcatcatcagcagggacaacgccaagaacagcctgtacctgcagatgaacagcctgagggccgaggacaccgccgtgtactactgcgccaggcccgacggcaactactggtacttcgacgtgtggggccagggcaccctggtgaccgtgagcagcaccacgacgccagcgccgcgaccaccaacaccggcgcccaccatcgcgtcgcagcccctgtccctgcgcccagaggcgtgccggccagcggcggggggcgcagtgcacacgagggggctggacttcgcctgtgatatctacatctgggcgcccttggccgggacttgtggggtccttctcctgtcactggttatcaccctttactgcaggagtaagaggagcaggctcctgcacagtgactacatgaacatgactccccgccgccccgggcccacccgcaagcattaccagccctatgccccaccacgcgacttcgcagcctatcgctccagagtgaagttcagcaggagcgcagacgcccccgcgtaccagcagggccagaaccagctctataacgagctcaatctaggacgaagagaggagtacgatgttttggacaagagacgtggccgggaccctgagatggggggaaagccgcagagaaggaagaaccctcaggaaggcctgtacaatgaactgcagaaagataagatggcggaggcctacagtgagattgggatgaaaggcgagcgccggaggggcaaggggcacgatggcctttaccagggtctcagtacagccaccaaggacacctacgacgcccttcacatgcaggccctgccccctcgcggcagcggcgaaggccgcggcagcctgctgacctgcggcgatgtggaagaaaacccgggccccatgtacagaatgcagctgctgagctgcatcgccctgagcctggccctggtgaccaacagcggcatccacgtgttcatcctgggctgcttcagcgccggcctgcccaagaccgaggccaactgggtgaacgtgatcagcgacctgaagaagatcgaggacctgatccagagcatgcacatcgacgccaccctgtacaccgagagcgacgtgcaccccagctgcaaggtgaccgccatgaagtgcttcctgctggagctgcaggtgatcagcctggagagcggcgacgccagcatccacgacaccgtggagaacctgatcatcctggccaacaacagcctgagcagcaacggcaacgtgaccgagagcggctgcaaggagtgcgaggagctggaggagaagaacatcaaggagttcctgcagagcttcgtgcacatcgtgcagatgttcatcaacaccagctccggcggcggctccggcggcggcggctccggcggcggcggctccggcggcggcggctccggcggcggctccctgcaggcccccagaagagccagaggctgcagaaccctgggcctgcccgccctgctgctgctgctgctgctgagaccccccgccaccagaggcatcacctgccccccccccatgagcgtggagcacgccgacatctgggtgaagagctacagcctgtacagcagagagagatacatctgcaacagcggcttcaagagaaaggccggcaccagcagcctgaccgagtgcgtgctgaacaaggccaccaacgtggcccactggaccacccccagcctgaagtgcatcagataagtttaaac

SEQ ID NO: 44 - protein, 1059 aa, Artificial Sequence
  Synthetic Sequence
DRTMALPVTALLLPLALLLHAARPDIQMTQSHKFMSTSVGDRVSITCKASQDVSTAVAWFQQKPGQSPKLLIYSPSYRYTGVPDRFTGSGSGTDFTFTISSVQAEDLAVYYCQQLYSTPYTFGGGTKLEIKGGGGSGGGGSGGGGSEVQLQQSGPELVKPGASVKMSCKASGYTFTDYYLDWVKQSHGESFEWIGRVNPYNGGTIYNQKFKGKATLTVDKSSSTAYMDLNSLTSEDSAVYYCARDHYRYDPLLDYWGQGTTLTVSSTTTPAPRPPTPAPTIASQPLSLRPEACRPAAGGAVHTRGLDFACDIYIWAPLAGTCGVLLLSLVITLYCRSKRSRLLHSDYMNMTPRRPGPTRKHYQPYAPPRDFAAYRSRVKFSRSADAPAYQQGQNQLYNELNLGRREEYDVLDKRRGRDPEMGGKPQRRKNPQEGLYNELQKDKMAEAYSEIGMKGERRRGKGHDGLYQGLSTATKDTYDALHMQALPPRGSGEGRGSLLTCGDVEENPGPMEYASDASLDPEAPWPPAPRARACRVLPWALVAGLLLLLLLAAACAVFLACPWAVSGARASPGSAASPRLREGPELSPDDPAGLLDLRQGMFAQLVAQNVLLIDGPLSWYSDPGLAGVSLTGGLSYKEDTKELVVAKAGVYYVFFQLELRRVVAGEGSGSVSLALHLQPLRSAAGAAALALTVDLPPASSEARNSAFGFQGRLLHLSAGQRLGVHLHTEARARHAWQLTQGATVLGLFRVTPEIPAGLPSPRSEGSGATNFSLLKQAGDVEENPGPMYRMQLLSCIALSLALVTNSGIHVFILGCFSAGLPKTEANWVNVISDLKKIEDLIQSMHIDATLYTESDVHPSCKVTAMKCFLLELQVISLESGDASIHDTVENLIILANNSLSSNGNVTESGCKECEELEEKNIKEFLQSFVHIVQMFINTSSGGGSGGGGSGGGGSGGGGSGGGSLQAPRRARGCRTLGLPALLLLLLLRPPATRGITCPPPMSVEHADIWVKSYSLYSRERYICNSGFKRKAGTSSLTECVLNKATNVAHWTTPSLKCIR

SEQ ID NO: 45 - DNA, 3190 bp, Artificial Sequence
  Synthetic Sequence
gcgatcgcaccatggccctgcccgtgaccgccctgctgctgcccctggccctgctgctgcacgccgccaggcccgacatccagatgacccagagccacaagttcatgagcaccagcgtgggcgacagggtgagcatcacctgcaaggccagccaggacgtgagcaccgccgtggcctggttccagcagaagcccggccagagccccaagctgctgatctacagccccagctacaggtacaccggcgtgcccgacaggttcaccggcagcggcagcggcaccgacttcaccttcaccatcagcagcgtgcaggccgaggacctggccgtgtactactgccagcagctgtacagcaccccctacaccttcggcggcggcaccaagctggagatcaagggaggggggggatccgggggaggaggctccggcggaggcggaagcgaggtgcagctgcagcagagcggccccgagctggtgaagcccggcgccagcgtgaagatgagctgcaaggccagcggctacaccttcaccgactactacctggactgggtgaagcagagccacggcgagagcttcgagtggatcggcagggtgaacccctacaacggcggcaccatctacaaccagaagttcaagggcaaggccaccctgaccgtggacaagagcagcagcaccgcctacatggacctgaacagcctgaccagcgaggacagcgccgtgtactactgcgccagggaccactacaggtacgaccccctgctggactactggggccagggcaccaccctgaccgtgagcagcaccaccacccccgcccccaggccccccacccccgcccccaccatcgccagccagcccctgagcctgaggcccgaggcctgcaggcccgccgccggcggcgccgtgcacaccaggggcctggacttcgcctgcgacatctacatctgggcccccctggccggcacctgcggcgtgctgctgctgagcctggtgatcaccctgtactgcaggagtaagaggagcaggctcctgcacagtgactacatgaacatgactccccgccgccccgggcccacccgcaagcattaccagccctatgccccaccacgcgacttcgcagcctatcgctccagggtgaagttcagcaggagcgccgacgcccccgcctaccagcagggccagaaccagctgtacaacgagctgaacctgggcaggagggaggagtacgacgtgctggacaagaggaggggcagggaccccgagatgggcggcaagccccagaggaggaagaacccccaggagggcctgtacaacgagctgcagaaggacaagatggccgaggcctacagcgagatcggcatgaagggcgagaggaggaggggcaagggccacgacggcctgtaccagggcctgagcaccgccaccaaggacacctacgacgccctgcacatgcaggccctgccccccaggggcagcggcgaaggccgcggcagcctgctgacctgcggcgatgtggaagaaaacccgggccccatggaatacgcctctgacgcttcactggaccccgaagccccgtggcctcccgcgccccgcgctcgcgcctgccgcgtactgccttgggccctggtcgcggggctgctgctgctgctgctgctcgctgccgcctgcgccgtcttcctcgcctgcccctgggccgtgtccggggctcgcgcctcgcccggctccgcggccagcccgagactccgcgagggtcccgagctttcgcccgacgatcccgccggcctcttggacctgcggcagggcatgtttgcgcagctggtggcccaaaatgttctgctgatcgatgggcccctgagctggtacagtgacccaggcctggcaggcgtgtccctgacggggggcctgagctacaaagaggacacgaaggagctggtggtggccaaggctggagtctactatgtcttctttcaactagagctgcggcgcgtggtggccggcgagggctcaggctccgtttcacttgcgctgcacctgcagccactgcgctctgctgctggggccgccgccctggctttgaccgtggacctgccacccgcctcctccgaggctcggaactcggccttcggtttccagggccgcttgctgcacctgagtgccggccagcgcctgggcgtccatcttcacactgaggccagggcacgccatgcctggcagcttacccagggcgccacagtcttgggactcttccgggtgacccccgaaatcccagccggactcccttcaccgaggtcggaaggaagcggagctactaacttcagcctgctgaagcaggctggagacgtggaggagaaccctggacctatgtacagaatgcagctgctgagctgcatcgccctgagcctggccctggtgaccaacagcggcatccacgtgttcatcctgggctgcttcagcgccggcctgcccaagaccgaggccaactgggtgaacgtgatcagcgacctgaagaagatcgaggacctgatccagagcatgcacatcgacgccaccctgtacaccgagagcgacgtgcaccccagctgcaaggtgaccgccatgaagtgcttcctgctggagctgcaggtgatcagcctggagagcggcgacgccagcatccacgacaccgtggagaacctgatcatcctggccaacaacagcctgagcagcaacggcaacgtgaccgagagcggctgcaaggagtgcgaggagctggaggagaagaacatcaaggagttcctgcagagcttcgtgcacatcgtgcagatgttcatcaacaccagctccggcggcggctccggcggcggcggctccggcggcggcggctccggcggcggcggctccggcggcggctccctgcaggcccccagaagagccagaggctgcagaaccctgggcctgcccgccctgctgctgctgctgctgctgagaccccccgccaccagaggcatcacctgccccccccccatgagcgtggagcacgccgacatctgggtgaagagctacagcctgtacagcagagagagatacatctgcaacagcggcttcaagagaaaggccggcaccagcagcctgaccgagtgcgtgctgaacaaggccaccaacgtggcccactggaccacccccagcctgaagtgcatcagataagtttaaac

SEQ ID NO: 46 - protein, 1060 aa, Artificial Sequence
  Synthetic Sequence
DRTMALPVTALLLPLALLLHAARPEIVMTQSPATLSVSPGERATLSCRSSQSLVHRNGNTYLHWYLQKPGQSPKLLIHKVSNRFSGVPDRFSGSGSGTDFTLKISRVEAEDLGVYFCSQSTHVPPLTFGAGTKLELKRGGGGSGGGGSGGGGSEVQLLQSGPELEKPGASVMISCKASGSSFTGYNMNWVRQNIGKSLEWIGAIDPYYGGTSYNQKFKGRATLTVDKSSSTAYMHLKSLTSEDSAVYYCVSGMEYWGQGTSVTVSSTTTPAPRPPTPAPTIASQPLSLRPEACRPAAGGAVHTRGLDFACDIYIWAPLAGTCGVLLLSLVITLYCRSKRSRLLHSDYMNMTPRRPGPTRKHYQPYAPPRDFAAYRSRVKFSRSADAPAYQQGQNQLYNELNLGRREEYDVLDKRRGRDPEMGGKPQRRKNPQEGLYNELQKDKMAEAYSEIGMKGERRRGKGHDGLYQGLSTATKDTYDALHMQALPPRGSGEGRGSLLTCGDVEENPGPMEYASDASLDPEAPWPPAPRARACRVLPWALVAGLLLLLLLAAACAVFLACPWAVSGARASPGSAASPRLREGPELSPDDPAGLLDLRQGMFAQLVAQNVLLIDGPLSWYSDPGLAGVSLTGGLSYKEDTKELVVAKAGVYYVFFQLELRRVVAGEGSGSVSLALHLQPLRSAAGAAALALTVDLPPASSEARNSAFGFQGRLLHLSAGQRLGVHLHTEARARHAWQLTQGATVLGLFRVTPEIPAGLPSPRSEGSGATNFLSLLKQAGDVEENPGPMYRMQLLSCIALSLALVTNSGIHVFILGCFSAGLPKTEANWVNVISDLKKIEDLIQSMHIDATLYTESDVHPSCKVTAMKCFLLELQVISLESGDASIHDTVENLIILANNSLSSNGNVTESGCKECEELEEKNIKEFLQSFVHIVQMFINTSSGGGSGGGGSGGGGSGGGGSGGGSLQAPRRARGCRTLGLPALLLLLLLRPPATRGITCPPPMSVEHADIWVKSYSLYSRERYICNSGFKRKAGTSSLTECVLNKATNVAHWTTPSLKCIR

SEQ ID NO: 47 - DNA, 3182 bp, Artificial Sequence
  Synthetic Sequence
atggccttaccagtgaccgccttgctcctgccgctggccttgctgctccacgccgccaggccggagatcgtgatgacccagagccccgccaccctgagcgtgagccccggcgagagggccaccctgagctgcaggagcagccagagcctggtgcacaggaacggcaacacctacctgcactggtacctgcagaagcccggccagagccccaagctgctgatccacaaggtgagcaacaggttcagcggcgtgcccgacaggttcagcggcagcggcagcggcaccgacttcaccctgaagatcagcagggtggaggccgaggacctgggcgtgtacttctgcagccagagcacccacgtgccccccctgaccttcggcgccggcaccaagctggagctgaagaggggcggcggcggcagcggcggcggcggcagcggcggcggcggcagcgaggtgcagctgctgcagagcggccccgagctggagaagcccggcgccagcgtgatgatcagctgcaaggccagcggcagcagcttcaccggctacaacatgaactgggtgaggcagaacatcggcaagagcctggagtggatcggcgccatcgacccctactacggcggcaccagctacaaccagaagttcaagggcagggccaccctgaccgtggacaagagcagcagcaccgcctacatgcacctgaagagcctgaccagcgaggacagcgccgtgtactactgcgtgagcggcatggagtactggggccagggcaccagcgtgaccgtgagcagcaccacgacgccagcgccgcgaccaccaacaccggcgcccaccatcgcgtcgcagcccctgtccctgcgcccagaggcgtgccggccagcggcggggggcgcagtgcacacgagggggctggacttcgcctgtgatatctacatctgggcgcccttggccgggacttgtggggtccttctcctgtcactggttatcaccctttactgcaggagtaagaggagcaggctcctgcacagtgactacatgaacatgactccccgccgccccgggcccacccgcaagcattaccagccctatgccccaccacgcgacttcgcagcctatcgctccagagtgaagttcagcaggagcgcagacgcccccgcgtaccagcagggccagaaccagctctataacgagctcaatctaggacgaagagaggagtacgatgttttggacaagagacgtggccgggaccctgagatggggggaaagccgcagagaaggaagaaccctcaggaaggcctgtacaatgaactgcagaaagataagatggcggaggcctacagtgagattgggatgaaaggcgagcgccggaggggcaaggggcacgatggcctttaccagggtctcagtacagccaccaaggacacctacgacgcccttcacatgcaggccctgccccctcgcggcagcggcgaaggccgcggcagcctgctgacctgcggcgatgtggaagaaaacccgggccccatggaatacgcctctgacgcttcactggaccccgaagccccgtggcctcccgcgccccgcgctcgcgcctgccgcgtactgccttgggccctggtcgcggggctgctgctgctgctgctgctcgctgccgcctgcgccgtcttcctcgcctgcccctgggccgtgtccggggctcgcgcctcgcccggctccgcggccagcccgagactccgcgagggtcccgagctttcgcccgacgatcccgccggcctcttggacctgcggcagggcatgtttgcgcagctggtggcccaaaatgttctgctgatcgatgggcccctgagctggtacagtgacccaggcctggcaggcgtgtccctgacggggggcctgagctacaaagaggacacgaaggagctggtggtggccaaggctggagtctactatgtcttctttcaactagagctgcggcgcgtggtggccggcgagggctcaggctccgtttcacttgcgctgcacctgcagccactgcgctctgctgctggggccgccgccctggctttgaccgtggacctgccacccgcctcctccgaggctcggaactcggccttcggtttccagggccgcttgctgcacctgagtgccggccagcgcctgggcgtccatcttcacactgaggccagggcacgccatgcctggcagcttacccagggcgccacagtcttgggactcttccgggtgacccccgaaatcccagccggactcccttcaccgaggtcggaaggaagcggagctactaacttcttgagcctgctgaagcaggctggagacgtggaggagaaccctggacctatgtacagaatgcagctgctgagctgcatcgccctgagcctggccctggtgaccaacagcggcatccacgtgttcatcctgggctgcttcagcgccggcctgcccaagaccgaggccaactgggtgaacgtgatcagcgacctgaagaagatcgaggacctgatccagagcatgcacatcgacgccaccctgtacaccgagagcgacgtgcaccccagctgcaaggtgaccgccatgaagtgcttcctgctggagctgcaggtgatcagcctggagagcggcgacgccagcatccacgacaccgtggagaacctgatcatcctggccaacaacagcctgagcagcaacggcaacgtgaccgagagcggctgcaaggagtgcgaggagctggaggagaagaacatcaaggagttcctgcagagcttcgtgcacatcgtgcagatgttcatcaacaccagctccggcggcggctccggcggcggcggctccggcggcggcggctccggcggcggcggctccggcggcggctccctgcaggcccccagaagagccagaggctgcagaaccctgggcctgcccgccctgctgctgctgctgctgctgagaccccccgccaccagaggcatcacctgccccccccccatgagcgtggagcacgccgacatctgggtgaagagctacagcctgtacagcagagagagatacatctgcaacagcggcttcaagagaaaggccggcaccagcagcctgaccgagtgcgtgctgaacaaggccaccaacgtggcccactggaccacccccagcctgaagtgcatcagataagtttaaac

SEQ ID NO: 48 - protein, 880 aa, Artificial Sequence
  Synthetic Sequence
RSLTSRMYLWLKLLAFGFAFLDTEVFVTGDIQVTQSPSSLSASLGERISLTCRTSQDISNYLNWFQQKPDGTFKRLIYATSSLDSGVPKRFSGSGSGSDYSLTISSLESEDFADYYCLQYASYPFTFGSGTKLEIKGGGGSGGGGSGGGGSEVQLQESGPGLVKPSQTLSLTCSVTGYSITSGYYWHWIRQFPGNKLQWMGYISYSGFTNYKTSLINRISITHDTSENQFFLNLNSVTTEDTATYYCAGDRTGSWFAYWGQGTLVTVSATTTPAPRPPTPAPTIASQPLSLRPEACRPAAGGAVHTRGLDFACDIYIWAPLAGTCGVLLLSLVITLYCRSKRSRLLHSDYMNMTPRRPGPTRKHYQPYAPPRDFAAYRSRVKFSRSADAPAYQQGQNQLYNELNLGRREEYDVLDKRRGRDPEMGGKPQRRKNPQEGLYNELQKDKMAEAYSEIGMKGERRRGKGHDGLYQGLSTATKDTYDALHMQALPPRGSGEGRGSLLTCGDVEENPGPMYLWLKLLAFGFAFLDTEVFVTGGQNDTSQTSSPSSPLFPGPSKPFWVLVVVGGVLACYSLLVTVAFIIFWVGSGATNFSLLKQAGDVEENPGPMYRMQLLSCIALSLALVTNSGIHVFILGCFSAGLPKTEANWVNVISDLKKIEDLIQSMHIDATLYTESDVHPSCKVTAMKCFLLELQVISLESGDASIHDTVENLIILANNSLSSNGNVTESGCKECEELEEKNIKEFLQSFVHIVQMFINTSSGGGSGGGGSGGGGSGGGGSGGGSLQAPRRARGCRTLGLPALLLLLLLRPPATRGITCPPPMSVEHADIWVKSYSLYSRERYICNSGFKRKAGTSSLTECVLNKATNVAHWTTPSLKCIR

SEQ ID NO: 49 - DNA, 2633 bp, Artificial Sequence
  Synthetic Sequence
atgtatttgtggcttaaactcttggcatttggctttgcctttctggacacagaagtatttgtgacaggggacatccaggtgacccagagccccagcagcctgagcgccagcctgggcgagagaatcagcctgacctgcagaaccagccaggacatcagcaactacctgaactggttccagcagaagcccgacggcaccttcaagagactgatctacgccaccagcagcctggacagcggcgtgcccaagagattcagcggcagcggcagcggcagcgactacagcctgaccatcagcagcctggagagcgaggacttcgccgactactactgcctgcagtacgccagctaccccttcaccttcggcagcggcaccaagctggagatcaagggaggggggggatccgggggaggaggctccggcggaggcggaagcgaggtgcagctgcaggagagcggccccggcctggtgaagcccagccagaccctgagcctgacctgcagcgtgaccggctacagcatcaccagcggctactactggcactggatcagacagttccccggcaacaagctgcagtggatgggctacatcagctacagcggcttcaccaactacaagaccagcctgatcaacagaatcagcatcacccacgacaccagcgagaaccagttcttcctgaacctgaacagcgtgaccaccgaggacaccgccacctactactgcgccggcgacagaaccggcagctggttcgcctactggggccagggcaccctggtgaccgtgagcgccaccacgacgccagcgccgcgaccaccaacaccggcgcccaccatcgcgtcgcagcccctgtccctgcgcccagaggcgtgccggccagcggcggggggcgcagtgcacacgagggggctggacttcgcctgtgatatctacatctgggcgcccttggccgggacttgtggggtccttctcctgtcactggttatcaccctttactgcaggagtaagaggagcaggctcctgcacagtgactacatgaacatgactccccgccgccccgggcccacccgcaagcattaccagccctatgccccaccacgcgacttcgcagcctatcgctccagagtgaagttcagcaggagcgcagacgcccccgcgtaccagcagggccagaaccagctctataacgagctcaatctaggacgaagagaggagtacgatgttttggacaagagacgtggccgggaccctgagatggggggaaagccgcagagaaggaagaaccctcaggaaggcctgtacaatgaactgcagaaagataagatggcggaggcctacagtgagattgggatgaaaggcgagcgccggaggggcaaggggcacgatggcctttaccagggtctcagtacagccaccaaggacacctacgacgcccttcacatgcaggccctgccccctcgcggcagcggcgaaggccgcggcagcctgctgacctgcggcgatgtggaagaaaacccgggccccatgtacctgtggctgaagctgctggccttcggcttcgccttcctggacaccgaggtgttcgtgaccggcggccagaacgacaccagccagaccagcagccccagcagcccgctgtttccgggcccgagcaaaccgttttgggtgctggtggtggtgggcggcgtgctggcgtgctatagcctgctggtgaccgtggcgtttattattttttgggtgggaagcggagctactaacttcagcctgctgaagcaggctggagacgtggaggagaaccctggacctatgtacagaatgcagctgctgagctgcatcgccctgagcctggccctggtgaccaacagcggcatccacgtgttcatcctgggctgcttcagcgccggcctgcccaagaccgaggccaactgggtgaacgtgatcagcgacctgaagaagatcgaggacctgatccagagcatgcacatcgacgccaccctgtacaccgagagcgacgtgcaccccagctgcaaggtgaccgccatgaagtgcttcctgctggagctgcaggtgatcagcctggagagcggcgacgccagcatccacgacaccgtggagaacctgatcatcctggccaacaacagcctgagcagcaacggcaacgtgaccgagagcggctgcaaggagtgcgaggagctggaggagaagaacatcaaggagttcctgcagagcttcgtgcacatcgtgcagatgttcatcaacaccagctccggcggcggctccggcggcggcggctccggcggcggcggctccggcggcggcggctccggcggcggctccctgcaggcccccagaagagccagaggctgcagaaccctgggcctgcccgccctgctgctgctgctgctgctgagaccccccgccaccagaggcatcacctgccccccccccatgagcgtggagcacgccgacatctgggtgaagagctacagcctgtacagcagagagagatacatctgcaacagcggcttcaagagaaaggccggcaccagcagcctgaccgagtgcgtgctgaacaaggccaccaacgtggcccactggaccacccccagcctgaagtgcatcagataagtttaaac

SEQ ID NO: 50 - protein, 1099 aa, Artificial Sequence
  Synthetic Sequence
DRTMALPVTALLLPLALLLHAARPDVVMTQSHRFMSTSVGDRVSITCRASQDVNTAVSWYQQKPGQSPKLLIFSASYRYTGVPDRFTGSGSGADFTLTISSVQAEDLAVYYCQQHYSTPWTFGGGTKLDIKGGGGSGGGGSGGGGSQIQLVQSGPDLKKPGETVKLSCKASGYTFTNFGMNWVKQAPGKGFKWMAWINTYTGESYFADDFKGRFAFSVETSATTAYLQINNLKTEDTATYFCARGEIYYGYDGGFAYWGQGTLVTVSATTTPAPRPPTPAPTIASQPLSLRPEACRPAAGGAVHTRGLDFACDIYIWAPLAGTCGVLLLSLVITLYCRSKRSRLLHSDYMNMTPRRPGPTRKHYQPYAPPRDFAAYRSRVKFSRSADAPAYQQGQNQLYNELNLGRREEYDVLDKRRGRDPEMGGKPQRRKNPQEGLYNELQKDKMAEAYSEIGMKGERRRGKGHDGLYQGLSTATKDTYDALHMQALPPRGSGATNFSLLKQAGDVEENPGPMEYASDASLDPEAPWPPAPRARACRVLPWALVAGLLLLLLLAAACAVFLACPWAVSGARASPGSAASPRLREGPELSPDDPAGLLDLRQGMFAQLVAQNVLLIDGPLSWYSDPGLAGVSLTGGLSYKEDTKELVVAKAGVYYVFFQLELRRVVAGEGSGSVSLALHLQPLRSAAGAAALALTVDLPPASSEARNSAFGFQGRLLHLSAGQRLGVHLHTEARARHAWQLTQGATVLGLFRVTPEIPAGLPSPRSEGSGEGRGSLLTCGDVEENPGPMYRMQLLSCIALSLALVTNSGIHVFILGCFSAGLPKTEANWVNVISDLKKIEDLIQSMHIDATLYTESDVHPSCKVTAMKCFLLELQVISLESGDASIHDTVENLIILANNSLSSNGNVTESGCKECEELEEKNIKEFLQSFVHIVQMFINTSSGGGSGGGGSGGGGSGGGGSGGGSLQITCPPPMSVEHADIWVKSYSLYSRERYICNSGFKRKAGTSSLTECVLNKATNVAHWTTPSLKCIRTTTPAPRPPTPAPTIASQPLSLRPEACRPAAGGAVHTRGLDFACDVAISTSTVLLCGLSAVSLLACY

SEQ ID NO: 51 - DNA, 3299 bp, Artificial Sequence
  Synthetic Sequence
atggccttaccagtgaccgccttgctcctgccgctggccttgctgctccacgccgccaggccggacgtggtgatgacccagagccacaggttcatgagcaccagcgtgggcgacagggtgagcatcacctgcagggccagccaggacgtgaacaccgccgtgagctggtaccagcagaagcccggccagagccccaagctgctgatcttcagcgccagctacaggtacaccggcgtgcccgacaggttcaccggcagcggcagcggcgccgacttcaccctgaccatcagcagcgtgcaggccgaggacctggccgtgtactactgccagcagcactacagcaccccctggaccttcggcggcggcaccaagctggacatcaagggaggggggggatccgggggaggaggctccggcggaggcggaagccagatccagctggtgcagagcggccccgacctgaagaagcccggcgagaccgtgaagctgagctgcaaggccagcggctacaccttcaccaacttcggcatgaactgggtgaagcaggcccccggcaagggcttcaagtggatggcctggatcaacacctacaccggcgagagctacttcgccgacgacttcaagggcaggttcgccttcagcgtggagaccagcgccaccaccgcctacctgcagatcaacaacctgaagaccgaggacaccgccacctacttctgcgccaggggcgagatctactacggctacgacggcggcttcgcctactggggccagggcaccctggtgaccgtgagcgccaccacgacgccagcgccgcgaccaccaacaccggcgcccaccatcgcgtcgcagcccctgtccctgcgcccagaggcgtgccggccagcggcggggggcgcagtgcacacgagggggctggacttcgcctgtgatatctacatctgggcgcccttggccgggacttgtggggtccttctcctgtcactggttatcaccctttactgcaggagtaagaggagcaggctcctgcacagtgactacatgaacatgactccccgccgccccgggcccacccgcaagcattaccagccctatgccccaccacgcgacttcgcagcctatcgctccagagtgaagttcagcaggagcgcagacgcccccgcgtaccagcagggccagaaccagctctataacgagctcaatctaggacgaagagaggagtacgatgttttggacaagagacgtggccgggaccctgagatggggggaaagccgcagagaaggaagaaccctcaggaaggcctgtacaatgaactgcagaaagataagatggcggaggcctacagtgagattgggatgaaaggcgagcgccggaggggcaaggggcacgatggcctttaccagggtctcagtacagccaccaaggacacctacgacgcccttcacatgcaggccctgccccctcgcggaagcggagccaccaacttcagcctgctgaagcaggccggcgacgtggaggagaaccccggccccatggaatacgcctctgacgcttcactggaccccgaagccccgtggcctcccgcgccccgcgctcgcgcctgccgcgtactgccttgggccctggtcgcggggctgctgctgctgctgctgctcgctgccgcctgcgccgtcttcctcgcctgcccctgggccgtgtccggggctcgcgcctcgcccggctccgcggccagcccgagactccgcgagggtcccgagctttcgcccgacgatcccgccggcctcttggacctgcggcagggcatgtttgcgcagctggtggcccaaaatgttctgctgatcgatgggcccctgagctggtacagtgacccaggcctggcaggcgtgtccctgacggggggcctgagctacaaagaggacacgaaggagctggtggtggccaaggctggagtctactatgtcttctttcaactagagctgcggcgcgtggtggccggcgagggctcaggctccgtttcacttgcgctgcacctgcagccactgcgctctgctgctggggccgccgccctggctttgaccgtggacctgccacccgcctcctccgaggctcggaactcggccttcggtttccagggccgcttgctgcacctgagtgccggccagcgcctgggcgtccatcttcacactgaggccagggcacgccatgcctggcagcttacccagggcgccacagtcttgggactcttccgggtgacccccgaaatcccagccggactcccttcaccgaggtcggaaggcagcggcgaaggccgcggcagcctgctgacctgcggcgatgtggaagaaaacccgggccccatgtacagaatgcagctgctgagctgcatcgccctgagcctggccctggtgaccaacagcggcatccacgtgttcatcctgggctgcttcagcgccggcctgcccaagaccgaggccaactgggtgaacgtgatcagcgacctgaagaagatcgaggacctgatccagagcatgcacatcgacgccaccctgtacaccgagagcgacgtgcaccccagctgcaaggtgaccgccatgaagtgcttcctgctggagctgcaggtgatcagcctggagagcggcgacgccagcatccacgacaccgtggagaacctgatcatcctggccaacaacagcctgagcagcaacggcaacgtgaccgagagcggctgcaaggagtgcgaggagctggaggagaagaacatcaaggagttcctgcagagcttcgtgcacatcgtgcagatgttcatcaacaccagctccggcggcggctccggcggcggcggctccggcggcggcggctccggcggcggcggctccggcggcggctccctgcagatcacctgccccccccccatgagcgtggagcacgccgacatctgggtgaagagctacagcctgtacagcagagagagatacatctgcaacagcggcttcaagagaaaggccggcaccagcagcctgaccgagtgcgtgctgaacaaggccaccaacgtggcccactggaccacccccagcctgaagtgcatcagaaccaccacccccgcccccaggccccccacccccgcccccaccatcgccagccagcccctgagcctgaggcccgaggcctgcaggcccgccgccggcggcgccgtgcacaccaggggcctggacttcgcctgcgacgtggctatctccacgtccactgtcctgctgtgtgggctgagcgctgtgtctctcctggcatgctactaagtttaaac

SEQ ID NO: 52 - protein, 1006 aa, Artificial Sequence
  Synthetic Sequence
DRTMALPVTALLLPLALLLHAARPDIQLTQSPSSLSASVGDRVTMTCRASSSVSYIHWFQQKPGKAPKPWIYATSNLASGVPVRFSGSGSGTDYTFTISSLQPEDIATYYCQQWTSNPPTFGGGTKLEIKRGGGGSGGGGSGGGGSQVQLQQSGAEVKKPGSSVKVSCKASGYTFSSYNMHWVRQAPGQGLEWMGAIYPGNGDTSYNQKFKGRATITADESTNTAYMELSSLRSEDTAFYFCARSTYYGGDWYFDVWGQGTTVTVSSTTTPAPRPPTPAPTIASQPLSLRPEACRPAAGGAVHTRGLDFACDIYIWAPLAGTCGVLLLSLVITLYCRSKRSRLLHSDYMNMTPRRPGPTRKHYQPYAPPRDFAAYRSRVKFSRSADAPAYQQGQNQLYNELNLGRREEYDVLDKRRGRDPEMGGKPQRRKNPQEGLYNELQKDKMAEAYSEIGMKGERRRGKGHDGLYQGLSTATKDTYDALHMQALPPRGSGATNFSLLKQAGDVEENPGPMALPVTALLLPLALLLHAARPEVQLQQSGPELIKPGASVKMSCKASGYTFTSYVMHWVKQKPGQGLEWIGYINPYNDGTKYNEKFKGKATLTSDKSSSTAYMELSSLTSEDSAVYYCARGTYYYGSRVFDYWGQGTTLTVSSGGGGSGGGGSGGGGSDIVMTQAAPSIPVTPGESVSISCRSSKSLLNSNGNTYLYWFLQRPGQSPQLLIYRMSNLASGVPDRFSGSGSGTAFTLRISRVEAEDVGVYYCMQHLEYPFTFGAGTKLELKRTTTPAPRPPTPAPTIASQPLSLRPEACRPAAGGAVHTRGLDFACDIYIWAPLAGTCGVLLLSLVITLYCKRGRKKLLYIFKQPFMRPVQTTQEEDGCSCRFPEEEEGGCELRVKFSRSADAPAYQQGQNQLYNELNLGRREEYDVLDKRRGRDPEMGGKPQRRKNPQEGLYNELQKDKMAEAYSEIGMKGERRRGKGHDGLYQGLSTATKDTYDALHMQALPPR

SEQ ID NO: 53 - DNA, 3020 bp, Artificial Sequence
  Synthetic Sequence
atggccttaccagtgaccgccttgctcctgccgctggccttgctgctccacgccgccaggccggacatccagctgacccagagccccagcagcctgagcgccagcgtgggcgacagggtgaccatgacctgcagggccagcagcagcgtgagctacatccactggttccagcagaagcccggcaaggcccccaagccctggatctacgccaccagcaacctggccagcggcgtgcccgtgaggttcagcggcagcggcagcggcaccgactacaccttcaccatcagcagcctgcagcccgaggacatcgccacctactactgccagcagtggaccagcaacccccccaccttcggcggcggcaccaagctggagatcaagaggggcggcggcggcagcggcggcggcggcagcggcggcggcggcagccaggtgcagctgcagcagagcggcgccgaggtgaagaagcccggcagcagcgtgaaggtgagctgcaaggccagcggctacaccttcagcagctacaacatgcactgggtgaggcaggcccccggccagggcctggagtggatgggcgccatctaccccggcaacggcgacaccagctacaaccagaagttcaagggcagggccaccatcaccgccgacgagagcaccaacaccgcctacatggagctgagcagcctgaggagcgaggacaccgccttctacttctgcgccaggagcacctactacggcggcgactggtacttcgacgtgtggggccagggcaccaccgtgaccgtgagcagcaccacgacgccagcgccgcgaccaccaacaccggcgcccaccatcgcgtcgcagcccctgtccctgcgcccagaggcgtgccggccagcggcggggggcgcagtgcacacgagggggctggacttcgcctgtgatatctacatctgggcgcccttggccgggacttgtggggtccttctcctgtcactggttatcaccctttactgcaggagtaagaggagcaggctcctgcacagtgactacatgaacatgactccccgccgccccgggcccacccgcaagcattaccagccctatgccccaccacgcgacttcgcagcctatcgctccagagtgaagttcagcaggagcgcagacgcccccgcgtaccagcagggccagaaccagctctataacgagctcaatctaggacgaagagaggagtacgatgttttggacaagagacgtggccgggaccctgagatggggggaaagccgcagagaaggaagaaccctcaggaaggcctgtacaatgaactgcagaaagataagatggcggaggcctacagtgagattgggatgaaaggcgagcgccggaggggcaaggggcacgatggcctttaccagggtctcagtacagccaccaaggacacctacgacgcccttcacatgcaggccctgccccctcgcggaagcggagccaccaacttcagcctgctgaagcaggccggcgacgtggaggagaaccccggccccatggccctgcccgtgaccgccctgctgctgcccctggccctgctgctgcacgccgccaggcccgaggtccagctgcagcagtctggacctgagctgataaagcctggggcttcagtgaagatgtcctgcaaggcttctggatacacattcactagctatgttatgcactgggtgaagcagaagcctgggcagggccttgagtggattggatatattaatccttacaatgatggtactaagtacaatgagaagttcaaaggcaaggccacactgacttcagacaaatcctccagcacagcctacatggagctcagcagcctgacctctgaggactctgcggtctattactgtgcaagagggacttattactacggtagtagggtatttgactactggggccaaggcaccactctcacagtctcctcaggtggagggggctcaggcggaggtggctctgggggtggaggctcggacattgtgatgactcaggctgcaccctctatacctgtcactcctggagagtcagtatccatctcctgcaggtctagtaagagtctcctgaatagtaatggcaacacttacttgtattggttcctgcagaggccaggccagtctcctcagctcctgatatatcggatgtccaaccttgcctcaggagtcccagacaggttcagtggcagtgggtcaggaactgctttcacactgagaatcagtagagtggaggctgaggatgtgggtgtttattactgtatgcaacatctagaatatccgttcacgttcggtgctgggaccaagctggagctgaaacggaccaccacccccgcccccaggccccccacccccgcccccaccatcgccagccagcccctgagcctgaggcccgaggcctgcaggcccgccgccggcggcgccgtgcacaccaggggcctggacttcgcctgcgacatctacatctgggcccccctggccggcacctgcggcgtgctgctgctgagcctggtgatcaccctgtactgcaaacggggcagaaagaaactcctgtatatattcaaacaaccatttatgagaccagtacaaactactcaagaggaagatggctgtagctgccgatttccagaagaagaagaaggaggatgtgaactgagggtgaagttcagcaggagcgccgacgcccccgcctaccagcagggccagaaccagctgtacaacgagctgaacctgggcaggagggaggagtacgacgtgctggacaagaggaggggcagggaccccgagatgggcggcaagccccagaggaggaagaacccccaggagggcctgtacaacgagctgcagaaggacaagatggccgaggcctacagcgagatcggcatgaagggcgagaggaggaggggcaagggccacgacggcctgtaccagggcctgagcaccgccaccaaggacacctacgacgccctgcacatgcaggccctgccccccaggtaagtttaaac

SEQ ID NO: 54 - protein, 784 aa, Artificial Sequence
  Synthetic Sequence
MALPVTALLLPLALLLHAARPDIVLTQSPASLAVSLGQRATISCRASKSVSTSGYSYLHWYQQKPGQPPKLLIYLASNLESGVPARFSGSGSGTDFTLNIHPVEEEDAATYYCQHSRELPFTFGSGTKLEIKGGGGSGGGGSGGGGSQVQLVESGGGLVQPGGSLKLSCAASGFDFSRYWMSWVRQAPGKGLEWIGEINPTSSTINFTPSLKDKVFISRDNAKNTLYLQMSKVRSEDTALYYCARGNYYRYGDAMDYWGQGTSVTVSTTTPAPRPPTPAPTIASQPLSLRPEACRPAAGGAVHTRGLDFACDIYIWAPLAGTCGVLLLSLVITLYCRSKRSRLLHSDYMNMTPRRPGPTRKHYQPYAPPRDFAAYRSRVKFSRSADAPAYQQGQNQLYNELNLGRREEYDVLDKRRGRDPEMGGKPQRRKNPQEGLYNELQKDKMAEAYSEIGMKGERRRGKGHDGLYQGLSTATKDTYDALHMQALPPRGSGEGRGSLLTCGDVEENPGPMYRMQLLSCIALSLALVTNSGIHVFILGCFSAGLPKTEANWVNVISDLKKIEDLIQSMHIDATLYTESDVHPSCKVTAMKCFLLELQVISLESGDASIHDTVENLIILANNSLSSNGNVTESGCKECEELEEKNIKEFLQSFVHIVQMFINTSSGGGSGGGGSGGGGSGGGGSGGGSLQAPRRARGCRTLGLPALLLLLLLRPPATRGITCPPPMSVEHADIWVKSYSLYSRERYICNSGFKRKAGTSSLTECVLNKATNVAHWTTPSLKCIR

SEQ ID NO: 55 - DNA, 2363 bp, Artificial Sequence
  Synthetic Sequence
atggccttaccagtgaccgccttgctcctgccgctggccttgctgctccacgccgccaggccggacatcgtgctgacccagagccccgccagcctggccgtgagcctgggccagagggccaccatcagctgcagggccagcaagagcgtgagcaccagcggctacagctacctgcactggtaccagcagaagcccggccagccccccaagctgctgatctacctggccagcaacctggagagcggcgtgcccgccaggttcagcggcagcggcagcggcaccgacttcaccctgaacatccaccccgtggaggaggaggacgccgccacctactactgccagcacagcagggagctgcccttcaccttcggcagcggcaccaagctggagatcaagggaggggggggatccgggggaggaggctccggcggaggcggaagccaggtgcagctggtggagagcggcggcggcctggtgcagcccggcggcagcctgaagctgagctgcgccgccagcggcttcgacttcagcaggtactggatgagctgggtgaggcaggcccccggcaagggcctggagtggatcggcgagatcaaccccaccagcagcaccatcaacttcacccccagcctgaaggacaaggtgttcatcagcagggacaacgccaagaacaccctgtacctgcagatgagcaaggtgaggagcgaggacaccgccctgtactactgcgccaggggcaactactacaggtacggcgacgccatggactactggggccagggcaccagcgtgaccgtgagcaccacgacgccagcgccgcgaccaccaacaccggcgcccaccatcgcgtcgcagcccctgtccctgcgcccagaggcgtgccggccagcggcggggggcgcagtgcacacgagggggctggacttcgcctgtgatatctacatctgggcgcccttggccgggacttgtggggtccttctcctgtcactggttatcaccctttactgcaggagtaagaggagcaggctcctgcacagtgactacatgaacatgactccccgccgccccgggcccacccgcaagcattaccagccctatgccccaccacgcgacttcgcagcctatcgctccagagtgaagttcagcaggagcgcagacgcccccgcgtaccagcagggccagaaccagctctataacgagctcaatctaggacgaagagaggagtacgatgttttggacaagagacgtggccgggaccctgagatggggggaaagccgcagagaaggaagaaccctcaggaaggcctgtacaatgaactgcagaaagataagatggcggaggcctacagtgagattgggatgaaaggcgagcgccggaggggcaaggggcacgatggcctttaccagggtctcagtacagccaccaaggacacctacgacgcccttcacatgcaggccctgccccctcgcggcagcggcgaaggccgcggcagcctgctgacctgcggcgatgtggaagaaaacccgggccccatgtacagaatgcagctgctgagctgcatcgccctgagcctggccctggtgaccaacagcggcatccacgtgttcatcctgggctgcttcagcgccggcctgcccaagaccgaggccaactgggtgaacgtgatcagcgacctgaagaagatcgaggacctgatccagagcatgcacatcgacgccaccctgtacaccgagagcgacgtgcaccccagctgcaaggtgaccgccatgaagtgcttcctgctggagctgcaggtgatcagcctggagagcggcgacgccagcatccacgacaccgtggagaacctgatcatcctggccaacaacagcctgagcagcaacggcaacgtgaccgagagcggctgcaaggagtgcgaggagctggaggagaagaacatcaaggagttcctgcagagcttcgtgcacatcgtgcagatgttcatcaacaccagctccggcggcggctccggcggcggcggctccggcggcggcggctccggcggcggcggctccggcggcggctccctgcaggcccccagaagagccagaggctgcagaaccctgggcctgcccgccctgctgctgctgctgctgctgagaccccccgccaccagaggcatcacctgccccccccccatgagcgtggagcacgccgacatctgggtgaagagctacagcctgtacagcagagagagatacatctgcaacagcggcttcaagagaaaggccggcaccagcagcctgaccgagtgcgtgctgaacaaggccaccaacgtggcccactggaccacccccagcctgaagtgcatcagataagtttaaac

SEQ ID NO: 56 - protein, 489 aa, Artificial Sequence
  Synthetic Sequence
DRTMALPVTALLLPLALLLHAARPEIVMTQSPATLSVSPGERATLSCRSSQSLVHRNGNTYLHWYLQKPGQSPKLLIHKVSNRFSGVPDRFSGSGSGTDFTLKISRVEAEDLGVYFCSQSTHVPPLTFGAGTKLELKRGGGGSGGGGSGGGGSEVQLLQSGPELEKPGASVMISCKASGSSFTGYNMNWVRQNIGKSLEWIGAIDPYYGGTSYNQKFKGRATLTVDKSSSTAYMHLKSLTSEDSAVYYCVSGMEYWGQGTSVTVSSTTTPAPRPPTPAPTIASQPLSLRPEACRPAAGGAVHTRGLDFACDIYIWAPLAGTCGVLLLSLVITLYCRSKRSRLLHSDYMNMTPRRPGPTRKHYQPYAPPRDFAAYRSRVKFSRSADAPAYQQGQNQLYNELNLGRREEYDVLDKRRGRDPEMGGKPQRRKNPQEGLYNELQKDKMAEAYSEIGMKGERRRGKGHDGLYQGLSTATKDTYDALHMQALPPR

SEQ ID NO: 57 - DNA, 1480 bp, Artificial Sequence
  Synthetic Sequence
gcgatcgcaccatggccttaccagtgaccgccttgctcctgccgctggccttgctgctccacgccgccaggccggagatcgtgatgacccagagccccgccaccctgagcgtgagccccggcgagagggccaccctgagctgcaggagcagccagagcctggtgcacaggaacggcaacacctacctgcactggtacctgcagaagcccggccagagccccaagctgctgatccacaaggtgagcaacaggttcagcggcgtgcccgacaggttcagcggcagcggcagcggcaccgacttcaccctgaagatcagcagggtggaggccgaggacctgggcgtgtacttctgcagccagagcacccacgtgccccccctgaccttcggcgccggcaccaagctggagctgaagaggggcggcggcggcagcggcggcggcggcagcggcggcggcggcagcgaggtgcagctgctgcagagcggccccgagctggagaagcccggcgccagcgtgatgatcagctgcaaggccagcggcagcagcttcaccggctacaacatgaactgggtgaggcagaacatcggcaagagcctggagtggatcggcgccatcgacccctactacggcggcaccagctacaaccagaagttcaagggcagggccaccctgaccgtggacaagagcagcagcaccgcctacatgcacctgaagagcctgaccagcgaggacagcgccgtgtactactgcgtgagcggcatggagtactggggccagggcaccagcgtgaccgtgagcagcaccacgacgccagcgccgcgaccaccaacaccggcgcccaccatcgcgtcgcagcccctgtccctgcgcccagaggcgtgccggccagcggcggggggcgcagtgcacacgagggggctggacttcgcctgtgatatctacatctgggcgcccttggccgggacttgtggggtccttctcctgtcactggttatcaccctttactgcaggagtaagaggagcaggctcctgcacagtgactacatgaacatgactccccgccgccccgggcccacccgcaagcattaccagccctatgccccaccacgcgacttcgcagcctatcgctccagagtgaagttcagcaggagcgcagacgcccccgcgtaccagcagggccagaaccagctctataacgagctcaatctaggacgaagagaggagtacgatgttttggacaagagacgtggccgggaccctgagatggggggaaagccgcagagaaggaagaaccctcaggaaggcctgtacaatgaactgcagaaagataagatggcggaggcctacagtgagattgggatgaaaggcgagcgccggaggggcaaggggcacgatggcctttaccagggtctcagtacagccaccaaggacacctacgacgcccttcacatgcaggccctgccccctcgctaagtttaaac

SEQ ID NO: 58 - protein, 764 aa, Artificial Sequence
  Synthetic Sequence
DRTMALPVTALLLPLALLLHAARPEIVMTQSPATLSVSPGERATLSCRSSQSLVHRNGNTYLHWYLQKPGQSPKLLIHKVSNRFSGVPDRFSGSGSGTDFTLKISRVEAEDLGVYFCSQSTHVPPLTFGAGTKLELKRGGGGSGGGGSGGGGSEVQLLQSGPELEKPGASVMISCKASGSSFTGYNMNWVRQNIGKSLEWIGAIDPYYGGTSYNQKFKGRATLTVDKSSSTAYMHLKSLTSEDSAVYYCVSGMEYWGQGTSVTVSSTTTPAPRPPTPAPTIASQPLSLRPEACRPAAGGAVHTRGLDFACDIYIWAPLAGTCGVLLLSLVITLYCRSKRSRLLHSDYMNMTPRRPGPTRKHYQPYAPPRDFAAYRSRVKFSRSADAPAYQQGQNQLYNELNLGRREEYDVLDKRRGRDPEMGGKPQRRKNPQEGLYNELQKDKMAEAYSEIGMKGERRRGKGHDGLYQGLSTATKDTYDALHMQALPPRGSGEGRGSLLTCGDVEENPGPMEYASDASLDPEAPWPPAPRARACRVLPWALVAGLLLLLLLAAACAVFLACPWAVSGARASPGSAASPRLREGPELSPDDPAGLLDLRQGMFAQLVAQNVLLIDGPLSWYSDPGLAGVSLTGGLSYKEDTKELVVAKAGVYYVFFQLELRRVVAGEGSGSVSLALHLQPLRSAAGAAALALTVDLPPASSEARNSAFGFQGRLLHLSAGQRLGVHLHTEARARHAWQLTQGATVLGLFRVTPEIPAGLPSPRSE

SEQ ID NO: 59 - DNA, 2294 bp, Artificial Sequence
  Synthetic Sequence
atggccttaccagtgaccgccttgctcctgccgctggccttgctgctccacgccgccaggccggagatcgtgatgacccagagccccgccaccctgagcgtgagccccggcgagagggccaccctgagctgcaggagcagccagagcctggtgcacaggaacggcaacacctacctgcactggtacctgcagaagcccggccagagccccaagctgctgatccacaaggtgagcaacaggttcagcggcgtgcccgacaggttcagcggcagcggcagcggcaccgacttcaccctgaagatcagcagggtggaggccgaggacctgggcgtgtacttctgcagccagagcacccacgtgccccccctgaccttcggcgccggcaccaagctggagctgaagaggggcggcggcggcagcggcggcggcggcagcggcggcggcggcagcgaggtgcagctgctgcagagcggccccgagctggagaagcccggcgccagcgtgatgatcagctgcaaggccagcggcagcagcttcaccggctacaacatgaactgggtgaggcagaacatcggcaagagcctggagtggatcggcgccatcgacccctactacggcggcaccagctacaaccagaagttcaagggcagggccaccctgaccgtggacaagagcagcagcaccgcctacatgcacctgaagagcctgaccagcgaggacagcgccgtgtactactgcgtgagcggcatggagtactggggccagggcaccagcgtgaccgtgagcagcaccacgacgccagcgccgcgaccaccaacaccggcgcccaccatcgcgtcgcagcccctgtccctgcgcccagaggcgtgccggccagcggcggggggcgcagtgcacacgagggggctggacttcgcctgtgatatctacatctgggcgcccttggccgggacttgtggggtccttctcctgtcactggttatcaccctttactgcaggagtaagaggagcaggctcctgcacagtgactacatgaacatgactccccgccgccccgggcccacccgcaagcattaccagccctatgccccaccacgcgacttcgcagcctatcgctccagagtgaagttcagcaggagcgcagacgcccccgcgtaccagcagggccagaaccagctctataacgagctcaatctaggacgaagagaggagtacgatgttttggacaagagacgtggccgggaccctgagatggggggaaagccgcagagaaggaagaaccctcaggaaggcctgtacaatgaactgcagaaagataagatggcggaggcctacagtgagattgggatgaaaggcgagcgccggaggggcaaggggcacgatggcctttaccagggtctcagtacagccaccaaggacacctacgacgcccttcacatgcaggccctgccccctcgcggcagcggcgaaggccgcggcagcctgctgacctgcggcgatgtggaagaaaacccgggccccatggaatacgcctctgacgcttcactggaccccgaagccccgtggcctcccgcgccccgcgctcgcgcctgccgcgtactgccttgggccctggtcgcggggctgctgctgctgctgctgctcgctgccgcctgcgccgtcttcctcgcctgcccctgggccgtgtccggggctcgcgcctcgcccggctccgcggccagcccgagactccgcgagggtcccgagctttcgcccgacgatcccgccggcctcttggacctgcggcagggcatgtttgcgcagctggtggcccaaaatgttctgctgatcgatgggcccctgagctggtacagtgacccaggcctggcaggcgtgtccctgacggggggcctgagctacaaagaggacacgaaggagctggtggtggccaaggctggagtctactatgtcttctttcaactagagctgcggcgcgtggtggccggcgagggctcaggctccgtttcacttgcgctgcacctgcagccactgcgctctgctgctggggccgccgccctggctttgaccgtggacctgccacccgcctcctccgaggctcggaactcggccttcggtttccagggccgcttgctgcacctgagtgccggccagcgcctgggcgtccatcttcacactgaggccagggcacgccatgcctggcagcttacccagggcgccacagtcttgggactcttccgggtgacccccgaaatcccagccggactcccttcaccgaggtcggaataagtttaaac

SEQ ID NO: 60 - protein, 1302 aa, Artificial Sequence
  Synthetic Sequence
DRTMALPVTALLLPLALLLHAARPDIQMTQSHKFMSTSVGDRVSITCKASQDVSTAVAWFQQKPGQSPKLLIYSPSYRYTGVPDRFTGSGSGTDFTFTISSVQAEDLAVYYCQQLYSTPYTFGGGTKLEIKGGGGSGGGGSGGGGSEVQLQQSGPELVKPGASVKMSCKASGYTFTDYYLDWVKQSHGESFEWIGRVNPYNGGTIYNQKFKGKATLTVDKSSSTAYMDLNSLTSEDSAVYYCARDHYRYDPLLDYWGQGTTLTVSSTTTPAPRPPTPAPTIASQPLSLRPEACRPAAGGAVHTRGLDFACDIYIWAPLAGTCGVLLLSLVITLYCRSKRSRLLHSDYMNMTPRRPGPTRKHYQPYAPPRDFAAYRSRVKFSRSADAPAYQQGQNQLYNELNLGRREEYDVLDKRRGRDPEMGGKPQRRKNPQEGLYNELQKDKMAEAYSEIGMKGERRRGKGHDGLYQGLSTATKDTYDALHMQALPPRGSGATNFSLLKQAGDVEENPGPMALPVTALLLPLALLLHAARPMADYKDIVMTQSHKFLLVSVGDRVSITCKASQDVSTAVAWYQQKPGQSPKLLIYSASYRYTGVPDRFIGSGSGTDFTLTISSVQAEDLADYFCQQHYSTPLTFGAGTKLEIKRGGGGSGGGGSGGGGSSGGGSEVQLKESGPGLVAPSQSLSITCTVSGFPLTSYGVSWVRQPPGKGLEWLGVIWGDGSTNYHSALISRLSISKDNSKSQVFLKLNNLQTDDTATYYCARDTYYPYYAMDYWGQGTSVTVSSTTTPAPRPPTPAPTIASQPLSLRPEACRPAAGGAVHTRGLDFACDIYIWAPLAGTCGVLLLSLVITLYCKRGRKKLLYIFKQPFMRPVQTTQEEDGCSCRFPEEEEGGCELRVKFSRSADAPAYQQGQNQLYNELNLGRREEYDVLDKRRGRDPEMGGKPQRRKNPQEGLYNELQKDKMAEAYSEIGMKGERRRGKGHDGLYQGLSTATKDTYDALHMQALPPRGSGEGRGSLLTCGDVEENPGPMYRMQLLSCIALSLALVTNSGIHVFILGCFSAGLPKTEANWVNVISDLKKIEDLIQSMHIDATLYTESDVHPSCKVTAMKCFLLELQVISLESGDASIHDTVENLIILANNSLSSNGNVTESGCKECEELEEKNIKEFLQSFVHIVQMFINTSSGGGSGGGGSGGGGSGGGGSGGGSLQAPRRARGCRTLGLPALLLLLLLRPPATRGITCPPPMSVEHADIWVKSYSLYSRERYICNSGFKRKAGTSSLTECVLNKATNVAHWTTPSLKCIR

SEQ ID NO: 61 - DNA, 3919 bp, Artificial Sequence
  Synthetic Sequence
gcgatcgcaccatggccctgcccgtgaccgccctgctgctgcccctggccctgctgctgcacgccgccaggcccgacatccagatgacccagagccacaagttcatgagcaccagcgtgggcgacagggtgagcatcacctgcaaggccagccaggacgtgagcaccgccgtggcctggttccagcagaagcccggccagagccccaagctgctgatctacagccccagctacaggtacaccggcgtgcccgacaggttcaccggcagcggcagcggcaccgacttcaccttcaccatcagcagcgtgcaggccgaggacctggccgtgtactactgccagcagctgtacagcaccccctacaccttcggcggcggcaccaagctggagatcaagggaggggggggatccgggggaggaggctccggcggaggcggaagcgaggtgcagctgcagcagagcggccccgagctggtgaagcccggcgccagcgtgaagatgagctgcaaggccagcggctacaccttcaccgactactacctggactgggtgaagcagagccacggcgagagcttcgagtggatcggcagggtgaacccctacaacggcggcaccatctacaaccagaagttcaagggcaaggccaccctgaccgtggacaagagcagcagcaccgcctacatggacctgaacagcctgaccagcgaggacagcgccgtgtactactgcgccagggaccactacaggtacgaccccctgctggactactggggccagggcaccaccctgaccgtgagcagcaccaccacccccgcccccaggccccccacccccgcccccaccatcgccagccagcccctgagcctgaggcccgaggcctgcaggcccgccgccggcggcgccgtgcacaccaggggcctggacttcgcctgcgacatctacatctgggcccccctggccggcacctgcggcgtgctgctgctgagcctggtgatcaccctgtactgcaggagtaagaggagcaggctcctgcacagtgactacatgaacatgactccccgccgccccgggcccacccgcaagcattaccagccctatgccccaccacgcgacttcgcagcctatcgctccagggtgaagttcagcaggagcgccgacgcccccgcctaccagcagggccagaaccagctgtacaacgagctgaacctgggcaggagggaggagtacgacgtgctggacaagaggaggggcagggaccccgagatgggcggcaagccccagaggaggaagaacccccaggagggcctgtacaacgagctgcagaaggacaagatggccgaggcctacagcgagatcggcatgaagggcgagaggaggaggggcaagggccacgacggcctgtaccagggcctgagcaccgccaccaaggacacctacgacgccctgcacatgcaggccctgccccccaggggaagcggagccaccaacttcagcctgctgaagcaggccggcgacgtggaggagaaccccggccccatggccctgcccgtgaccgccctgctgctgcccctggccctgctgctgcacgccgccaggcccatggccgactacaaggacatcgtgatgacccagagccacaagttcctgctggtgagcgtgggcgacagggtgagcatcacctgcaaggccagccaggacgtgagcaccgccgtggcctggtaccagcagaagcccggccagagccccaagctgctgatctacagcgccagctacaggtacaccggcgtgcccgacaggttcatcggcagcggcagcggcaccgacttcaccctgaccatcagcagcgtgcaggccgaggacctggccgactacttctgccagcagcactacagcacccccctgaccttcggcgccggcaccaagctggagatcaagaggggcggcggcggcagcggcggcggcggcagcggcggcggcggcagcagcggcggcggcagcgaggtgcagctgaaggagagcggccccggcctggtggcccccagccagagcctgagcatcacctgcaccgtgagcggcttccccctgaccagctacggcgtgagctgggtgaggcagccccccggcaagggcctggagtggctgggcgtgatctggggcgacggcagcaccaactaccacagcgccctgatcagcaggctgagcatcagcaaggacaacagcaagagccaggtgttcctgaagctgaacaacctgcagaccgacgacaccgccacctactactgcgccagggacacctactacccctactacgccatggactactggggccagggcaccagcgtgaccgtgagcagcaccaccacccccgcccccaggccccccacccccgcccccaccatcgccagccagcccctgagcctgaggcccgaggcctgcaggcccgccgccggcggcgccgtgcacaccaggggcctggacttcgcctgcgacatctacatctgggcccccctggccggcacctgcggcgtgctgctgctgagcctggtgatcaccctgtactgcaaacggggcagaaagaaactcctgtatatattcaaacaaccatttatgagaccagtacaaactactcaagaggaagatggctgtagctgccgatttccagaagaagaagaaggaggatgtgaactgagggtgaagttcagcaggagcgccgacgcccccgcctaccagcagggccagaaccagctgtacaacgagctgaacctgggcaggagggaggagtacgacgtgctggacaagaggaggggcagggaccccgagatgggcggcaagccccagaggaggaagaacccccaggagggcctgtacaacgagctgcagaaggacaagatggccgaggcctacagcgagatcggcatgaagggcgagaggaggaggggcaagggccacgacggcctgtaccagggcctgagcaccgccaccaaggacacctacgacgccctgcacatgcaggccctgccccccaggggcagcggcgaaggccgcggcagcctgctgacctgcggcgatgtggaagaaaacccgggccccatgtacagaatgcagctgctgagctgcatcgccctgagcctggccctggtgaccaacagcggcatccacgtgttcatcctgggctgcttcagcgccggcctgcccaagaccgaggccaactgggtgaacgtgatcagcgacctgaagaagatcgaggacctgatccagagcatgcacatcgacgccaccctgtacaccgagagcgacgtgcaccccagctgcaaggtgaccgccatgaagtgcttcctgctggagctgcaggtgatcagcctggagagcggcgacgccagcatccacgacaccgtggagaacctgatcatcctggccaacaacagcctgagcagcaacggcaacgtgaccgagagcggctgcaaggagtgcgaggagctggaggagaagaacatcaaggagttcctgcagagcttcgtgcacatcgtgcagatgttcatcaacaccagctccggcggcggctccggcggcggcggctccggcggcggcggctccggcggcggcggctccggcggcggctccctgcaggcccccagaagagccagaggctgcagaaccctgggcctgcccgccctgctgctgctgctgctgctgagaccccccgccaccagaggcatcacctgccccccccccatgagcgtggagcacgccgacatctgggtgaagagctacagcctgtacagcagagagagatacatctgcaacagcggcttcaagagaaaggccggcaccagcagcctgaccgagtgcgtgctgaacaaggccaccaacgtggcccactggaccacccccagcctgaagtgcatcagataagtttaaac